European Patent Specification EP 3 244 727 B1, published October 22, 2025. Title: INSECTICIDAL PROTEINS AND METHODS FOR THEIR USE. Applicant: Pioneer Hi-Bred International INc. Steve, Gruver Heather, Kozy Jessica, O'Rear Rosen, Barbara Schellenberger, Ute Wei, Zun-Zhi Xie, Weiping Zhong, Xiaohong Zhu, Genhai. The sequence listing filed with the application follows.

SEQUENCE LISTING (245 sequences)

SEQ ID NO: 1 - protein, 578 aa, Pseudomonas brenneri
MSTPFKQFTSPAGQAPKDYNKLGLENQLPQFETDWNNDLTGWTQSAIIGNPWSGLNDAPRSGYYNPLVEGYGPTTPPAITWAPFPNRLWTFFYNNGTAVIPQLGGKAMSLQQVMELTDNGQITINNTLYMLYDPNKQGTLLQLPVTRCPTIDWQGKYKDFSPSGPRGWLDEYCEWSIVRDADGNMRKITFTCENPAYFLAMWRIDPNAVLGLYRDYIDPQVQLEDLYLRYTADCPTGKAGDPVIDPTTGQPAYDTVNKWNAGTACVPGQYGGAMHLTSGPNTLSAEVYLAAAATILRPLASSQNSQALICCAQYGQNYRNSDPHIGFSANSVAVNNRLSLTNPIGLYLQQPTDFSAWKGPQGQDVSQYWKITRGTAKSAANGSDQILQAVFEVPVSAGFSINDITISGQPIDYVWVIAQQLLVGLSVTTTPISPTPDSCPCVKDRVNGVQPWPVQLLPLDLFYGQSPTDLPAWLAPGTSGQFALVVQGADLKTTAETARVQFSNPGVTAQVTQFLPDASAIPGQTNSGGTQGYLLTITVSPTAAPGLVTVRALNPGEADNPSATEHPWESGLALVPGA

SEQ ID NO: 2 - protein, 535 aa, Pseudomonas brenneri
MSRLRLSVLSLLTSVVLSLFAMQAAYASPTSDADACVQQQLVFNPKSGGFLPINNFNATGQSFMNCFGWQLFIALNWPVNPGWPATPALAGEPDMNSTLAQFGVPTASGQPMSVAPVWASYKDANDIFLPGAPAPTGWGVQTLVPSNCSTQGSLRAISVGARKFMTATSESAINARHGFHLSSGTLASIPDPIMEASGGWLTDQSQNLVFFERKVGKAEFDYIVSKGLYDAANQLTVAQNLDNQNPGGLSLPIGEPMRSLPPNPVPQEQLGALEVKAAWRILTGKPELYGRYLTTVAWLKNPATLQCTQQVVGLVGLHIINKTQASPNFIWTTFEQVDNVPEPNQVPPQQTPPDSFAFNNPNCGTGPECTPNVARIQCKQHHPDRDCTEPFPRDQPVQTTREHPLPTELQALNGAVQANFAQQSQGKSVFQYYKLINVLWTLTPNPPTQPEPGVSAQVPLSYGPFISQGNVPVANTTLETYVQGDNCNACHQYATIAGSSTLASDFSFLFNSADSASKNSLVKRVKAFQTLKDQP

SEQ ID NO: 3 - protein, 578 aa, Pseudomonas sp. Ag1
MSTPFKQFTSPAGQAPKDYNKLGLENQLPQFETDWNNDLTGWTQSAIIGNPWSGLNDAPRSGYYNPLVEGYGPTTPPAITWAPFPNRLWTFFYNNGTAVIPQLGGKAMSMQQVMELTDNGQITINNTLYMLYDPNKQGTLLQLPVTRCPSIDWQGKYKDFSPSGPRGWLDEYCEWSIVRDADGNMRKITFTCENPAYFLAMWRIDPTAVLGLYRDYIDPQVQLEDLYLRYTADCPTGKAGDPVIDPTTGQPAYDTVNKWNAGTACVPGQYGGAMHLTSGPNTLSAEVYLAAAATILRPLSSSQNSQALICCAQYGQNYRNSDPHIGFSANSVAVNNRLSLTNPIGLYLQQPTDFSAWKGPQGQDVSQYWKITRGTAKSAANGSDQILQAVFEVPVSAGFSINEITISGQPIDYVWVIAQQLLVGLSVTTTPISPTPDSCPCVTDRVNGVQPWPVQLLPLDLFYGQSPTDLPAWLAPGTSGQFALVVQGADLKTTAETARVQFSNPGVTAQVTKFLPDASAIPGQTNSGGTQGYLLTITVSPTAAPGLVTVRALNPGEADNPSAAEHPWESGLALVPGA

SEQ ID NO: 4 - protein, 536 aa, Pseudomonas sp. Ag1
MSRLRLSVLSLLTSVVLSLFAMQAAYASPTSDADACVQQQLVFNPKSGGFLPINNFNATGQSFMNCFGWQLFIALNWPVNPGWPATPALAGEPDMNSTLAQFGVPTASGQPMSVAPVWASYKDANDIFLPGAPAPTGWGVQTLVPSNCSTQGSLRAMSVGARKFMTATSESAINARHGFHLSSGTLASIPDPIMEASGGWLTDQSQNLVFFERKVGKAEFDYIVSKGLYDAANQLKVAQNLDNQNPGGLSLPIGEPMRSLPPNPVPQEQLGALEVKAAWRILTGKPELYGRYLTTVAWLKNPATLQCTQQVVGLVGLHIINKTQASPNFIWTTFEQVDNVPEPDQVPPQQTPPDSFAFNNPNCGTGPECTPNVARIQCKQQHPDRDCTEPFPRDQPVQTTREHPLPTELQALNGAVQANFAQQSQGKSVFQYYKLINVLWTLTPNPPTQPEPGVSAQVPLSYGPFISQGNVPVANTTLETYVQGDNCNACHQYATIAGSSTLASDFSFLFNSADSASKKSLVKRVKAFQTLKDGSP

SEQ ID NO: 5 - protein, 579 aa, Pseudomonas sp. PAMC 25886
MSTPFNQFTSPAGQAPKDYNKLGLENQLPQFETDWNNDLTGWTQSAIIGNPWSGLNDAPRSGYYNPLVEGYGPTTPPAITWAPFPNRLWTFFYNNGTAVIPQLGGKAMTLQQVMELTDNGQITLNNTLYTLYDPNKQGTLLQLPVTRCPSIDWQGKYKDFSPSGPRGWLDEYCEWSIVRDPGTQNMRKITFTCENPAYFLAMWRIDPNAVLGLYRDYIDPQVQLEDLYLRYTADCPTGNKGDPVMDPTTGQPAYDTVNKWNAGTACVPGQYGGAMHLTSGPNTLSAEVYLAAAATILRPLASSQNSQALICCAQYGQNYRNSDPHIGFSANSVAVNNRLSLTNPIGLYLQQPTDFSAWKGPQGQDVSQYWKITRGTAKSAANGSDQILQAVFEVPVSAGFSINDITISGQSIDYVWVIAQQLLVGLSVTTTPISPTPESCPCVTDRVTGVQPWPVQLLPLDLFYGQSPTDLPAWLAPGTSGQFALVVQGADLKTTAETARVQFSNPGVTAVVTKFLPDASAIPGQTNSGGTQGYLLTITVSPTAAPGLVTVRALNPGEADNPSAAQHPWESGLALVPGA

SEQ ID NO: 6 - protein, 535 aa, Pseudomonas sp. PAMC 25886
MSRLRLSVLSLLTSVVLSLFAVQSAYATPQSDADACVQQQLVFNPASGGFLPVNNFNATGQSFMNCFGWQLFIALNWPVNPGWPATPALAGEPDMHSSLAQFGVPPASGQPMTVAPVWASYKDANDIFLPGAPVPTGWGVQTLVPSNCSTQGSLKAMAVGARKFMTATSESAINARHGFHLSSGTLASIPDPIMEASGGWLTDQSKNLVFFERKVGKAEFDYIVSKGLYDAANQLTVAQNLDNQNPGGLSLPIGEPMRSLPPDPVPQEQLGALEVKAAWRILTGKPELYGRYLTTVAWLKNPATLQCTQQVVGLVGLHIINKTQASPNFIWTTFEQVDNVPEPDQVPPQQTPPDSFAFNNPNCGTGPECTPNVARIQCKQHHPDRDCTEPYPRDQPVQTTREHPLPTELQALNGAVQANFAQQSQGKSVFQYYKLINVLWTLTPNPPTQPEPGVSAQVPLSYGPFISQGNVPVANTTLETYVQGDNCNACHQYATIAGSSTLASDFSFLFNSADSASKKSLVKRVKAFETLKDQP

SEQ ID NO: 7 - protein, 579 aa, Pseudomonas sp. PAMC 25886
MSTPFKQFTSPAGQAPKDYNKLGLENQLPQFETDWNNDLTGWTQSAIIGNPWSGLNDAPRSGYYNPLVEGYGPTTPPAITWAPFPNRLWTFFYNNGTAVIPQLGGKAMTLQQVMELTDNGQITLNNTLYTLYDPNKQGTLLQLPVTRCPSIDWQGKYKDFSPSGPRGWLDEYCEWSIVRDPGTQNMRKITFTCENPAYFLAMWRIDPNAVLGLYRDYIDPQVQLEDLYLRYTADCPTGNKGDPVMDPTTGQPAYDTVNKWNAGTACVPGQYGGAMHLTSGPNTLSAEVYLAAAATILRPLSSSQNSQALICCAQYGQNYRNSDPHIGFSANSVAVNNRLSLTNPIGLYLQQPTDFSAWKGPQGQDVSQYWKITRGAAKSAANGSDQILQAVFEVPVSAGFSINDITISGQSIDYVWVIAQQLLVGLSVTTTPISPTPDSCPCVTDRVNGVQPWPVQLLPLDLFYGQSPTDLPAWLAPGTSGQFALVVQGADLKTTAETARVQFSNPGVTAVVTKFLPDASAIPGQTNSGGTQGYLLTITVSPTAAPGLVTVRALNPGEADNPSAAEHPWESGLALVPGA

SEQ ID NO: 8 - protein, 535 aa, Pseudomonas sp. PAMC 25886
MSRLRLSVLSLLASVVLSLFALQSAYATPQSDADACVQQQLVFNPKSGGFLPVNNFNATGQSFMNCFGWQLFIALNWPVNPGWPTTAALAGEPDMNSSLAQFGVPTTAGQPMTVAPVWASYKDANDIFLPGAPVPSGWGVQTLVPSNCSTQGSLKAMSVGARKFMTATSESAINARHGFHLSSGTLATIPDPIMEASGGWLTDQAGQLVFFERKVGKAEFDYIVSKGLYDAANQLKVAQNLDNQNPGGLSLPIGEPMRSLPPTPVPQEQLGALELKAAWRILTGKPELYGRYLTTVAWLKNPATLQCTQQVVGLVGLHIINKTQASPNFIWTTFEQVDNVPEPNQLPPQQTPPDSFAFNNPNCGTGPECTPNVARIQCQQHHPDRDCTEPYPRDQPVQTTREHPLPTELQALNGAVQANFAQQSQGKSVFQYYKLINVLWTLTPNPPVQPEPGVSAAVPLSYGPFISQGNVPVANTTLETYVQGDNCNACHQYATIAGSSTLASDFSFLFNSADSASKKSLVKRVKAFETLKDQP

SEQ ID NO: 9 - protein, 578 aa, Pseudomonas fluorescens
MSTPFKQFTSPAGQAPKDYNKLGLENQLPQFETDWNNDLTGWTQSAIIGNPWSGLNDAPRSGYYNPLVEGYGPTTPPAITWAPFPNRLWTFFYNNGTAVIPQLGGKAMSMQQVMELTDNGQITINNTLYMLYDPKKQGTLLQLPVTRCPSIDWQGKYKDFSPSGPRGWLDEYCEWSIVRDADGNMRKITFTCENPAYFLAMWRIDPTAVLGLYRDYIDPQVQLEDLYLRYTADCPTGKAGDPVIDPTTGQPAYDTVNKWNAGTACVPGQYGGAMHLTSGPNTLSAEVYLAAAATILRPLSSSQNSQALICCAQYGQNYRNSDPHIGFSANSVAVNNRLSLTNPIGLYLQQPTDFSAWKGPQGQDVSQYWKITRGTAKSAANGSDQILQAVFEVPVSAGFSINDITISGQPIDYVWVIAQQLLVGLSVTTTPISPTPDSCPCVTDRVNGVQPWPVQLLPLDLFYGQSPTDLPAWLAPGTSGQFALVVQGADLKTTAETARVQFSNPGVTAQVTKFLPDASAIPGQTNSGGTQGYLLTITVSPTAAPGLVTVRALNPGEADNPSAAEHPWESGLALVPGA

SEQ ID NO: 10 - protein, 536 aa, Pseudomonas fluorescens
MSRLRLSVLSLLTSVVLSLFAMQAAYASPTSDADACVQQQLVFNPKSGGFLPINNFNATGQSFMNCFGWQLFIALNWPVNPGWPATPALAGEPDMNSTLAQFGVPTASGQPMSVAPVWASYKDANDIFLPGAPVPTGWGVQTLVPSNCSTQGSLRAMSVGARKFMTATSESAINARHGFHLSSGTLASIPDPIMEASGGWLTDQSQNLVFFERKVGKAEFDYIVSKGLYDAANQLKVAQNLDNQNPGGLSLPIGEPMRSLPPNPVPQEQLGALEVKAAWRILTGKPELYGRYLTTVAWLKNPATLQCTQQVVGLVGLHIINKTQASPNFIWTTFEQVDNVPEPNQVPPQQTPPDSFAFNNPNCGTGPECTPNVARIQCKQQHPDRDCTEPFPRDQPVQTTREHPLPTELQALNGAVQANFAQQSQGKSVFQYYKLINVLWTLTPNPPTQPEPGVSAQVPLSYGPFISQGNVPVANTTLETYVQGDNCNACHQYATIAGSSTLASDFSFLFNSADSASKKSLVKRVKAFQTLKDGSP

SEQ ID NO: 11 - protein, 578 aa, Pseudomonas sp. PAMC 26793
MSTPFKQFTSPAGQAPKDYNKLGLENQLPQFETDWNNDLTGWTQSAIIGNPWSGLNDAPRSGYYNPLVEGYGPSTPPAITWAPFPNRLWTFFYNNGTAVIPQLGGKAMSMQQVMELTDNGQITINNTLYMLYDPNKQGTLLQLPVTRCPTIDWQGKYKDFSPSGPRGWLDEYCEWSIVRDANGNMRKITFTCENPAYFLAMWRIDPNAVLGLYRDYIDPQVQLEDLYLRYTADCPTGKAGDPVIDPTTGQPAYDTVNKWNAGTACVPGQYGGAMHLTSGPNTLSAEVYLAAAATILRPLASSQNSQALICCAQYGQNYRNSDPHIGFSANSVAVNNRLSLTNPIGLYLQQPTDFSAWKGPQGQDVSQYWKITRGTAKSAANGSDQILQAVFEVPVSAGFSINDITISGQPINYVWVIAQQLLVGLSVTTTPISPTPDSCPCVTDRVNGVQPWPVQLLPLDLFYGQSPTDLPAWLAPGTSGQFALVVQGADLKTTAETARVQFSNPSVTAQVTQFLPDASAIPGQTNSGGTQGYLLTITVSPTAAPGLVTVRALNPGEADNPSATEHPWESGLALVPGA

SEQ ID NO: 12 - protein, 535 aa, Pseudomonas sp. PAMC 26793
MSRLRLSVLSLLTSVVLSLFAMQAAYASPTSDADACVQQQLVFNPKSGGFLPINNFNATGQSFMNCFGWQLFIALNWPVNPGWPATPALAGEPDMNSTLAQFGVPPASGQPMSVAPVWASYKDANDIFLPGAPAPTGWGVQTLVPSNCSTQGSLRAMSVGARKFMTATSESAINARHGFHLSSGTLASIPDPIMEASGGWLTDQSQNLVFFERKVGKAEFDYIVSKGLYDAANQLKVAQNIDNQNPGGLSLPIGEPMRSLPPNPVPQEQLGALEVKAAWRILTGKPELYGRYLTTVAWLKNPATLQCTQQVVGLVGLHIINKTQASPNFIWTTFEQVDNVPEPNQVPPQQTPPDSFAFNNPNCGTGPECTPNVARIQCKQHHPDRDCTEPFPRDQPVQTTREHPLPTELQALNGAVQANFAQQSQGKSVFQYYKLINVLWTLTPNPPTQPEPGVSAQVPLSYGPFISQGNVPVANTTLETYVQGDNCNACHQYATIAGSSTLASDFSFLFNSADSASKKSLVKRVKAFQTLKDQP

SEQ ID NO: 13 - protein, 578 aa, Pseudomonas putida
MSTPFKQFTSPAGQAPKDYNKLGLEDQLPQFETDWNNNLTGWTESSIIGNPWSGLNDAPRSGYYNPLVEGFGDVTAPAITWAPFPNRLWTFFYNNGAAVIPQLGGKAMTLDQVMELTDHGQITLDNTLYMLYDPNKQGTVLQLPAKRCPSIDWNGKYTAFSPSGPRGWLDEYCEWSIVRDANGNMRKITFTCENPAYFLTMWRIDPNAVLGLYRDYIDPNVQLEDLYLRYTVDCPTGKAGDPVIDPTTGKPAYDTVNKWNAGTACVPGQYGGAMHLTSGPNTLSAEVYLAAAATILRPVSSSQNAQSLICCAQYGQNYRNSDPHIGFMANTTAVNNRLSLTNPIGLYLQQPTDFSAWKGPQGQDVSQYWRITRGTAKSAANGSDQILQAVFEVPESAGFSINDITINNQKVNYVWVIAQQLLVGLSVTVKPLSATLQAFPCVQDRVAGLQPWPVQLLPLDLFYGQSPTDLPAWLAPGSSNQFVLVVQGADPTTTAQNARVQFSNPGVTAQVTQYLPDASAIPGQTNSGGTQAYILTITVSPSAAPGLVTVRALNPGEDVNVSATDHPWESGLALVPGA

SEQ ID NO: 14 - protein, 535 aa, Pseudomonas putida
MMSRSRLSPLSLLCGILLCLSTLQPATAATLSDADTCVQQQLVFNPASGGFLPVNNFNATSQAFMNCFGWQLFIALNWPVNPGWPATASLAGEPDMQSTLAQFGVPSAPGQPMSVAPVWASYKDANDIFLPGAPTPTGWGVQTLVPSGCSTQGSLKALKVGARKFMNATSEGAINALHGFHLSTGTLASIPDPVMEASGGWLTDQAGKLVFFERKVGKAEFDYIVDKGLYDAANQLKVAQNLDGQTPEGLSLPIGEPMRSLPTSPVPQEQLGAIELKAAWRVLTGKPELFGRYLTTVAWLKRPDTLECTQEVVGLVGLHIINKTQASPNFIWTTFEQVDNVPEPAQVPPQQTPPNGFAFNNPDCGDGPECTPNQARIQCKQTHPDKDCTDLFPRDQPVQTTREHPVPGDLQALNSAVQANFAQHSQGKSVFQYYKLINVLWTLAPNPPSPEPGANAQVPLSYGPFISQGNVPVANTTMETYVQGDDCNQCHQYATIAGSPSLASDFSFLFNSAGSASNKSLIKSVKAFETLKDRP

SEQ ID NO: 15 - protein, 578 aa, unknown
  Fungus garden combined
MSTPFKQFTSPAGQAPKDYNKLGLEDQLPQFETDWNNNLTGWTESSIIGNPWSGLNDAPRSGYYNPLVEGFGDVTAPAITWAPFPNRLWTFFYNNGAAVIPQLGGKAMTLDQVMALTDHGQITLDNTLYMLYDPNKQGTVLQLPAKRCPSIDWNGKYTAFSPSGPRGWLDEYCEWSIVRDANGNMRKITFTCENPAYFLTMWRIDPNAVLGLYRDYIDPNVQLEDLYLRYTVDCPTGKAGDPVIDPTTGKPAYDTVNKWNAGTACVPGQYGGAMHLTSGPNTLSAEVYLAAAATILRPVSSSQNAQSLICCAQYGQNYRNSDPHIGFMANTTAVNNRLSLTNPIGLYLQQPTDFSAWKGPQGQDVSQYWRITRGTAKSAANGSDQILQAVFEVPESAGFSINDITINNQKVNYVWVIAQQLLVGLSVTVKPLSTTPQAFPCVQDRVAGRQPWPVQLLPLDLFYGQSPTDLPAWLAPGSSNQFVLVVQGADPTTTAQNARVQFSNPGVTAQVTQYLPDASAIPGQTNSGGTQAYILTITVSPSAAPGLVAVRALNPGEDVNVSATDHPWESGLALVPGA

SEQ ID NO: 16 - protein, 534 aa, unknown
  Fungus garden combined
MSRSRLSLLSLLCGILLCLSTPQPATAATLSDADTCVQQQLVFNPASGGFLPVNNFNATSQAFMNCFGWQLFIALNWPVNPGWPATASLAGEPDMQSTLAQFGVPSAPGQPMSVAPVWASYKDANDIFLPGAPTPTGWGVQTLVPSGCSTQGNLKALKVGARKFMNATSEGAINALHGFHLSTGTLASIPDPVMEASGGWLTDQAGKLVFFERKVGKAEFDYIVDKGLYDAANQLKVAQNLDGQTPEGLSLPIGEPMRSLPTSPVPQEQLGAIELKAAWRVLTGKPELFGRYLTTVAWLKRPDTLECTQEVVGLVGLHIINKTQASPNFIWTTFEQVDNVPEPAQVPPQQTPPNGFAFNNPDCGDGPECTPNQARIQCKQTHPDKDCTDLFPRDQPVQTTREHPVPGDLQALNSAVQANFAQHSQGKSVFQYYKLINVLWTLAPNPPSPEPGANAQVPLSYGPFISQGNVPVANTTMETYVQGDDCNQCHQYATIAGSPSLASDFSFLFNSAGSASNKSLIKSVKAFETLKDRP

SEQ ID NO: 17 - protein, 578 aa, Pseudomonas monteilii
MSTPFKQFTSPAGQAPKDYNKLGLEDQLPQFETDWNNNLTGWTESSIIGNPWSGLNDAPRSGYYNPLVEGFGDVTAPAITWAPFPNRLWTFFYNNGAAVIPQLGGKAMTLDQVMELTDHGQITLDNTLYMLYDPNKQGTVLQLPAKRCPSIDWNGKYTAFSPSGPRGWLDEYCEWSIVRDANGNMRKITFTCENPAYFLTMWRIDPNAVLGLYRDYIDPNVQLEDLYLRYTVDCPTGKAGDPVIDPTTGKPAYDTVNKWNAGTACVPGQYGGAMHLTSGPNTLSAEVYLAAAATILRPVSSSQNAQSLICCAQYGQNYRNSDPHIGFMANTTAVNNRLSLTNPIGLYLQQPTDFSAWKGPQGQDVSQYWRITRGTAKSAANGSDQILQAVFEVPESAGFSINDITINNQKVNYVWVIAQQLLVGLSVTAKPLSATPQAFPCVQDRVAGLQPWPVQLLPLDLFYGQSPTDLPAWLAPGSSNQFVLVVQGADPTTTAQNARVQFSNPGVTAQVTQYLPDASAIPGQTNSGGTQAYILTITVSPSAAPGLVALRALNPGEDVNVSATDHPWESGLALVPGA

SEQ ID NO: 18 - protein, 535 aa, Pseudomonas monteilii
MMSRSRLSLLSLLCGILLCLSTPQPATAATLSDADTCVQQQLVFNPASGGFLPVNNFNATSQAFMNCFGWQLFIALNWPVNPGWPATASLAGEPDMQSTLAQFGVPSTPGQPMSVAPVWASYKDANDIFLPGAPTPTGWGVQTLVPSDCSTQGSLKTLKVGARKFMNATSEGAINALHGFHLSTGTLASIPDPVMEASGGWLTDQAGKLVFFERKVGKAEFDYIVDKGLYDAANQLKVARNLDGQTPEGLSLPIGEPMRSLPTSPVPQEQLGAIELKAAWRVLTGKPELFGRYLTTVAWLKRPDTLECTQEVVGLVGLHIINKTQASPNFIWTTFEQVDNVPEPAQVPPQQTPPNGFAFNNPDCGNGPECTPNQARIQCKQTHPDKDCTDLFPRDQPVQTTREHPVPGDLQALNSAVQANFAQHSQGKSVFQYYKLVNVLWTLAPNPPSPEPGANAQVPLSYGPFISQGNVPVANTTMETYVQGDNCNQCHQYATIAGSPSLASDFSFLFNSAGSASNKSLIKSVKAFETLKDRP

SEQ ID NO: 19 - protein, 578 aa, Pseudomonas monteilii
MSTPFKQFTSPAGQAPKDYNKLGLEDQLPQFETDWNNNLTGWTQSSIIGNPWSGLNDAPRSGYYNPLVEGFGDVTPPAITWAPFPNRLWTFFYNNGAAVIPQLGGKAMTLDQVMELADHGQITLDNTLYTLYDPNKKGTVLQLPVKRCPSIAWNGTYKDFTPSGPRGWLDEYCEWSIVRDANGNMRKITFTCENPAYFLAMWRIDPNAVLGLYREYIDPSVQLEDLYLRYAEDCPTGKAGDPVMDPTTGKPAYDTVNKWNAGTACVPGQYGGAMHLTSGPNTLSAEVYLAAAATILRPVSSSQNAQSLICCAQYGQNYRNSDPHIGFMANTTAVNNRLSLTNPIGLYLQQPTDFSAWKGPQGQDVSQYWRITRGTAKSAANGSDQILQAVFEVPESAGFSINDITINNQKVNYVWVIAQQLLVGLSVTVKPLSVTPQSFPCVQDRVAGLQPWPVQLLPLDLFYGNSPTDLPAWLAPGSSNQFVLVVQGADKTTTAQNARVQFSNPGVTAQVTQYLPDASAIPGQTNAGGTQAYILTITVSPTAAPGLVTVRALNPDEDVNVSAADHPWESGLALVPGA

SEQ ID NO: 20 - protein, 534 aa, Pseudomonas monteilii
MSRSRLSLLSLLCGILLCLSTPQPAMAATLSDADACVQQQLVFNPASGGFLPVNNFNATSQAFMNCFGWQLFIALNWPVNPGWPATASLAGEPDMNSTLAQFGVPSAPGQPMSVAPVWASYKDANDIFLPGAPTPTGWGVQTLVPSGCSTQGSLKSLKVGARKFMNATSEGAINALHRFHLSTGTLASIPDPVMEASGGWLTDQSGNLVFFERKVGKAEFDYIVDKGLYDAANQLKVAQNQDGKTPEGLSLPIGEPMRSLPPSPVPQEQLGAIELKAAWRVLTGKPELFGRYLTTVAWLKRPDTLNCTQEVVGLVGLHIINKTQASPNFIWTTFEQVDNVPEPAQAPPQQTPPNGFAFNNPDCGSGPECTPNQARIQCKQHHPDKQCTDLFPRDQPVQTTREHPIPSDLQALNSAVQANFAQHSQGQSVFQYYKLINVLWTLAPNPPSPEPGANAQVPLSYGPFISQGNVPVANTTMETYVQGDDCNQCHQYATIAGSPSLASDFSFLFNSAGSASTKSLIKSVKAFQTLKDQP

SEQ ID NO: 21 - protein, 581 aa, Pseudomonas brenneri
MSTPFKQFTSPAGQAPKDYNKLGLEDQLPQFETDWNNDITGWTEAAIIGNPWSGLYDAPRSAYYNPLVEGYGDTTLPAITWQPFPNRLWTFFYNNGTAVIPQLGNKAMTLQQVMELTDNGQITINGTLYTLYDPDKKGTLLQLPVTRCPTIDWNGKYKDFSPSGPRGWLDEYCEWSIVRDTNGNMRKITFTSENPAYFLAMWRIDPNAVLGLYRDYIDPNVQLQDLYLRYTADCKTGKAGDPVIDPTTGLPAYDTVNKWNSGTACTPGQFGGAMHLTSGPNTLSAEVYLAAAATIMRPLKSSQSAQALICCAQYGQNYRNSDPHIGFAANGATNDGATPSRISLTNPIALYLQQPTNFNAWKGPQGQDVSQYWRITRGTAKSAINGSDQILQAVFEVPESAGFSINDITINGQAVDYVWVIAQQLLVGLSVTTMPSTAQQQSPCVQDRVNGLQPWPVQLLPLDLFYGQSPTDLPAWLAPGTSGQFALVVQGADLKTTAATARIQFNNPGVTAQVTEFLPDASAIPGQTNAGGTQGYIMTITVAKDAAPGLVTVRALNPGEADNVSAADHPWESGLALVPST

SEQ ID NO: 22 - protein, 532 aa, Pseudomonas brenneri
MYRFRLRGLLLVGTLLSLFLLPTAQASDADTCVQQQLVFDPNSGGFLPVNNFNTTGQSFMNCFGWQLFIALNWPVDPGWPANAALAGEPNRKISMAQFGVPQVAGQPMTTAPVWASFKDANDIFLPGARPPTGWGVQTLVPSNCSSEGSLKALSVGARKFMNATSESATNAKHRFHLSSGTLASIPDPIMEAAGGWLTDQTGNLVYFERKVGKAEFDYIVKYGLYDAANQMVVAQNSDGNHPAGLSLPAGELMRSMPAQPLPQEQLGALELKAAWRILTGKPQLYGRYLTTVAWLKNPATLQCTQQVVGLVGLHIINKTQSSPNFIWTTFEQVDNVQEPGQVPAQQTPPDGFTFYNPNCTGGPDVCTPNVARIQCQQHHPDRECTEPYPRNQPVQTTREHPLPSDMQALNGAVQANFAQQTNGQSVFQYYKLVNVLWITAPTAPDPEPGAGAKVPLSYGAFISDSNVPVANTTMETYVQSMDCNACHQQATIAGSSSLASDFSFLFNNADSAKQKSLIKRVNAFETLKDGPP

SEQ ID NO: 23 - protein, 577 aa, Pseudomonas gessardii
MSTPFKQFTSPAGQAPKDYNKLGLEDQLPQFETDWNNDVTGWTEAAIIGNPWSGLYDAPRSGYYNPLVEGYGDTTPPAITWQPFPNRLWTFFYSNGTAVIPQLGGKAMTLQQVMELTDNGQITINDTLYTLYDPDKKGTLLQLPVTRCPSIDWNGKYKDFSPSGPRGWLDEYCEWSIVRDANGDMRKITFTSENPAYFLAMWRIDPNAVLGLYRDYIDPNVQLEDLYLRYATDCPTGNAGDPVIDPTTGLPAYDTVNKWNAGTACTPGQFGGAMHLTSGPNTLSAEVYLAAAATIMRPLKSSQNPQSLICCAQYGQNYRNSDPHIGFAANEAAISNRISLTNPIALYLQQPTNFSAWKGPQGQDVSQYWRITRGTAKSAINGSDQILQAVFEVPQSAGFSINDITINGQAVDYVWVIAQQLLVGLSVTVMPSTTAAPSPCVQDRVNGLQPWPVQLLPLDLFYGQSPTDLPAWLAPGSSGQFVLVVQGADLQTTAATARIQFSNPGVTAQVTKFMPDASAIPGQTNAGGTQGYIMTISVAANAAPGLVTVRALNPGEADNVSAADHPWESGLALVPST

SEQ ID NO: 24 - protein, 532 aa, Pseudomonas gessardii
MSRFRLSRLLLVSTLLSLFILPLAHASDADNCVQQQLVFNPKSGGFMPVNNFNTTGQSFMNCFGWQLFIALNWPVDPGWPANASLAGEPDRTITVAQFGVPTTAGQPMSVAPVWASYKDANEIFLPGAPKPSGWGVQTLVPPNCSSQDSLQALSVGARKFMNATSESATNAKHRFHLSSGTLASIPDPIMEAAGGWLTDQTGNLVYFERKVGKAEFDYIVDNGLYDAANQLIVAQNSDGKHPAGLSLPAGELMRSMPTTPLPQEQLGALELKAAWRILTGQPQLYGRYLTTVAWLKNPATLQCTQQVVGLVGLHIINKTQSSPNFIWTTFEHVDNVPEPGQVPAQQLPPDGYTFNNPNCTGGPDVCTPNVARIQCKQHHPDRECTEPYPRDQPVQTTREHPLSSDMQALNGAVQASFAQQTNGQSVFQYYKLINVLWITAPTPPDPEPGPNAKVPLSYGAFISDSNVPVANTTLETYVQGMNCNDCHQQATIAGSATLASDFSFLFNNADSAKHTSLIKRVHAFETLKDGQP

SEQ ID NO: 25 - protein, 578 aa, Pseudomonas putida
MSAPFKQFTSPAGQAPKDYNKLGLEDQLPQFETDWNNNLTGWTESSIIGNPWSGLNDAPRSGYYNPLVEGFGDVTAPAITWAPFPNRLWTFFYNNGAAVIPQLGGKAMTLDQVMALTDHGQITLDNTLYMLYDPNKQGTVLQLPAKRCPSIDWNGKYTAFSPSGPRGWLDEYCEWSIVRDANGNMRKITFTCENPAYFLTMWRIDPNAVLGLYRDYIDPNVQLEDLYLRYTVDCPTGKAGDPVIDPTTGKPAYDTVNKWNAGTACVPGQYGGAMHLTSGPNTLSAEVYLAAAATILGPVSSSQNAQSLICCAQYGQNYRNSDPHIGFMANTTAVNNRLSLTNPIGLYLQQPTDFSAWKGPQGQDVSQYWRITRGTAKSAANGSDQILQAVFEVPESAGFSINDITINNQKVNYVWVIAQQLLVGLSVTVKPLSTAPQAFPCVQDRVAGLQPWPVQLLPLDLFYGQSPTDLPAWLAPGSSNQFVLVVQGADPTTTAQNARVQFSNPGVTAQVTQYLPDASAIPSQTNSGGTQAYILTITVSPSAAPGLVAVRALNPGEDVNVSATDHPWESGLALVPGA

SEQ ID NO: 26 - protein, 534 aa, Pseudomonas putida
MSRSRLSLLSLLCGILLCLSTPQPATAATLSDADTCVQKQLVFNPASGGFLPVNNFNATSQAFMNCFGWQLFIALNWPVNPGWPATASLAGEPDMQSTLAQFGVPSAPGQPMSVAPVWASYKDANDIFLPGAPTPTGWGVETLVPSGCSTQGSLKALKVGARKFMNATSEGAINALHGFHLSTGTLASIPDPVMEASGGWLTDQAGKLVFFERKVGKAEFDYIVDKGLYDAANQLKVAQNLDGQTPEGLSLPIGEPMRSLPTSPVPQEQLGAIELKAAWRVLTGKPELFGRYLTTVAWLKRPDTLECTQEVVGLVGLHIINKTQASPNFIWTTFEQVDNVPEPAQVPPQQTPPNGFAFNNPDCGDGPECTPNQARIQCKQTHPDKDCTDLFPRDQPVQTTRVHPVPGDLQALNSAVQANFAQHSQGKSVFQYYKLINVLWTLAPNPPSPEPGANAQVPLSYGPFISQGNVPVANTTMETYVQGDDCNQCHQYATIAGSPSLASDFSFLFNSAGSASNKSLIKSVKAFETLKDRP

SEQ ID NO: 27 - protein, 578 aa, Pseudomonas plecoglossicida
MSTPFKQFTSPAGQAPKDYNKLGLEDQLPQFETDWNNNLTGWTESSIIGNPWSGLNDAPRSGYYNPLVEGFGDVTAPAITWAPFPNRLWTFFYNNGAAVIPQLGGKAMTLDQVMELTDHGQITLDNTLYMLYDPNKRGTVLQLPAKRCPSIDWNGKYTAFSPSGPRGWLDEYCEWSIVRDANGNMRKITFTCENPAYFLTMWRIDPNAVLGLYRDYIDPNVQLEDLYLRYTADGPTGKAGDPVIDPTTGKPAYDTVNKWNAGTACVPGQFGGAMHLTSGPNTLSAEVYLAAAATILRPVSSSQNAQSLICCAQYGQNYRNSDPHIGFMANTTAVNNRLSLTNPIGLYLQQPTDFSAWKGPQGQDVSQYWRITRGTAKSAANGSDQILQAVFEVPESAGFSINDITINNQKVNYVWVIAQQLLVGLSVTVKPLSTTPQAFPCVQDRVAGLQPWPVQLLPLDLFYGQSPTDLPAWLAPGSSNQFVLVVQGADPTTTAQNARVQFSNPGVTAQVTQYLPDASAIPGQTNSGGTQAYILTITVSPSAAPGLVTVRALNPGEDVNVSATDHPWESGLALVPGA

SEQ ID NO: 28 - protein, 534 aa, Pseudomonas plecoglossicida
MSRSRLSLLSLLCGILLCLSTLQPATAATLSDADTCVQQQLVFNPASGGFLPVNNFNATSQAFMNCFGWQLFIALNWPVNPGWPATASLAGEPDMQSTLAQFGVPSAPGQPMSVAPVWASYKDANDIFLPGAPTPTGWGVQTLVPSGCSTQGSLKALKVGARKFMNATSEGAINALHGFHLSTGTLASIPDPVMEASGGWLTDQAGKLVFFERKVGKAEFDYIVDKGLYDAANQLKVAQNLDGQTPEGLSLPIGEPMRSLPTSPVPQEQLGAIELKAAWRVLTDKPELFGRYLTTVAWLKRPDTLECTQEVVGLVGLHIINKTQASPNFIWTTFEQVDNVPEPAQVPPQQTPPNGFAFNNPDCGNGPECTPNQARIQCKQTHPDKDCTDLFPRDQPVQTTREHPVPGDLQALNSAVQANFAQHSQGKSVFQYYKLINVLWTLAPNPPSPEPGANAQVPLSYGPFISQGNVPVANTTMETYVQGDDCNQCHQYATIAGSPSLASDFSFLFNSAGSASNKSLIKSVKAFETLKDRP

SEQ ID NO: 29 - protein, 578 aa, Pseudomonas putida
MSTPFKQFTSPAGQAPKDYNKLGLEDQLPQFETDWNNNLTGWTESSIIGNPWSGLNDAPRSGYYNPLVEGFGDVTAPAITWAPFPNRLWTFFYNNGAAVIPQLGGKAMTLDQVMALTDHGQITLDNTLYMLYDPNKQGTVLQLPAKRCPSIDWNGKYTAFSPSGPRGWLDEYCEWSIVRDANGNMRKITFTCENPAYFLTMWRIDPNAVLGLYRDYIDPNVQLEDLYLRYTVDCPTGKAGDPVIDPTTGKPAYDTVNKWNAGTACVPGQYGGAMHLTSGPNTLSAEVYLAAAATILRPVSSSQNAQSLICCAQYGQNYRNSDPHIGFMANTTAVNNRLSLTNPIGLYLQQPTDFSAWKGPQGQDVSQYWRITRGTAKSAANGSDQILQAVFEVPESAGFSINDITINNQKVNYVWVIAQQLLVGLSVTVKPLSTAPQAFPCVQDRVAGLQPWPVQLLPLDLFYGQSPTDLPAWLAPGSSNQFVLVVQGADPTTTAQNARVQFSNPGVTAQVTQYLPDASAIPGQTNSGGTQAYILTITVSPSAAPGLVAVRALNPGEDVNVSATDHPWESGLALVPGA

SEQ ID NO: 30 - protein, 534 aa, Pseudomonas putida
MSRSRLSLLSLLCGILLCLSTPQPATAATLSDADTCVQKQLVFNPASGGFLPVNNFNATSQAFMNCFGWQLFIALNWPVNPGWPATASLAGEPDMQSTLAQFGVPSTPGQPMSVAPVWASYKDANDIFLPGAPTPTGWGVQTLVPSDCSTQGSLKTLKVGARKFMNATSEGAINALHGFHLSTGTLASIPDPVMEASGGWLTDQAGKLVFFERKVGKAEFDYIVDKGLYDAANQLKVARNLDGQTPEGLSLPIGEPMRSLPTSPVPQEQLGAIELKAAWRVLTGKPELFGRYLTTVAWLKRPDTLECTQEVVGLVGLHIINKTQASPNFIWTTFEQVDNVPEPAQVPPQQTPPNGFAFNNPDCGNGPECTPNQARIQCKQTHPDKDCTDLFPRDQPVQTTREHPVPGDLQALNSAVQANFAQHSQGKSVFQYYKLVNVLWTLAPNPPSPEPGANAQVPLSYGPFISQGNVPVANTTMETYVQGDNCNQCHQYATIAGSPSLASDFSFLFNSAGSASNKSLIKSVKAFETLKDRP

SEQ ID NO: 31 - protein, 578 aa, Pseudomonas putida
MSTPFKQFTSPAGQAPKDYNKLGLEDQLPQFETDWNNNLTGWTESSIIGNPWSGLNDAPRSGYYNPLVEGFGDVTPPAITWAPFPNRLWTFFYNNGTAVIPQLGGKAMTLDQVMELADHGQISLDNTVYRLYDPNKQGNLLQLPAKRCPSIAWNGPYKDFSPSGPRGWLDEYCEWSIVRDGNGKMRKITFTCENPAYFLTMWRIDPNAVLGLYREYIDPNVQLEDLYLRYTEDGPTGKAGEPVIDPTTGKPAYDTVNKWNAGTVSVPGQYGGAMHLTSGPNTLSAEVYLAAAATILRPVSSSQNAQSLICCAQYGQNYRNSDPHIGFMANSTAVNNRLSLTNPIGLYLQQPTDFSTWKGPQGQDVSQYWHITRGAAKSAANGSDQILQAVFEIPESAGFSINEVTINKQPVNHVWVIAQQLLVGLSVTVKPLAATPASYPCVQDRVAGLQPWPVQLLPLDLFYGNSPTDLPAWLAPGSSNQFVLVVQGADENTTAENARVQFSNPGVTAQVTQYLPDATAIPGQTNTGGTQAYILTITVSPTAAPGLVTVRALNPDEDANVSAADHPWESGLALVPGA

SEQ ID NO: 32 - protein, 534 aa, Pseudomonas putida
MSSLRLSLLSLLSGILLCLSAQQTATAATQSDADSCVQQQLVFNPASGGFLPVNNFNATSQAFMNCFAWQLFIALNWPVNLGWPGTASLAGEPDLNSSLAQFGVPATPGQPMSVAPVWASYKDANDIFLPGAPTPSGWGVQTLVPANCSTQGSLKALKVGARKFMNATSKSAINVLHGFHLSSGTLASSPDPFMEASGGWLTDQSGNLVFFERKVGKAEFDYIVDNGLYDAANQLKVAQNQDGKSPAGLSLPAGEPMRSLPAAPVPQEQLGAIEVKAAWRVLTGKPELFGRYLTTVAWLKRPDTLACTQEVVGLVGLHIINKTQASPNFIWTTFEQVDNVPEPAQAPPQQTPPNGFAFNNPDCGSGPECTPNQARIQCKQHHPDKDCTDRFPRDQPVQTTREHPVPGDLQALNSAVQANFAQHSQGQSVFQYYKLINVLWTLAPNPPSPEPGANAQVPLSYGPFISQGNVPVANTTLETYVQGDDCNQCHQYATIAGSPSLASDFSFLFNSADSASNKSLIKSVKAFETLKDLP

SEQ ID NO: 33 - protein, 578 aa, Pseudomonas monteilii
MSTPFNQFTSPAEQAPKDYNKLGLENQLPQFESDWNNYLTGWTESSIIGNPWSSLYDAPRSGYYNPLVEGFGDVVVPAITWAPFPNRLWTFFYNNGAAVIPQLGGKAMTLQQVMELADYGQITLNDTLYTLYDPDNKGTLLQLPAKRCPSIDWNGKYTAFSPSGPRGWLDEYCEWSIVRDANGNMRKITFTCENPAYYLAMWRIDPNAVLGLYREYIDPNVQLEDLYLRYTVDCPTGKAGDPVIDPTTGLPAYDTVNKWNAGTACVPGQFGGAMHLTSGPNTLSAEVYLAAAATILRPVTSSQNAQSLICCAQYGQNYRNSDPHIGFMANSKAVNNRLSLTNPIGLYLQQPTDFSTWKGPQGQDVSQYWRVTRGTAKSAANGSDQILQAVFEVPESAGFSINEITINKQPVDYVWVIAQQLLVGLSVSALPPATTPPSFPCVQDRVTGLQPWPVQLLPLDLFYGQSPTDLPACLAPGSSNQFVLVVQGADPNTTAQSARVQFSNPGISAQVTQFLPDASAIPGQTNAGGTQAYILTITVSPSAAPGLVTVRALNPGEDGNVSAADHPWESGLALVPGA

SEQ ID NO: 34 - protein, 534 aa, Pseudomonas monteilii
MSRLRLSLLSLLSGMLLCLSTLPAATAAPMTEADACVQQQLVFNPASGGFLPVNNFNASNQAFMNCFAWQLFIALNWPVNPGWPATASLAGEPDMNSTLAQFGVPSDPGQPMSVAPVWASYKDANDIFLPGAPKPSGWGVQTLVPSGCGTQGSLKALKVGARKFMNATSESAINAVHGFHLSSGTLASLPDSIMEASGGWLTDQAGNLVFFERKVGKAEFDYIVGKGLYDAANQLKVAQNADGTTPEGLSLPIGEPMRSLPPSPVPQEQLGAIELKAAWRILTGKPELFGRYLTTVAWLKRPDTLTCTQEVVGLVGLHIINKTQASPNFIWTTFEQVDNVPEPGQVPPQQTPPNGFAFNNPDCGSGPECEPNQPRIQCKQHHPDRDCTDLFPRDQPVQTTREHPVPSDLQALNGAVQATFAQHSQGKSVFQYYKLINVLWTLAPNPPSPEPGANAPVPLSYGAYISQGNVPVANTTLETYVQGDDCNQCHQYATIAGSSSLASDFSFLFNSASSASKHSLIKRVQAFETLKDRR

SEQ ID NO: 35 - protein, 577 aa, Pseudomonas poae
MSTPFTQFTSPAEQAPKDYNKLGLEDQLPAFETDWNNNVTGWTQMSIIGNPWSNLNDAPRSGYYNPLESGYGTLTPKTITWQPFPNRLWTFFYNEGAAVVPQLGGKAMTLDQVMQLTDHGQITLNDTLYSLYPDPKATQLQIPSVLCKSINWNGPYADFSPSGPRGWLDEYCEWSITRDPDGNMRSIMFTSENPAYFLTMWNIDPGAVLGLYQAYVDPQVKLEDLYLRYTADGPTGKAGEPVLDPTTGQPAYDTVNKWNSGTVRIPGVSGGAMHLTSGPNTLSAEIYLAAAATILRPLTSSQNQQSLICCAQYGQNYRNSDPHIGFSANQAAVNNLISLTNPIGLYLQQPKSFSTWKGPQGQDVSSYWRVTRGTAGTGPNNSDQILQAVFEVPASAGFSINEITINGTPIDYVWVIANELNVALSVTPAPLTAQPKECACVAANTTDAQPWPVQLLPIDLFYGQSPSDLPASFAPGSSGQFVLVVQGADPNTTAADARVQFSNPGITAQVTQFLPDASAIPGQTDGGGTQGYIMTITVSSNAAPGLVSVRALNPSEAANPSASEHPWESGLALVPSA

SEQ ID NO: 36 - protein, 529 aa, Pseudomonas poae
MNGWLRPLRRARLRIACAITCTLLPLLAATPANAASDAQSCVSQLVFDPTSGGFLPVNNFGTEQAFLNCFGWQLFIAMNWPVNPGWPANPSLAGEPDTQSSAAQFGVPPTPGQPMSNAPVWASYKDASEIFLPGAAKPSGWGVETLVPSNCTATGNLKAFATGARKFITATSESAINRKHRFHLSSGTQVTLPDSIMEASGGWLTDQSGNLVFFERKVGKAEFDYIVDNGLYDAANQLIVAQNSDNRHPAGLSLPAGKPVRELPAKALPQEELGALELKAAWRVLTNKPDLYGRYLTTVAWLQRPDTLQCTQEVIGLVGLHIINKTQTQPNFIWTTFEQIDNVPDGGAAPPQGYSFNNPECTGDACAPNVARVQCDATHTPPDCTPLDQPVQATRLNATPQDMQALNTAVQQTFAQQTQGQSVFQYYKLVNVLWSKTPNAPNDPGPGPNVKVPLSYGPFVSDQSVVVANTTMETYVQTDNCNDCHQYAAIAGKSGLASDFSFLFGNADSAKNTRLIKRIESFKTLKDNP

SEQ ID NO: 37 - protein, 577 aa, unknown
  Mountain Pine Beetle microbial communities
MSTPFTQFTSPAEQAPKDYNKLGLENQLPTFETNWNNNVTGWTQMSVIGNPWSNLNDAPRSGYYNPLESGYGTQTPVTITWQPFPNRLWTFFYNNGAAVVPQLGGKAMTLDQVMQLTDHGQITLNNTLYSLYPDPKATQLQIPSVLCKSINWNGPYADFSPSGPRGWLDEYCEWSITRDPDGNMRSIMFTSENPAYFLTMWNIDPQAVLGLYKAYVDPQVKIEDLYLRYTANGPTGQAGEPVLDPTTGQPAYDTVNKWNSGTVRIPGVSGGAMHLTSGPNTLSAEIYLAAAATILRPLNSSRNQQSLICCAQYGQNYRNSDPHIGFSANQAAVNNLISLTNPIGLYLQQPKSFSTWKGPQGQDVSSYWRVTRGTAGTGPNNSDQILQAVFEVPQSAGFSINDITINGTPIDYVWVIANELNVALSVTPAPLPAPPKECDCVAANNTDAQPWPVQLLPIDLFYGQSPSDLPASFAPGSSGQFVLVVQGADPNTTAADARVQFSNPGITAQVTQFLPDASAIPGQTDSGGTQGYIMTVTVSSNAAPGLVSVRALNPSEGANPSATQHPWESGLALVPDA

SEQ ID NO: 38 - protein, 529 aa, unknown
  Mountain Pine Beetle microbial communities
MNGWLRPLRRARLRVFCWITCALLPLLAPSPANAATDAQSCVSQLVFDPTSGGFLPVNNFGTEQDFLNCFGWQLFIAMNWPVNPGWPANASLAGEPDTQSSVAQFGVPATPGQPMSNAPVWASYKDASEIFLPGAPKPSGWGLETLVPSNCTASGNLKAYATGARKFITATSESAINRKHRFHLSSGTQVTLPDSIMEASGGWLTDQSGNLVFFERKVGKAEFDYIVDNGLYDAANQLIVAQNSDNRHPAGLSLPAGKLVRELPAQALPQEELGALELKAAWRVLTNKPELYGRYLTTVAWLQRPDTLQCTQEVVGLVGLHIINKTQTQPNFIWTTFEQVDNVPDAGPTPPQGYSFNNPACSGTACTPNVARVQCDATHAPPNCTPLDQPVQATRVNATPQDLQALNTAVQQTFAQKTQGQSVFQYYKLVNVLWSKTPNAPNDPGPGPNVKTPLSYGPFVSDQSVVVANTTMETYVQADNCNDCHQYAAIAGKSGLASDFSFLFGNADSAKNTRLIKRIEGFKTLKDDQ

SEQ ID NO: 39 - protein, 577 aa, Pseudomonas trivialis
MSTPFTQFTSPAEQAPKDYNKLGLEDQLSTFETNWNNNVTGWTQMSVIGNPWSNLNDAPRSGYYNPLESGYGTQTPLTITWQPFPNRLWTFFYNNGAAVVPQLGGTAMTLDQVMQLTDHGQITLNNTLYSLYPDPAATQLQIPKVLCKSINWHGPYADFSPSGPRGWLDEYCEWSITRDPDGNMRSIMFTSENPAYFLTMWNIDPNAVLGLYQAYVDPQVKLEDLYLRYTANGPTGNAGDPVIDETTGRPAYDTVNKWNAGTVRIPGVSGGAMHLTSGPNTLSAEIYLAAAATILRPIQSSGNQQNLICCAQYGQNYRNSDPHIGFSANQAAVKNLISLTNPIGLYLQQPKSFSTWKGPQGQDVSSYWRVTRGTAGTGPNNSDQILQAVFEVPQSAGFSINDITINGTPIDYVWVIANELNVALSVTPAPLTATPKECDCVAANNTDAQPWPVQLLPLDLFYGQSPSDLPASFAPGSSAQFVLVVQGADPNTTVADARVQFSNPGISAQVTQFLPDASAIPGQTDSGGTQGYVMTVNVSGNAAPGLVSVRALNPSEAANPSAAQHPWESGLALVPGA

SEQ ID NO: 40 - protein, 528 aa, Pseudomonas trivialis
MYGWPRPLCRARLNVFSLLAGALLSLVAPPPASASDAQTCVQQLVFDPASGGFLPVNNFGTEQDFLNCFGWQLFIAMNWPVNPGWPADPTLAGEPDTQSSAAQFGVPQTPGKPMSNAPVWASYKDANDIFLPGAPKPTGWGVETLVPSNCTATGNLKALSTGARKFITATSESAINRKHRFHLSSGTQVTLPDSIMEAAGGWLTDQSGNLVFFERKVGKAEFDYIVNNGLYDAANQLIVAQNSDNRHPAGLSLPAGKLVRELPAKALPQEELGALELKAAWRVLTHKPELYARYLTTVAWLQRPDTLQCTQEVVGLVGLHIINKTQTQPNFIWTTFEQVDNVPDGGATPPQGYSFNNPACTGDACTPNVARVQCDATHTPPNCTPFNQPVQATRANATPEDMQALNTAVQQTFAQQTQGQSVFQYYKLVNVLWSKTPNAPNDPGPGPNVKTPLSYGPFVSDQSVAVANTTLETYVQTENCNDCHQYAAIAGGSKLASDFSFLFGSADSAKNTRLIKRIEAFKTLKDDH

SEQ ID NO: 41 - protein, 577 aa, Pseudomonas sp. R81
MSTPFTQFTSPAEQAPKDYNKLGLENQLPTFETDWNNNVTGWTQMSVIGNPWSNLNDAPRSGYYNPLDSGYGTQTPVTITWQPFPNRLWTFFYNDGAAVVPQLGGKAMTLDQVMQLTDHGQITLNNTLYSLYPDPKATQLQIPSVLCKSINWNGPYADFSPSGPRGWLDEYCEWSITRDPDGNMRSIMFTSENPAYFLTMWNIDPQAVLGLYKAYVDPQVKIEDLYLRYTANGPTGKAGEPVLDPTTGQPAYDTVNKWNSGTVRIPGVSGGAMHLTSGPNTLSAEIYLAAAATILRPIKSSANQQSLICCAQYGQNYRNSDPHIGFSANQEAVKALISLTNPIGLYLQQPKSFSTWKGPQGQDVSSYWHVTRGTAGTGPNKSDQILQAVFEVPQSAGFSINEITINGTPIDYVWVIANELSVALSVTPAPLTATPEECDCVAANTTDAQPWPVQLLPIDLFYGQSPSDLPASFAPGSSGQFVLVVQGADPNTTAADARVQFSNPGITAQVTEFLPDASAIPGQTDSGGTQGYIMTVTVSSNAVPGLVSVRALNPSEAANPSATQHPWESGLALVPGV

SEQ ID NO: 42 - protein, 528 aa, Pseudomonas sp. R81
MNKWLRPLRRARLSVLCWIPCALLPLAPAPAIAASDAQSCVSQLVFDPTSGGFLPVNNFGTEQDFLNCFGWQLFIAMNWPVNPGWPADPSLAGEPDTQSTAAQFGVPPTSGQPMGNAPVWASYKDASEIFLPGAPKPSGWGVETLVPSNCTATGNLKAFATGARKFMAATSESAINRKHRFHLSSGTQVTLPDSIMEASGGWLTDQSGNLVFFERKVGKAEFDYIVDNGLYDAANQLIVAQNSDNRHPAGLSLPAGKLVRELPAKALPQEELGALELKAAWRVLTNKPQLYGRYLTTVAWLQRPDTLQCTQEVVGLVGLHIINKTQTQPNFIWTTFEQVDNVPDNGTAAPEGYSFNNPTCTGDACTPNVARVQCDATHTPPDCTPLDQPVQATRVNATPQDLQMLNTAVQQTFAQKTQGQSVFQYYKLVNVLWSKTPNAPNDPGPGPNVKVPLSYGPFVSDQSVVVANTTLETYVQNKNCNDCHQYAAIAGTSQLTSDFSFLFGNADSAKNARLIKRIEAFKTLKDSP

SEQ ID NO: 43 - protein, 577 aa, Pseudomonas libanensis
MSTPFTQFTSPAEQAPKDYNKLGLENQLPTFETDWNNNVTGWTQMSVIGNPWSNLNDAPRSGYYNPIESGYGTQTPVTITWQPFPNRLWTFFYNNGAAVVPQLGGKAMTLDQVMQLTDHGQITLNNTLYSLYPDPKATQLQIPSVLCKSINWNGPYADFSPSGPRGWLDEYCEWSITRDPDGNMRSIMFTSENPAYFLTMWNIDPQAVLGLYKAYVDPQVKIEDLYLRYTANGPTGKAGDPVLDPTTGQPAYDTVNKWNSGTVRIPGVSGGAMHLTSGPNTLSAEIYLAAAATILRPLNSSRNQQSLICCAQYGQNYRNSDPHIGYSANQEAVKALISLTNPIGLYLQQPKSFSTWKGPQGQDVSSYWRITRGTAGTGPNNSDQILQAVFEVPASAGFSINDITINGTPIDYVWVIANELNVALSVTPAPLSGTPKECDCVAANNTDAQPWPVQLLPIDLFYGQSPSDLPASFAPGSSGQFVLVVQGADPNTTAADARVQFSNPGITAQVTQFLPDASAIPGQTDSGGTQGYIMTVTVSSNAAPGLVSVRALNPSEAANPSATQHPWESGLALVPVA

SEQ ID NO: 44 - protein, 528 aa, Pseudomonas libanensis
MNGWLRPLRRARLNVLCWITCALLPFAPAPVSAASDAQSCVSQLVFDPTSGGFLPVNNFGTEQDFLNCFGWQLFIAMNWPVNPGWPANPSLAGEPDTQSTAAQFGVPPTPGQPMSNAPVWASYKDASEIFLPGAPKPSGWGVETRVPSNCTATGNLKAFSTGARKFITATSESAINRKHRFHLSSGTQVTLPDSIMEASGGWLTDQSGNLVFFERKVGKAEFDYIVDNGLYDAANQLIVAQNSDNRHPAGLSLPAGKLVRELPAQALPQEELGALELKAAWRVLTNKPELYGRYLTTVAWLQRPDTLQCTQEVVGLVGLHIINKTQTQPNFIWTTFEQVDNVPDGGATPPGGYSFNNPACTGDTCTPNVARVQCDATHTPPNCTPLDQPVQATRVNATPQDMQALNTAVQQTFAQKTQGQSVFQYYKLVNVLWSKTPNAPNDPGPGPNVKVPLSYGPFVSDQSVVVANTTMETYVQSDNCNDCHQYATIAGGSKLASDFSFLFGNADSAKNTRLIKRIEAFKTLKDNP

SEQ ID NO: 45 - protein, 576 aa, Pseudomonas asplenii
MSIPFTRFSPPANQAQKDYQKLGLEQQQAQFDTDWSNNLAGWTEAAIIGNPWTGLNDAPRTGYFNPLISGFGDAPPAVIDWTPFPNRLITYLTQADSAKNPQLGGKPLTMDQVMQLADTGEIDINGTPLKLYDPLGSNTLQLPSIRCPQIDWTGPYAAFTPSGPRGWLDEYCEWSITLDANGNMRSVMFTCENPAYYLTMWRIDPKAVLGLYRMYIDSAVQLEDLYLRYPVDQPTGKQGEPVIDPTTGLPAYDVTNKWNSGTARKPGLFGGALHLTSAPNTLSAEIYLAGASTIQRSDKSSETPQTLICCAKYGRNYRNSDPHIGYVANGIAYGNRISLTDPVGLYLQQPKNFSKWKDPQGNSVSQYWQITRGTAGTGPLGSDQILHAVFEVPEQAGFSINDITIDGQKITHVGVIANQMKVALSASPLDAIKPVIQPCVTDRSTGLQPCPVQLLPLSLFYGLSPSDLPAWLAPSSSNQFILLVQGSDAATTAANARIQFSNPGVKAQVIEFQTNATPIAGTTDNSGTQGYIITITVAANAAPGLVQLRVLNPDEPVNPSDTDHPWASSLAIVPAL

SEQ ID NO: 46 - protein, 518 aa, Pseudomonas asplenii
MFSLDCSRGNGRFCLPPLLLIIWLLGSLVARNAYALSDPETPAQCVQQLVFDPTNGSFLTSDTPFVAQQATFNCYAWQMFIAMNWPVNPGWPTHPELAGEPDTKSPAAQFGVPTIADQPMSVAPVWASYKDANDIFLHGAAIPTAWGMQPPEPVGCQTKPSLLSLRVGARKFMTATSESAVNAKHRFHLSSSTLVTASDPTLEATGGWLTDQAGKLVYFERKVGKAEFDYIVSNELYDAANQLQVAKNQGLSLPAGAHFRSPPTSPIAQEKLGAFELKAAWRILTDKPQLYDRYLTTVTWLKHPETGQCTQEVVGLVGLHIIHKTASQPDFIWTTFEHVDNVPDGGSTPTAGYTFNNPKCTGPDCTPNQRRITCTALGCKDNYPRNEPVQVTREDSVPSTINDLNTVVQQAISTKTAGKSVFQYYKLVNVLWDASPHIPDPEPGANATVPLVYGSFSSDGNNTPVSNTTMETYIQNRSCDFCHRNAKVAGSKSLTSDFSFLFESADSSKIPTLIKKMP

SEQ ID NO: 47 - protein, 580 aa, Thalassospira xiamenensis
MSTPFARFTSPAHQAPKDYKKLGMENELSAFETDWNNNVAGWTEMAIIGDPWSNLNDAPRADYYNPLTEGFGEAGDAVISWTPFPNRLIAFLTPPEASNNPQLHRPLTMDEVMSLADSGEITVDGTLYKLYDPSGSAPILKIPAKRCPEIDWTGEYVDFSPSGPRGWLDEYCEWSITYDASGSKMQSVMFTCENPAYYLTMWRINPEAVLGLYQMYVDPAVKLEDLYLRYTVDQPTGKKGDPVMDPTTGRPAYDVTNKWNRGTVRVPGQSGGALHLTSGPNTLSAEIYLAAAATIQRPDLSSRDPQSLICCAQYGQNYRNSDPHIGFIANRAAARYRISLTDPVGLYIQQPQNLSNWKGPNGEDISQYWKITRGTAGTGPNNSDQILHAVFDIPPSAGFTINDCTINGQKIAHIGDIANQMKIALSATQMTPNQPLQSPMKCVSSRSSGSMQPWPVQFVPIDLFYGESPTDLPALMVPGTVNSFVLIVQGADKNTTIDNARIEFSNPGIKAKVTKFLPDASAIPGQTDGGGTQGFIMDVAVSSSAKPGSVSLRVLNPNEPANPSDADHPWESGLAVIPSH

SEQ ID NO: 48 - protein, 539 aa, Thalassospira xiamenensis
MNRLHLGAGCVIAGFCILAIAGLLWVIDVPAGRADEINISRVTEIAQSAQQCPDQLVFDPTSGSFMTSDNLFLPTQQGNNCYAWQMFIAMNWPVSSSWPGTPSAAGEPDQNVSVENWGVPENPTSPLTSVPVWGSFKDAQAIFLPDAAKPTDWGVPQAVPSGCKSDKMLLGYPAGSAKILTTLSKNAVNTAHRFHLSSGTRDTQSDEIMEATGGWLTDQNGNLVFFERKVGKAEFDYIMNNALYDAAYQMRVATNADGRHPAGLSLPSGKFLRVPPTEPQGQDALGAFEIKAAWRVLTGQSDIYDRYLTSVAWLKRPDTGECSQEVVGLVGLHIIHKTDTFPDLIWATFEQVDNVPDGQATLPPGGYSFNNPNCTGPDCKPNQPRIDCNDQNQCKDLYPRDQPVQVTREQALTSEMDTLNAGVAQKIASQTGGKSVFQYYKLVNVLWDGSPSPPVMEPGANASIPLRYGTFESEGNLKVANTTMETYIQDQSCDFCHANATIAGSDTLASDFSFIFRDAGSAKNPSLVEEVKQFMEQAQ

SEQ ID NO: 49 - protein, 577 aa, Paracoccus denitrificans
MTIFTEFSTPAQQGPKDYQLLGLPAADLAAFEADWSANIAGWTQMSIIGNPWSNLNDTPRDNYYDPLVEGMGEATAAVISWPPFPNRLIQFLTNPGIVKGGQLTAPLSQDAVQELADSGRITQGGTSFVLFDPEPGQVLLKIPADRCPAIDWDGKYVDFSPSGPRGWQDEYCEWSILRNAQGKMQSIAFTCENPAYYLTMWRQNPKAVLGIYQRYIDPAVQLEDLFLRYEYDQPTGKKGDPVLDPTTGNPAYDPTNKWNRGPARVPGSFGGAMHLTSPPNTLSAEIYLAAAATIQRPSSVNGNPQSLICCAQYGQNFRNSDPNIGYGANVAARTARLTLTDPVGLYIQQPQNFQGWSGPNGEDVSGYWQILRGTAGTGPNGSDQILHAVFAIPESAGYSIEDCTIYGLPISHVGVILDQMKVALAVTPNNAAPDTTAFACVTDRTDGTQPWPVQMVPESLFYGESPSDLPALLRPGSKFRFVLIVQGADENTTPATARVEFSDPNITVTVEQFLKNASAVPGQTNGGGTQGYVMDIAVGANAQPGPVSVRALNPSEGPAPTPEQHPWEAGLAVISSR

SEQ ID NO: 50 - protein, 502 aa, Paracoccus denitrificans
MRTGQILIALVAGVMLAFAASGGKAQTACSAMLITDPTSADFLTGDTPFGHTQDGMNCYGWQMFLSLNWPADPGWPQTPAMAGEPDRSATIADFGLPGPAGQPMQRPTVWQSFMPAPEIFKPFAAMPTGWGETSPPPASCGSASLAASAGSIRMLNAVSKSAVSPRHGFNLDTGTMSSISDEIEEATGGWLTDQKGKLVFFERMIGKAEYDYIVAKGLYDAANQLKVATNADGATPEGLSLPKGTPPGSAVQNQDELGAFELKAAWRNLTGLDDLYGRYLTSTVYLLYPDGSCEKAVVGLVGLHIIHKTASMPDFVWSTFEQIDNVPGASAPEVDFSFNNPASNAKPNQMPHCVNGVCDYSLPIQVTREVAIPAGVAQTNRDVQQLLADRTGGKSVFQYYQLVNVLWDGAPTPPSPEPGANAQVPLVYGTFQTDGSVPVANTTMETYAQQFTPGLGPSCTACHKGATIANSATLASDFSFLFSTASSATKLPGLFISRDFVP

SEQ ID NO: 51 - protein, 580 aa, Cellvibrio japonicus
MSAFTFSTPALIQDFSDNPSLQQQLNQNWDLAIDAYTQAALVSNPWTVDYQAPCDWYVNPKQADITAANPVEPIFWTAFPNRLKIYFSAAEKSPYQMANAQVFALADFGNVPQSKAFPTGLPFIIPSKRCPNLNWQQSIAEWVQYDPKGPRGWLDEYCEWSVTRNADGKITKIAFTCENPEYWFTLWQVSPEKVLALYQQLVSPNVVLEDLQLPSADGKGFVIDPTTGRPAYNPLNKWNSGTVATETYGGAVHLTSPPNTIGAEIMLAAQATLLRDLPPDQYNMQRMVCAGAYGRAYRNSDPHIGLQANQLVKNLGVKITLTNPVGLYLQRPDFSSYKTPDGKDAGQFYKVIRGRTAQQAGTTYDQILHAEFSVPEELGYTVSDILIGNAVPGSSQVPVPILYAGQIAETFHVCLAGTAIAPATGEPSQAFLPPVTDKTGNTNGQVSMLLANPVLLAMQAVNPFPPFVQLPVQIAQGQTLTNMALQVSYANDNFQEAQIAFWDAQGNSEPGISVTVTAIETADGTPAGKSAGGDGLFNYIISISVAPGVSPGFKGVTVRNPACDMPLPLPGVLFVTAKGN

SEQ ID NO: 52 - protein, 506 aa, Cellvibrio japonicus
MKHTLLIGVTTGLLVAACQQPVQESSAAVDAPAVSTVSSSSAPISFPCLNKPAVNYNTPGDTPITSQDGVNCFAWQTFIGLNWPVDASHPGEPDKTASASVFGEPGLHQTSVWETYANSKSVFRANAQPPLPWGHTPDVPSSCQKISQTLGLRVMQASRMPGSFNMSKEASQAFPGNNPNWLADKSGNLVYYEILIGKDEYDYINNNGLYNANTQAAHIQQNKNIAMPLGHDKVLGGLEIKAAWLSVSDPQNPKWKNYKLSTSVIYDPVSKDCHASTIALVGMHIIRKTASQPQWIWATFEHKDNAPDTASIKSDGTVDGDYTFYSNSCTVKPVPAGCKAKVENGTSVTQTSCHVNVSPAYYLDTSGNCPAYPIQVSRDFAIKDSTDNHVASLNRAVQQLIASSNADSVYTHYQLVNVLWSSAAVNDNAPPGNPPLTPLSISGETPSLNTVPVANTMLETYAQGFNCLSCHAYASVARDARAQLGGKAYATDYSFIFSFATSPAAK

SEQ ID NO: 53 - protein, 256 aa, Pseudomonas brenneri
MGSITDHNQLLAWVASLDIPEASGVKTRSRNVVARANAEDEGAAVVRGSITSFVTGLSQQARDDVQNSTLLMQLAADKKFNPEKQREEWFKFYTDGLANLGWGRVSSYYQSYQPRNTNVTMDQVVLEVIAAVVGADSAVYKVTEKTFSSLQDNPKNQAPLKLFDSSSTRDSVGTFQILPVMQDRDGNVVMVLTTVNASTTVQRGSFLFWSWSKTTAWMYRAAQQTVLNESVYATVRQSVIKKLGKNAEEFIDDLEI

SEQ ID NO: 54 - protein, 260 aa, Pseudomonas brenneri
MKLSADEVYVISGNLLSATPSLTDPTVLEDIANSNLLCQLAADKNQGTRFIDPAAWLDFYRSSLGRLFWRISNSGTVSYAIPQLVHKITVKEVLEKTFYKTLDRPQRIRVEESIELLGEQSADSPSATLYSLKTQVNFNETTSSPGLLPHSISSVNLQLSVVHSETCISVCSVYFKTSTRIGDDVFNQKFPVKELLGNVSVSTFEAKLLESSYAGIRQSIIDKLGEDNIRENILLVPAVSPSLSNTRHAGALQFVQELDI

SEQ ID NO: 55 - protein, 260 aa, Pseudomonas gessardii
MKLSTDEVYVISGNLLSATPSLTDPAVLEDIANSNLLCQLAADKNQGTRFIDPAAWLDFYRNSLGKLFWRISNSGTVSYAIPQLVHKITVKEVLEKTFYKNLDRPQRIRVEDSIELLGEQSVDSPSATLYSLKTQVNFNETTSSPGLLPHSVSSVNLQLSVVHSETCISVCSVYFKTSTRIGDDVFNQKFPVKELLGNVSVSTFEAKLLESSYASIRQSIIDKLGEDNIRENILLVPAVSPSLSNSRHAGARQFVQELDI

SEQ ID NO: 56 - protein, 260 aa, Pseudomonas fluorescens
MGSITDHGKLLAWVESLDVPKSTGNANLKRASAVLRSAAQNSDEDGAAVVRGSITSFVTGLTPQARDDVQNSTLLMQLAADKKYNPDTQREEWFKFYTDGLANLGWGRVSSAYQKYKPTNTNATMDQVVLEIISSVVSPESALYKVTEKTFLALKNNPNNKDALKLFDVSSTRNDLGTFQILPVMQDKDGNVVTVLTCINAHTEVQKGSFLFWHWSSTSAEMYRAAQQVVLNQNVYATVRQSVLKKLGKNAEDFIDGLDI

SEQ ID NO: 57 - protein, 259 aa, Pseudomonas fluorescens
MSFTAPEVHVVSGNLISAMPSVNSPQVLEDILESNLLCQMAADKSLGSRFNNPAAWLDFYRNSLGKLFWKITNFNTVSYPVPSPTRSVSVMGILEHTFFKVLAQPLRHQIEADIELLMELPLTSPASQLYTSKTHVEMSTRARSSFDGRSESVISLQISVVHSGSLISVCSVYFKTAEPVAADVFSQKFKVRDLLGNISVNSFEADLLEGSYEGVRQQIKTKLGEANIRENILLIADNPIPVDELPHANAHQFLKGLDI

SEQ ID NO: 58 - protein, 255 aa, Alcaligenes faecalis
MSTITDHKQVLAWINALDIPDAPAGGNRVAARATSSADEDGAVVAKASIPCFVSGLTEQSRADVQNSTLLMQLAADKKYPNENDREKWFKFYSDGLTNLGWGSSSSFFERFQPKNTDVTMDQVVLEVILTVVNNVNNPLYKIAQETFGALNKPANQKPMKLFDHSSTKEDRGKFQILPAGQDQHGTVSMVLTAINARTDIQSGSFLFWKWSKSTAWLYRAANLIVLNESVYSKVRQAVIDKLGDNAVNFVLDLDI

SEQ ID NO: 59 - protein, 268 aa, Alcaligenes faecalis
MAFSTEQTYVVSGNLISATTEDTNTLSYEDFIHSNLLAQMGADKKLGSRFVDPAGWLSFFKNTVGNLFWNLSEQGTSTLKISAGTASITVQQILEQSFFKRLNQAQIDSATASVDLFSQLSEDDPAFILYNAKSHAQISTATKVIKPPQKETYSVNLQISIAHTGSEIALCNIFFQTSQAVSDELFTQKFAIKDLIGNINVFYLKALLSETNYGHIRQQVIEKLGENINTNIVLVADNSDKPSPPFSHRGAQFHTQPENLIQQRTGPP

SEQ ID NO: 60 - protein, 255 aa, Alcaligenes faecalis
MSTITDHKQVLAWINALDIPDAPAGGNRVAARASSSADEDGAVVAKASIPCFVSGLTEQSRADVQNSTLLMQLAADKKYPDENDREKWFKFYSDGLTNLGWGSSSSFFERFQPKNTDVTMDQVVLEVILTVVNNVNNPLYKIAQETFGALNKPANQKPMKLFDHSSTKEDRGKFQILPAGQDQHGTVSMVLTAINARTDIQSGSFLFWKWSKSTAWLYRAANLIVLNESVYSKVRQAVIDKLGDNAVNFVLDLDI

SEQ ID NO: 61 - protein, 259 aa, Alcaligenes faecalis
MAFSTEQTYVVSGNLISATTKDTNTLSYEDFIHSNLLAQMGADKKLGSRFVDPAGWLSFFKNTVGNLFWNLSEQGTSTLKISAGTASITVLQILEQSFFKRLNQAQIDSATASIDLFDQLPEDDPAFILYNVKSHAQISAAAKAIKPPQKATYSVNLQISIAHTGSEIALCNVFFQTSQAVSDELFTQKFAIKDLIGNINIFYLKAQLSETNYGQIRQQVIEKLGENINTNILLVADNSETPSPPSPAEARSFIRSLKI

SEQ ID NO: 62 - protein, 255 aa, Alcaligenes sp. HPC1271
MSTITDHKQVLAWINALDIPDAPAGGNRVTARATSSADEDGAVVAKASIPCFVSGLTEQSRADVQNSTLLMQLAADKKYPNENDREKWFKFYSDGLTNLGWGSSSSFFERFQPKNTDVTMDQVVLEVILTVVNNVNNPLYKIAQETFGALNKPANQKPMKLFDHSSTKEDRGKFQILPAGQDQHGTVSMVLTAINARTDIQSGSFLFWKWSKSTAWLYRAANLIVLNESVYSKVRQAVIDKLGDNAVNFVLDLDI

SEQ ID NO: 63 - protein, 259 aa, Alcaligenes sp. HPC1271
MAFSTEQTYVVSGNLISATTEDTNTLSYEDFIHSNLLAQMGADKKLGSRFVDPAGWLSFFKNTVGNLFWNLSEQGTSTLKISAGTASITVLQILEQSFFKRLNQAQIDSATASVDLFSQLSEDDPAFILYNAKSHAQISAATKVIKPPQKETYSVNLQISIAHTGSEIALCNIFFQTSQAVSDELFTQKFAIKNLIGNINVFYLKALLSETNYGHIRQQVIEKLGENINTNIVLVADNSDKPSPPSPTEARSFIRSLKI

SEQ ID NO: 64 - protein, 260 aa, Enterobacter sp.
MNTNALDFVLKTPIETTADLAPLLERLKGVPDHGQSKRKTMLTDNKVSAQVNAGSLISFTERLDGQNKQDVQNSTLFAQLAADKHCNRYTAPMDWYRFYVNVLGQIGWNQPAFAFDTYTSGASTVKLDEAVLGIIAQIATVGEVALVAAAMKALSSLSDTSKQMLIWDAKSNSENTGNFQIFPADLLPNGDVVMMLDGMQFDAKRNEGRFLWVTWQSTSIKIQRAANKFVLNEGVYKGVRQAVIDKLGDRAIDMIANIEI

SEQ ID NO: 65 - protein, 258 aa, Pseudomonas fluorescens
MSFEVCDSSVAACVARLESYDIYPDISPRSLYSGDIEPPAKGSVVGEGILAFAGGLSSQHQEDAQHAFLFASLVANRQYPLESQGREWYYKFVEVMTNAGWVATQRFYDDLSIAGNTVRMDKLVLDILASVVSGIALGSATSALLLRVADSAITALQKKEKTLTLFERNLLEHGVGGMAAGTCVEIDGEVSMLLGTVRFIRRNSATQVLFADWNSREVKLYKGESVFRKVPSIVERTRGIIIGRLGNHAVSKIEEYEI

SEQ ID NO: 66 - protein, 242 aa, Pseudomonas fluorescens
MDKAYSIFVNAAAIVLVSSTVRGTGVEDLMNSVLLAQLVANKNLQRIPSADWYASYMDVLSVAWVAGAKRRKDLLPKQDAASSPVEWVTAIPLDDRPDQQQQIMAVLDRVAALPGSLPALSILRKHMQKPNEPEPTQSPSASSPVRLLVIVAHSPVSMTGICLQFNTGKAINANPWGQCFDGKDIDGCVSARYLRMQLSETLFAPAREVIARKVGTVVGDNVVDITGAIEDSVVRPAEEVGR

SEQ ID NO: 67 - protein, 258 aa, Pseudomonas brassicacearum
MSFEMCDSAVAACVARLESYDIYPDVSPRSLYVDDVEPPAKGSVVGEGILAFAGGLSPQHQEDAQHAFLFASLVANRQYPLESQGREWYYKFVEVMTNAGWVATQRFYDDLSVGGNTVRMDKLVLDILASVVSGIALGSATSALLLRVVDSAITALQKKEETLTLFERNLLEHGVGGMAAGTCVEIDGEVSMMLGTVRFIRRNSATQVLFADWNSREVKLYKGESVFRKVPSVVERTRDIIIGRLGNHAVSKIEEYEI

SEQ ID NO: 68 - protein, 242 aa, Pseudomonas brassicacearum
MDKEYSVFVNAAAIVLAPCALRRTEVDDLMNSVLLAQLVADKSLLRAPAVDWYATYLEVLSVAWISAAKRRKDLQPQKEDTHSPLEWVAAIPLDDQVDQQQRIMAVMERIAALPGSLPAMGIVRKHVQKQYEPDAAQSPSSSSPVRLLVIVAQSPVSMAGVYLQFNTAKVIEANPWRQCFDGKDIDGCVTARYFRTQLSETLFAPAREVIARKVAAAVGDNIVDITKAIDDSGVLPAEEVCR

SEQ ID NO: 69 - protein, 263 aa, unknown
  Switchgrass rhizosphere microbial community from Michigan
MSVNMIDSATVAACVRRLESYEIDEVPVVRSRAFAASGIVVEEPSKGAVVGEGILSFVGNLSEQNQVDAMHAFLFASLVANKQFPYEYQGKEWYYKFVEVMTSAGWLTSQKYYNDIEISGNTVRMDQLVLEILGSVVAGLAIPGTASALMLKVAGDAITALKKKETALTLYERNLLEHGVGGMAAGTCTEVNGEVTLALGTVRFIRKNTATQVLFMDWDSRDVQLYKGESVFRKVPYIADQTRDLIRTKLGTNAVSKIEGYEI

SEQ ID NO: 70 - protein, 242 aa, unknown
  Switchgrass rhizosphere microbial community from Michigan
MAREYSVFVNAAAIVLLPSNPVESATNDLMNSVLLAQLVANKRAEATSAVDWYETYVGVLGDFWLTRARSRQDIQPGKDDTASPLEWIAAVLASSTEDEARLVTALLKGIARLSDSLPAMSLLRKHVQKESDDEPAEISLQSKPVRLVVIVAQDNASMTSVCLQFKTRQMLDPNPWGQRFHVEDMEGCVSAHFFHAHLSETLYAPAREAVARKVEGVLSDNIVDITEAIDALAFLPTEEAGT

SEQ ID NO: 71 - protein, 261 aa, unknown
  Miscanthus rhizosphere microbial communities from Kellogg
MNVHDVEDCTVAECIHRLESYELDGAEVMRPRSFSVPVVNEPGKGSIVGEGILSFTGNLSEQNREDVQHAFLFASLVANKKYPYEYQGKEWYYQFLEVMTHAGWLPTSKYYNDMNISGNTVRMDQLVLEILGSVVAGLAVPGSASVLMLKVAGDAITALKKRETALTLYERNMLEHGVGGMAAGTCTEVNGEVTMALGTVRFIRKNTAKQVLFMDWDSREVKLYRGDSVFRKVPYIVEQTRDTIRAKLGLNAKPKIEDYDI

SEQ ID NO: 72 - protein, 240 aa, unknown
  Miscanthus rhizosphere microbial communities from Kellogg
MSYEYSVLIVGACVVIIPAADGAAQYTDLVNSVLLAQLIANKKIEKAPEIDWYNAYVEFLDDYWLRRTRARQDWSIAQDRVESVSDWVIAAISQDAVDKGSATAATLQRLARLSGNEPAMGLLRGHMQKISTDESGDVLAPAKAVRLLVVIAQTPTSVASVYIELKTRQIISANPLAQRHLAEDVQGSVCMRYAAANLSETLYSPVRDAIALKVRDKYQDNVAMLTLSDDASAMEICAVD

SEQ ID NO: 73 - protein, 555 aa, Pseudomonas rhodesiae
MAKLTQFSTPADIQDFSDSPAQQERMNAAWSGNINRWVNAALVGDVWDLINYGPRPAFYNPLDTDTPSTSVNAPITWNAFPGRIPALFPNQSANWLQWADQGVPANVTTNLCTQQSVPPAPYSPTGPRGWQDEYCEWSVTRNAAGQITSVMFTCENPEYWMTLWQVDPGKVLQRYQQLINPAVQLADLSLKDAQGQTVIDPVTGAPCYNPLNKWNSGTQTLPGSGGAMHLTSSPNTLGAEYDLAAAATMPRELNNEPVTSASQLVCYARYGRIGRHSDPTIGQNVNQYVNYTSGLTEVRATLTNPPGLYIQTPDFSGYTTPDGSPAAACWTINRGHLAQTSDDIDRILHATFSVPAGKNFTVSDISINGAKIQYASQIAGTITMGLMATVFGNSGVTQQPVAGTLDSDNPSPSVSALQPLSVFNAYRAQELASNEQALSIPILALAIRPGQQVDNIALLLNTSQTPNGASFSVVEGGVSISITGTQDLPGLDMSLYLVSISADANAAPGDRTVLASVPGMASTQQAAIGLLTVGGPTLVTSQTGPSKPNFRRGRG

SEQ ID NO: 74 - protein, 451 aa, Pseudomonas rhodesiae
MRRRPTVLLGLALLLGLPATQAMGAPLCGSPFVPSPTLQPTLAPPNFSASDSAVDCFMWQTMVYLNWPATPGQRGVPNAAASLGSPGPSVWQTYKDYNELYLPNGQQPPAWNDNFLSVQRLQTRGVARALPSIRLLNSTSKVFRAANANESPALREIEQVGGGVLYDQAGSPVYYEMLVNEVNFDFIYNNQLYNPAQQNLYAKQKGIVLPNNSIEIKAAWKVLSDPDNPQRFLTAQALLPGSSTPVTVGLVGLHVFQMPSSAFNQGFWATFQQLDNAPTVAGATPGAHYSFNNPQCAPAQCPPNDKTSNPTQVVQNFPPTPEAQNINHYMQNLIAQQAPGSALQYYQLVDVQWPTSPQAIGQPGATAPAPSGTPNHDTLINPVLETFLQANHKSCLGCHVYASVAADGSNPPTHYQASFSFLLGHAKSPALGSNLKSLAQQIEDASLSLQH

SEQ ID NO: 75 - protein, 555 aa, Pseudomonas orientalis
MAKLTQFSTPADIQDFSDSPAQQERMNAAWSGNINRWVNAALVGDVWDLINYGPRPAFYNPLDTDTPSTSVNAPITWNAFPGRIPALFPNQSANWLQWADQGVPANVTTNLCTQQSIPAAPYSPTGPRGWQDEYCEWSVTRNAAGQITSVMFTCENPEYWMTLWQVDPGKVLQRYQQLINPAVQLADLSLKDAQGQTVIDPVTGAPCYNPLNKWNSGTQTLPGSGGAMHLTSSPNTLGAEYDLAAAATMPRELNNEPVTSASQLVCYARYGRIGRHSDPTIGQNVNQYVNYTSGLTEVRATLTNPPGLYIQTPDFSGYTTPDGSPAAACWTINRGHLAQTSDDIDRILHATFSVPAGKNFTVSDISINGAKIQYASQIAGTITMGLMATVFGNSGVTQQPVAGTLDSDNPSPSVSALQPLSVFNAYRAQELASNEQALSIPILALAIRPGQQVDNIALLLNTSQTPNGASFSVVEGGVSISITGTQDLPGLDMSLYLVSISADANAAPGDRTVLASVPGMASTQQAAIGLLTVGGPTLVTSQTGPSKPNFRRGRG

SEQ ID NO: 76 - protein, 451 aa, Pseudomonas orientalis
MRRRPTVLLGLALLLGLPATQAMGAPLCGSPFVPSPTLQPTLANPNFSASDSAVDCFMWQTMVYLNWPATPGQRGVPNAAASLGSPGPSVWQTYKDYNELYLPNGQQPPAWNDNFLSVQRLQTRGVARALPSIRLLNSTSKVFRAANANESPALREIEQVGGGVLYDQAGSPVYYEMLVNEVNFDFIYNNQLYNPAQQNLYAKQKGIVLPNNSIEIKAAWKVLSAPDNPQRFLTAQALLPGSSTPVTVGLVGLHVFQMPSSAFNQGFWATFQQLDNAPTVAGASPGAHYSFNNPQCAPAQCPPNDKTSNPTQVVQNFPPTPEAQNINQYMQNLIAQQAPGSALQYYQLVDVQWPTSPQAIGQPGATAPAPSGTPNHDTLINPVLETFLQTNHTSCLGCHVYASVAADGSKPATDYQASFSFLLGHAKSPALGSNLKSLAQQIEDASLSLQH

SEQ ID NO: 77 - protein, 556 aa, Pseudomonas sp. PKRS11
MAKLAQFSPPARIQDFSNDPAQQECLNAAWSGNINRWVNAALLGDVWDRINYGPRPAFYNPLVTDTPDTAGNVPITWNAFPGRLQALFPNQGASWQQWADQGVPDKVTTDLCSGKPIDPAPYSPTGPRGWQDEYCEWSVTRNGAGQITSVMFTCENPEYWMTLWQVDPGKVLQIYQQVINPAVQLSDLCLKDSHGQTVNDPLTGQPCYNPLNKWNSGTRTLANSGGAMHLTSSPNTLGAEYDLAAAATMPREKDHDPVTSAAALVCFARYGRIGRHSDPTIGQNVNQYANYTPTLPHPQATLADPPGLYMQTPQFSDYVTPDNTPAQTFWTVVRGSLKDPNTSEDIDRILHATFSVPPELGYTVSDIKIGNQPIRYGSQIAATITMALLATAFPNSGVVQTPVGATLDNSNPSPSVSALQALAVFTAYRAQELASNEQPLSIPVLALAVSPGQQVSNIALLLNTSDTPDGAVFTVPEGGVSIRIDGTQALPNAELSLYQVTLCVDANAAIGDRSILASVPSMPATQQAAIGLLTVVAPPQVRLAGGPRKPHARHSR

SEQ ID NO: 78 - protein, 448 aa, Pseudomonas sp. PKRS11
MRAILALLLYAGLSLAPVAARAAGNPCGSPFSPEPVIQPVLANPQISNLDPSVDCFMWQTMVYLNWPAQAGQRGLPNTDAHLGDPGPTVWQTFKDFNELYLPGGQRPAPWNDNFLTMQRLELRGVERPRPSIRLLNSTSKVFRNADASEQKALDEFKQVGGGVLYDQNGQPVYYEMLINQINFDYIYSNQLYNAAQQNLHAAKQGIVLPSNSIELKAAWKVLSPQEAAPPLRFLTAQALLPGSQVPVTVGLVGLHVFQMPSKDFAQGFWATFSQVDNAPTLNTPGQAHYSFNNPQCSQCPVNDLGSKPTQVVQVQANAVYAQAVNQYMQALIQQQAPNSALQYYQLINVQWPNSSVPIGQPGQPTPAPTGSPSTDTLVNPVLETFMQVSNMSCLGCHKSASVADNGTQPPSGYQASYSFLLGHAQNPPPQGSLKSLARQVEEASTARQ

SEQ ID NO: 79 - protein, 96 aa, Pseudomonas Antarctica
MKLSNVLLLSIVFAWQGMAFADTQKSNAETLLSNDKPPLTQAAQEKEQENVEADRNECWSAKNCSGKILNNKDAHNCKLSGGKSWRSKTTGQCTNL

SEQ ID NO: 80 - protein, 96 aa, Pseudomonas orientalis
MKMSSVLLMSIAFVCQGMVFADTQKSNTETLFSNDKPPLIQTAQEQEQKEVEVDRNQCWSAKNCSGKILNNKDAHNCKLSGGKSWRSKTTGQCTNL

SEQ ID NO: 81 - protein, 95 aa, Enterobacter asburiae
MKTLVIAILTAVLCQGMAMADTQKPATGALPANEKPPLVQPADEHKTSEANANRNECWSAKNCTGKILNNKDAHNCKNSGGKSWRSKTTGQCTNL

SEQ ID NO: 82 - protein, 95 aa, Enterobacter sp.
MKTLVIAILTAVLCQGMAMAETQQPASGALPANEKPPLVLTADEKKASEANADRNECWSARNCSGKILNNKDAHNCKNSGGKSWRGKNSSQCTNL

SEQ ID NO: 83 - protein, 105 aa, Acidovorax avenae
MKKLLLIASLLVSISGANVFAQAPSSGDAPAAVAGKQDGASHKDTEQAANVECDVNATVQQCCSAAKCQGKVLSNRDAHNCKDKSKGKSWHAAAQGGQPAACQRM

SEQ ID NO: 84 - protein, 94 aa, Serratia plymuthica
MQCNGAILKLLCAQRKDQFMNLRIRTHAMKNLSILVVLSSCLLLPLTASAAAGTCYSAKNCSGKVLSHRDAHNCKVKDKGKSWRSDITNQCTNL

SEQ ID NO: 85 - protein, 93 aa, Serratia liquefaciens
MREEAILKLLCAQRKDQFMNSRIRTHAMKNLSILVVLSSCLLLPLTASAASGKCYSAKNCSGKVLSKRDAHNCKVKDRGKSWLSDVTGKCTNL

SEQ ID NO: 86 - protein, 78 aa, Serratia sp.
MKLKYERIRIYVMKSLSIVITLASCLLLPLTASAAAGTCYSAKNCSGKVLSHRDAHNCKVKDKGKSWRSDITGQCTNL

SEQ ID NO: 87 - protein, 75 aa, Serratia sp.
MNSRIRTYAMKNLSILVVLSSCLLLPLTASAAAGTCYSAKNCSGKVLSHRDAHNCKVKDKGKSWRSDITGKCTNL

SEQ ID NO: 88 - protein, 89 aa, Pseudomonas chlororaphis
MSAQENFVGGWTPYHKLTPKDQEVFKEALAGFVGVQYTPELVSTQVVNGTNYRYQSKATLPGSSESWQAVVEIYAPIKGKPHITQIHRI

SEQ ID NO: 89 - protein, 89 aa, Pseudomonas chlororaphis
MSAQENFVGGWTPYHKLTPKDQEVFKEALAGFVGVHYTPEQVSTQVVNGTNYRYLSKATVPGSSDSWQAVVEIYAPIKGKPHITQIHRI

SEQ ID NO: 90 - protein, 89 aa, Pseudomonas brassicacearum
MSAQENFVGGWTPYHELTPKDREVFKEALAGFVGVQYTPEKVSTQVVNGTNYRYLSKATVPGSSDSWQAVVEIYAPIKGKPHITQIHRI

SEQ ID NO: 91 - protein, 89 aa, Pseudomonas chlororaphis
MSAQENFVGGWTPYHELTPKDREVFKEALAGFVGVHYTPEKVSTQVVNGTNYRYLSKATVPGSSDSWQAVVEIYAPIKGKPHITQIHRI

SEQ ID NO: 92 - protein, 89 aa, Pseudomonas chlororaphis
MSAQEHFVGGWTPYHELTPKDKEVFKEALAGFVGVHYTPEKVSTQVVNGTNYRYLSKATLPGSSDSWQAVVEIYAPIKGKPHITQIHRI

SEQ ID NO: 93 - protein, 89 aa, Pseudomonas fluorescens
MSAQENLVGGWTPYHELTPKDQEVFDEALAGLVGVHYTAELVSTQVVNGTNYRYQTKATQPGSSNSWQAVVEIYAPINGKPHITQIIRI

SEQ ID NO: 94 - protein, 89 aa, Pseudomonas fluorescens
MSAQENLVGGWTPYHELTPKDQEVFDEALAGLVGVHYTAELVSTQVVNGTNYRYQAKATQPGSPNSWQAVVEIYAPINGKPHITQIIRI

SEQ ID NO: 95 - protein, 89 aa, Pseudomonas fluorescens
MSAQENLVGGWTPYHELTPKDQEVFDEALAGLVGVHYTAELVSTQVVNGTNYRYQAQATQPGSPNSWQAVVEIYAPINGKPHITQIIRI

SEQ ID NO: 96 - protein, 89 aa, Pseudomonas fluorescens
MSAQENLVGGWTPYHELTPKDQEVFDEALAGLVGVHYTAELVSTQVVNGTNYRYQAKATQPGSPNSWQAVVEIYAPINGKPYVTQIIRI

SEQ ID NO: 97 - protein, 89 aa, Pseudomonas fluorescens
MSAQENLVGGWTGYHELTPKDKEVFKEALEGLVGVHYTPELVSSQIVNGTNYRYQTKATQPGSSTSWQAIVEIYAPIKGKPHITQIIRI

SEQ ID NO: 98 - protein, 89 aa, Pseudomonas rhodesiae
MSAQENLVGGWTPYHELTPKDQEVFDVALAGLVGVHYTAELVSTQVVNGTNYRYQAKATQPGSPNSWQAVVEIYAPINGKPYVTQIIRI

SEQ ID NO: 99 - protein, 89 aa, Pseudomonas-sp
MTAQEHLVGGWTPYHKLTPKDQEVFKEALAGFVGVSYTPEEVSSQVVNGTNYRYKSKATLPGSPNGWQAIVEIYAPTNGKPHITQIHRI

SEQ ID NO: 100 - protein, 91 aa, Pseudomonas fluorescens
MSAQENHVGVGGWTAYHELTPKDHAVFKEALEGFVGVQYTPETVSTQVVAGTNYRYHSKAQQPGSPAIWAAIVEIYAPLKGKPHITQIIRI

SEQ ID NO: 101 - protein, 92 aa, Enterobacter-sp
MSEQQTLLPGGWTAYHPLTAQDRKVFEEALNGHLGVDYEPQKVKTQVVAGTNYRFLCEASVPPSTAVWEAIVEIYAPLPGQGAPHITQIIRI

SEQ ID NO: 102 - protein, 89 aa, Shewanella denitrificans
MSNNETIVGGWTAYNAITSAEREIFNKAMEGFVGVSYMPETVSTQVVAGMNYRFKCEASMPPSEVLWEAIVEIYQPLKGIPHITNITKI

SEQ ID NO: 103 - protein, 90 aa, Aeromonas diversa
MSDQAVLVGGWTAYHRLTAEDQAVFQEALKGFVGVEYKPFEVSTQVVAGMNYRYKCKTTVPLPTPIHGEAVVQIFQSLDGSAHITSITPI

SEQ ID NO: 104 - protein, 90 aa, Aeromonas salmonicida
MSEQAVLVGGWTAYHKLTAEDQAVFDQALKGFVGVQYVPFEVCTQVVAGTNYRFKCKSTVPLAKPIHGEAVVQIFQSLDGSAHITSITPI

SEQ ID NO: 105 - protein, 90 aa, Aeromonas veronii
MSEQAVLVGGWTAYHKLTAEDQAVFDQALKGFVGVQYVPFEVSTQVVAGTNYRFKCKSTVPLAKPIHGEAVVQIFKSLDGDAHITSITPI

SEQ ID NO: 106 - protein, 88 aa, Aeromonas molluscorum
MSEQAVLLGGWTAYHKLSAKDQAVFNQALEGFVGVQYTPFEVSTQVVAGTNYRFKCKSTVPLPNPIHGEAVVQIFQALFPKSMQLEWN

SEQ ID NO: 107 - protein, 90 aa, Aeromonas aquariorum
MSEQAVLLGGWTAYHKLSAKDQAVFNQALEGFVGVQYTPFEVSTQVVAGTNYRFKCKTTVPLPNPIHGEAVVQIFQSLDGSAHITSITPI

SEQ ID NO: 108 - DNA, 1737 bp, Pseudomonas brenneri
atgagcacacccttcaaacaattcacctcccccgccgggcaagcccccaaggactacaacaagctgggcctggaaaaccagctgccgcagtttgaaaccgactggaacaatgacctcaccggctggacccagtccgcgatcatcggcaacccgtggtcgggcctcaatgacgcgccgcgctcgggctattacaacccgctggtggaaggctacggccccaccacgccgccggcgattacctgggcgcccttccccaatcggctgtggacgttcttctacaacaacggcacggcggtgattccgcaattgggcggcaaggccatgtccctgcaacaggtgatggagctgaccgacaacggccagattacgatcaacaacaccctgtacatgctctacgacccgaacaagcaaggcaccctgctgcaactgcccgtcacccgctgcccgaccatcgactggcaaggcaagtacaaggatttctcgccctcggggccccgtggctggcttgacgaatactgcgagtggtccatcgtgcgcgatgccgacggcaacatgcgcaagatcaccttcacctgcgaaaacccggcgtatttcctggccatgtggcgcattgatccaaatgcagtgctgggcctgtaccgcgactacatcgacccgcaggtgcagctcgaagacctctacctgcgctacaccgccgactgtccgaccggcaaagcgggcgatccggtcatcgaccctaccaccggccaaccggcctacgacacggtcaacaaatggaacgccggcaccgcctgcgtacccggccaatacggcggggcgatgcacctgacctccggccccaacaccctgagcgccgaggtgtacctggccgccgcggcgaccatcctgcgtccactggccagcagccagaattcccaggcattgatctgctgcgcgcaatacgggcagaactaccgcaactccgacccgcatatcggtttctcggccaacagcgtggcggtgaataaccggctgtccctgaccaatcccatcggcctttacctgcaacaacccaccgatttctcggcgtggaaaggccctcaaggccaggacgtcagccagtactggaaaatcacccgtggcaccgccaagtccgccgccaacggctccgaccagatcctgcaagcggtgtttgaagtgccggtcagcgccgggttttcgatcaacgacatcaccatcagtggccagccgatcgactatgtgtgggtgattgcccagcagttgctggtgggcctgagtgtgacaaccacgcccatcagcccgacgccggattcctgcccctgcgtgaaggatcgggtcaacggcgtgcaaccctggccggtgcaactgctgcccctggatctgttctacgggcagtcgcctaccgacctgccggcctggctggcacccggcaccagcggacagttcgccctggtggtgcaaggcgccgatctcaagaccaccgccgagacggcgcgggtgcaattttccaatcccggcgtgacggcgcaggtcacccagttcctgccggatgcctccgccatccccgggcaaaccaactccggcggcacccagggctacttgctgaccatcaccgtaagccccactgccgctccggggctggtgacggtgcgcgcgctcaacccgggcgaagccgataaccccagcgcgacggaacacccatgggaatccggattggcgctggtgcctggcgcctga

SEQ ID NO: 109 - DNA, 1608 bp, Pseudomonas brenneri
atgtccaggttacgcttaagtgttttatcgctgctgaccagtgtggtgctgagcctgttcgccatgcaggccgcctacgcatcccccacgtccgacgccgacgcttgcgtgcagcaacagttggtgttcaatccgaaaagcggcggtttcctgccgattaacaacttcaacgccaccggccagagctttatgaattgctttggctggcagttgttcattgccctgaactggccggtgaatcccggttggccagccacgcccgccctcgcgggtgagccggacatgaacagtacattggcgcaattcggtgtaccgactgcctccgggcagccgatgagcgtggcgcccgtgtgggccagctacaaggatgccaacgatatcttcctgcccggcgcgcccgcgcccaccggctggggcgtgcaaaccctggtgccgtccaattgcagcacccagggcagcctcagggcgatatcggtgggggcgcgcaagttcatgaccgccacctccgaaagcgcgatcaacgcgcgtcatgggtttcacctgtccagcggcaccctcgcctcgattccagacccgatcatggaagcctccggcggctggctgacggaccagtcgcagaacctggtgttttttgaacgcaaggtgggcaaggccgagttcgactacatcgtcagcaaagggctgtacgacgcagccaaccagctgacagtcgcgcagaacctcgacaaccagaacccgggcgggctgtctctgcccatcggtgaacccatgcgctcgctgccgcccaacccggtgccgcaggagcaactgggagcgctggaggtcaaggcggcgtggcggatccttaccggcaaacccgagctctacgggcgttacctgaccaccgtcgcctggctcaaaaacccggccaccttgcagtgcacccaacaagtggtgggcctggtgggcctgcatatcatcaacaagacccaagcctcgcccaacttcatctggaccaccttcgagcaggtggacaacgtgccggaacccaaccaggtgccgccacaacagacgccgcccgacagctttgccttcaacaacccgaactgcggcaccggccccgaatgcacgccgaacgtggcgcgtatccagtgcaaacagcaccatcccgaccgcgactgcaccgagccgtttccacgggaccaacccgtgcagaccacccgggaacatccgctgcccactgaactgcaggcgcttaacggcgcggtgcaggccaactttgcccagcagagccagggcaagtcggtgttccagtactacaaactgatcaacgtactctggaccctcacccccaacccgcccacccagccggaaccgggtgtcagtgcgcaagtgccgctgtcctacgggccgtttatcagccagggcaacgtaccggtggccaacaccaccctggagacctacgtccagggcgataactgcaatgcctgtcatcagtacgcgaccatcgccggcagctccaccctggcttcggacttttcgttcctgttcaacagcgccgactcggccagcaagaacagcctggtcaagcgcgtgaaagccttccagaccctcaaggatcaaccgtga

SEQ ID NO: 110 - DNA, 1737 bp, Pseudomonas sp. Ag1
atgagcacacccttcaaacaattcacctctcccgccgggcaagctcccaaggactacaacaagctgggcctggaaaaccagttgccgcagtttgaaaccgactggaacaacgacctcaccggctggacccagtccgcgatcatcggcaacccgtggtcgggcctcaatgacgcgccgcgctcgggctattacaacccactggtggaaggctacggccccaccacgccgccggcgattacctgggcgcccttccccaatcggctgtggacgtttttctacaacaacggcacggcggtgattccacagttgggcggcaaggccatgtccatgcaacaggtgatggagctgaccgacaacggccagattacgatcaacaacaccctgtacatgctctacgacccgaacaagcaaggcaccctgctgcaactccccgtcactcgctgcccgagcatcgactggcaaggcaagtacaaggatttctcgccttcgggcccccgtggctggcttgacgaatattgcgagtggtccatagtgcgcgatgccgacggcaacatgcgcaagatcaccttcacttgcgaaaacccggcgtatttcctggccatgtggcgcatcgatccgactgctgtactggggctgtatcgcgactacatcgacccgcaggtgcaactcgaagacctgtacctgcgctacaccgccgactgcccgaccggtaaggccggcgacccggtcatcgaccccaccaccggtcaaccggcctacgacaccgtcaacaaatggaacgccggcaccgcctgtgtgccaggccaatacggcggtgcgatgcacctgacctccggccccaacaccctgagcgccgaggtgtacctggctgccgcggcgaccatcctgcggccattgagcagcagccagaattcccaggcgttgatctgctgcgcgcaatacgggcagaactaccgcaactccgatccgcatatcggtttctcggccaacagcgtggcagtgaataaccggctgtcgctgacgaaccccatcggcctgtacctgcaacaacccaccgacttctcggcgtggaaaggcccccagggccaggacgtcagccagtactggaaaatcacccgtggcaccgccaagtccgccgccaacggctccgaccagattctgcaagcggtgtttgaagtgccggtcagcgccgggttttcgatcaacgagatcaccatcagcggccagccgatcgactacgtgtgggtgattgcccagcagttgctggtgggcctgagtgtgacaaccacgcccatcagcccgacgccggattcctgcccgtgcgtgacggaccgggtcaacggcgtgcaaccctggccggtacagctgctgccgctggacctgttctacgggcagtcacccaccgacctgccggcctggctggcacccggcaccagcgggcagtttgccctggtggtgcaaggcgccgacctcaagaccaccgccgagacggcgcgggtgcaattctccaatcctggggtgacggcgcaggtcacaaagttcctgccggatgcctcggccatccccgggcaaaccaactccggtggcacccagggctacctgctgaccatcaccgtaagccccactgccgcaccggggctggtgacagtgcgcgccctcaacccgggcgaagccgataaccccagcgcggcggaacacccatgggaatccggattggcgctggtgcctggcgcctga

SEQ ID NO: 111 - DNA, 1611 bp, Pseudomonas sp. Ag1
atgtccaggttacgcttgagtgttttatcgctgctgaccagtgtggtgctgagcctgttcgccatgcaggccgcctacgcatcccccacttccgacgccgacgcttgcgtgcagcaacagttggtgttcaacccgaaaagcggcggcttcctgccgatcaacaacttcaacgccaccggccagagcttcatgaattgctttggctggcagttgttcattgccctgaactggccggtgaatcccggttggccagccacacctgccctcgcgggtgagccggacatgaacagtaccctggcgcaattcggcgtaccgactgcctccgggcagccgatgagcgtggcgccggtatgggccagctacaaggacgccaacgatatcttcctgcccggcgcgcccgcgcccaccggctggggcgtgcaaaccctggtgccgtccaattgcagcacccagggcagcctcagggcgatgtcggtgggggcgcgcaagttcatgaccgccacctccgaaagcgcgatcaacgcgcggcatgggtttcacctgtccagcggcaccctggcctcgattccggacccgatcatggaagcctccggcggctggctgacggaccagtcgcagaacctggtgttttttgaacgcaaggtgggcaaggccgagttcgactacatcgtcagcaaagggctgtacgacgcggccaaccagctgaaagtcgcgcagaacctcgacaaccagaaccccggcgggctgtccttgcccatcggtgaacccatgcgctcgctgccgcccaacccggtgccgcaggagcaactgggagctctggaggtcaaggcagcatggcgaatcctcaccggcaaacccgagctctacgggcgttacctgaccaccgtcgcctggctcaaaaacccggccaccttgcagtgcacccagcaagtggtgggcctggtgggcctgcatatcatcaacaagacccaggcctcgcccaacttcatctggaccaccttcgagcaggtagacaacgtgccggaacccgaccaggtgccgccacaacaaacgccgcccgacagctttgccttcaataacccgaactgcggcaccggccccgaatgcacgccgaacgtggcgcgtatccagtgcaagcagcagcatccggaccgcgactgcaccgagccgtttccacgggaccaacccgtgcagaccacccgggaacatccgctgcccactgaactgcaggcgcttaacggcgcggtgcaggccaattttgcccagcagagccagggcaagtcggtgttccagtactacaaactgatcaacgtactctggaccctcacccccaacccgcccacccagccggaaccgggtgtcagtgcgcaagtgccgctgtcctacgggccgtttatcagccagggcaacgtaccggtggccaacaccaccctggagacctacgtccagggcgataactgcaatgcctgtcatcagtacgcgaccatcgccggcagctcgaccctggcctcggacttttcgttcctgttcaacagtgccgattcggccagcaagaaaagcctggtcaagcgcgtaaaagccttccagaccctcaaggacggttcaccctga

SEQ ID NO: 112 - DNA, 1740 bp, Pseudomonas sp. PAMC 25886
atgagcacacccttcaatcaattcacctcgcccgccgggcaagcccccaaggactacaacaagctgggcctggaaaaccagttgccgcagtttgaaaccgactggaacaacgacctcaccggctggacccagtccgcgatcatcggcaacccgtggtcgggcctcaatgacgcgccgcgctcgggctattacaacccgctggtggaaggctacggccccaccacgccaccggcgatcacctgggcgcccttccccaaccggctgtggacgttcttctacaacaatggcaccgcggtgattccgcaattgggcggcaaggccatgacgttgcagcaggtgatggagctgaccgacaacggccagataaccctcaacaacaccttgtacacgctctacgatccgaacaagcaaggcaccctgctgcaactgcccgtgacccgctgcccgagcatcgactggcaaggcaagtacaaggatttctcgccctcggggccccgtggctggctggacgaatattgcgagtggtcgatcgtgcgcgaccccggtacccagaacatgcgcaagatcacctttacctgcgaaaacccggcgtatttcctcgccatgtggcgcatcgacccgaacgcggtgctgggcctgtatcgcgactacatcgacccgcaggtgcaactcgaggacctgtacttgcgatacaccgccgactgcccgaccggcaacaaaggcgatccggtcatggaccccaccaccggccaaccggcctatgacacggtcaacaaatggaacgccggcaccgcctgcgtgcccggccaatatggcggggcaatgcacctgacctccggccccaataccctgagcgccgaggtgtacctggcggccgcagcaaccatcctgcgtccactggccagcagccagaattcccaggcgttgatctgctgcgcgcaatacgggcagaactaccgcaactccgacccgcatatcggcttttcggccaacagcgtggcggtgaataaccggctgtccctgaccaaccccatcggcctgtacctgcaacaacccaccgacttctcggcgtggaaaggtcctcagggccaggacgtcagccagtactggaaaatcacccggggcaccgcaaaatctgcggccaacggctccgaccagatcctgcaggcggtgttcgaagtgccggtcagcgccgggttctcgatcaacgacatcaccatcagcggccagtccatcgactacgtgtgggtgattgcccagcaactgctggtggggctgagcgtgaccaccacgcccatcagcccgacaccggaatcctgcccgtgcgtgaccgatcgggtcaccggtgtgcaaccctggccggtacaactgctgccgctggatctgttctacgggcagtcgcccaccgacctgcccgcgtggctggcacccggtaccagcgggcagtttgccctggtggtgcaaggcgccgacctcaagaccaccgccgagacggcgcgggtgcagttttccaatcccggcgtcacggcggtggtcacgaagttcctgcccgacgcctcggccatccccgggcaaaccaactccggcggcacccagggctacctgctgaccatcaccgtgagccccaccgccgcaccggggctggtgacggtgcgcgcgctcaacccgggcgaagccgataaccccagcgcggcgcagcacccatgggaatccgggttggcgctggtgcctggcgcctga

SEQ ID NO: 113 - DNA, 1608 bp, Pseudomonas sp. PAMC 25886
atgtccaggttacgcttgagtgttttatcgctgctgaccagtgtggtgctgagcctgtttgcggtgcagtcggcctatgcgacgccacaatccgatgccgacgcctgcgtccagcaacagttggtgttcaacccggccagcggtggattcctgccggtcaataacttcaacgccaccggccagagctttatgaactgcttcggctggcagttgttcattgccctgaactggccggtgaatcccggttggccagccacgcccgccctggcgggtgagccggacatgcacagcagcctcgcccagttcggcgtgccgcccgcctccgggcagccgatgaccgtggcgccggtgtgggccagttacaaggacgccaacgatatcttcctgcccggcgcccccgtgcccaccggatggggcgtgcaaaccctggtaccgtccaattgcagcacccagggcagcctcaaggcgatggcggtgggggcgcgcaagttcatgaccgccacctcggaaagcgcgatcaacgcgcggcacgggtttcacctgtccagcggcaccctggcctcgattccggacccgatcatggaagcctccggcggctggctgacggaccagtcgaagaacctggtgttttttgaacgcaaggtcggcaaggccgagtttgactacatcgtcagcaaagggctgtacgacgccgccaaccagctgacagtggcgcagaacctcgacaaccagaacccgggcgggctgtccctgcccatcggtgaacccatgcgctcgctgccgccagacccggtgccgcaggagcaactcggggccctggaggtcaaggccgcgtggcggatcctcaccggtaaacccgagctctacgggcgctacctgaccaccgtcgcctggctcaaaaacccggccacgttgcagtgcacccagcaagtggtgggcctggtgggcctgcacatcatcaacaagacccaggcttcgcccaacttcatctggaccaccttcgagcaggtggacaacgtgccggaacccgaccaggtgccgccacagcagacaccgcccgacagctttgccttcaacaacccgaactgtggcaccggccccgaatgcacgccgaacgtggcgcgtatccagtgcaaacagcatcatcccgaccgcgactgcaccgagccgtatccacgtgaccaaccggtgcaaaccacccgggaacatccgctgcccactgagctgcaggccctgaacggcgcggtgcaggccaacttcgctcagcagagccagggcaagtcggtgttccagtactacaaactgatcaacgtgctctggaccctcacgcccaacccgcccacccagccggagccgggcgtcagcgcgcaggtgccgctgtcctacgggccgtttatcagccagggcaatgtgcccgtggccaacaccaccctggagacctacgtccagggcgacaactgcaacgcctgtcaccagtacgcgaccatcgccggcagctcgaccctggcctcggacttttcgttcctgttcaacagcgccgactcggccagcaagaaaagcctggtcaagcgggtgaaggcgttcgagaccctcaaggaccagccctga

SEQ ID NO: 114 - DNA, 1740 bp, Pseudomonas sp. PAMC 25886
atgagcacacccttcaaacagttcacctcgcccgccgggcaagcgcccaaggactacaacaagctgggcctggaaaaccagttgccgcagtttgaaaccgactggaacaacgacctcaccggctggacccagtccgcgatcatcggcaacccgtggtcgggcctcaatgacgcgccgcgttcgggctattacaacccgctggtggagggctacggccccaccacgccaccggcgatcacctgggcgcccttccccaaccggctgtggacgtttttctacaacaacggcaccgcggtgattccgcagctgggcggcaaggccatgacgttgcagcaggtgatggagctgaccgacaacggccagatcaccctcaacaacaccctgtacacgctctacgatccaaacaagcaaggcaccctgctgcaactgcccgtgacccgctgcccgagcattgactggcaaggcaagtacaaggatttctcgccctcgggcccgcgcggctggctggacgaatactgcgagtggtcgatcgtgcgcgaccccggtacccagaacatgcgcaagatcacctttacctgcgaaaacccggcgtatttcctcgccatgtggcgcatcgacccgaacgcggtactgggcctgtatcgcgactacatcgacccgcaggtgcaactcgaggacctgtacttgcgctacaccgccgactgcccgaccggcaacaagggcgacccggtgatggaccccaccaccggccagccagcctatgacacggtgaacaaatggaacgccggcaccgcctgcgtgcccggccaatatggcggcgcgatgcacctgacctccggccccaacaccctgagcgccgaggtgtacctggcggccgcggccaccatcctgcggccgctgagcagcagccagaactcccaggcgctgatctgctgcgcacaatacgggcagaactatcgcaactccgacccgcatatcggtttttcggccaacagcgtggcggtgaataaccggctgtccctgaccaaccccatcggcctgtacctgcagcaacccaccgacttctcggcgtggaaaggtccacaaggccaggacgtcagccagtactggaaaattacccggggcgccgcaaagtccgccgccaacggctccgaccagatcctgcaggcggtgttcgaggtgccggtcagcgccgggttctcgatcaacgacatcaccatcagcggccagtccatcgactacgtgtgggtgattgcccagcaattgctggtggggctgagcgtgaccaccacgcccatcagcccgacaccggattcttgcccgtgcgtgacggatcgggtcaacggtgtgcaaccctggccggtacaactgctgccgctggatctgttctacgggcagtcgcccaccgacctgcccgcgtggctggctcccggtaccagcgggcagtttgccctggtggtgcaaggcgccgacctcaagaccaccgccgagacggcgcgggtgcagttttccaatcccggcgtcacggcggtggtcacgaaattcctgcccgacgcctcggccatccccgggcagaccaactccggcggcacccagggctacctgctgaccatcactgtgagccccaccgccgcaccggggctggtgacggtgcgcgcgctcaacccgggcgaagccgataaccccagcgcggcggagcacccatgggaatccgggttggcgctggtgcctggcgcctga

SEQ ID NO: 115 - DNA, 1608 bp, Pseudomonas sp. PAMC 25886
atgtccaggttacgcttgagtgttttatcgctgctggccagtgtggtgctgagcctgtttgcgctgcagtcggcctatgcaacaccccaatccgatgccgacgcctgcgtgcagcaacagctggtgttcaatccgaaaagcggcggcttcctgccggtcaacaacttcaacgccaccggccagagcttcatgaactgctttggctggcagctgttcattgccctgaactggccggtgaaccccggctggccgaccaccgccgccctggcgggcgaaccggacatgaacagcagcctggcgcagttcggcgtgccgaccaccgccgggcaaccgatgacggtggcgccggtatgggccagctacaaggacgccaacgatatcttcctgccgggtgcgcctgtgccctcgggctggggcgtgcaaaccctggtgccgtccaattgcagcacccagggcagcctcaaggcgatgtcggtgggggcgcgcaagttcatgactgccacctcggaaagcgcgatcaacgcccgccacggtttccacttgtccagcggcaccctggcgacgattcccgacccgatcatggaagcctccggcggctggctgacggatcaggcgggccagctggtgttttttgaacgcaaagtcggcaaggccgagtttgattacatcgtcagcaaagggctgtacgacgccgccaatcagttgaaggtggcgcaaaacctcgacaaccagaacccgggcgggctgtccttgcccattggcgaaccgatgcgctccctgccgccgaccccggtgccacaggaacaactcggggcgctggagctcaaggccgcgtggcgcattctcaccggcaagcccgaactctacggacgctacctgaccaccgtcgcctggctgaaaaacccggccaccttgcagtgcacccagcaagtggtgggcctggtgggcctgcatatcatcaacaagacccaagcctcgccgaacttcatctggaccaccttcgaacaggtggacaacgtcccggaacccaaccagctgccgccacagcagacgccgcccgacagctttgccttcaacaaccccaactgcggcaccggcccggaatgcacgccgaacgtggcacgcatccagtgccaacagcaccatcccgatcgcgattgcaccgagccgtacccacgggaccaaccggtgcaaaccacccgggaacatccgctgcccacggagctgcaggccctgaacggcgcggtgcaggccaacttcgcccagcagagccagggtaaatcggtgttccagtactacaaactgatcaacgtactctggaccctcacccccaacccgcccgtccagccggagccgggggtcagtgcggcggtgccgctgtcctacgggccgtttatcagccagggcaatgtgccggtggccaacacgaccctggaaacctatgtgcagggcgataactgcaacgcctgtcaccagtacgcgaccatcgccggcagctcgaccctggcctcggacttttcattcctgttcaacagcgccgactcggccagcaagaaaagcctggtcaagcgggtgaaggcgtttgaaaccctcaaggaccaaccctga

SEQ ID NO: 116 - DNA, 1737 bp, Pseudomonas fluorescens
atgagcacacccttcaaacaattcacctctcccgccgggcaagctcccaaggactacaacaagctgggcctggaaaaccagttgccgcagtttgaaaccgactggaacaacgacctcaccggctggacccagtctgcgatcatcggcaacccgtggtcgggcctcaatgacgcgccgcgctcgggctattacaacccactggtggaaggctacggccccaccacgccgccggcgattacctgggcgcccttccccaatcggctgtggacgtttttctacaacaacggcacggcggtgattccgcagttgggcggcaaggccatgtccatgcaacaggtgatggagctgaccgacaacggccagattacgatcaacaacaccctgtacatgctctacgacccgaagaagcaaggcaccctgctgcaactccccgtcactcgctgcccgagcatcgactggcaaggcaagtacaaggatttctcgccctctggcccccgtggctggcttgacgaatattgcgagtggtccatcgtgcgcgatgccgacggcaacatgcgcaagatcaccttcacttgcgaaaacccggcgtatttcctggccatgtggcgcatcgatccgactgctgtactggggctgtatcgcgactacatcgacccacaggtgcaactcgaagacctgtacctgcgctacaccgccgactgcccgaccggtaaggccggcgatccggtcatcgaccccaccaccggtcaaccggcctacgacaccgtcaacaaatggaacgccggcaccgcctgtgtgcctggccagtacggcggtgcgatgcatctgacctccggccccaacaccctgagcgccgaggtgtacctggctgccgcggcgaccatcctgcggccattgagcagcagccagaattcccaggcgttgatctgctgtgcgcaatacgggcagaactaccgcaactccgatccgcatatcggtttctcggccaacagcgtggcagtgaacaaccggctgtcgctgaccaaccccatcggcctgtacctgcaacaacccaccgacttctcggcgtggaaaggcccccagggccaggacgtcagccagtactggaaaatcacccgtggcaccgccaagtccgccgccaacggctccgaccagattctgcaagcggtgtttgaagtgccggtcagcgccgggttctcgatcaacgacatcaccatcagcggccagccgatcgactacgtgtgggtgattgcccagcagttgctggtgggcctgagtgtgacaaccacgcccatcagcccgacgccggattcctgcccgtgcgtgacggaccgggtcaacggtgtgcaaccctggccggtacagctgctgccgctggacctgttctacgggcagtcacccaccgacctgccggcctggctggcacccggcaccagcgggcagtttgccctggtggtgcaaggcgccgacctcaagaccaccgccgagacggcgcgggtgcaattctccaatcctggggtgacggcgcaggtcacaaagttcctgccggatgcctcggccatccccgggcaaaccaactccggtggcacccagggctacctgctgaccatcaccgtaagccccactgccgcaccggggctggtgacagtgcgcgccctcaacccgggcgaagccgataaccccagcgcggcggaacacccatgggaatccggattggcgctggtgcctggcgcctga

SEQ ID NO: 117 - DNA, 1611 bp, Pseudomonas fluorescens
atgtccaggttacgcttgagtgttttatcgctgctgaccagtgtggtgctgagcctgttcgccatgcaggccgcctacgcatcccccacttccgacgccgacgcttgcgtgcagcaacagttggtgttcaacccgaaaagcggcggcttcctgccgatcaacaacttcaacgccaccggccagagcttcatgaattgctttggctggcagttgttcattgccctgaactggccggtgaatcccggttggccagccacgcctgccctcgcgggtgagccggacatgaacagtaccctggcgcaattcggcgtaccgactgcctccgggcagccgatgagcgtggcgccggtatgggccagctacaaggacgccaacgatatcttcctgcccggcgcgcccgtgcccaccggctggggcgtgcaaaccctggtgccgtccaattgcagcacccagggcagcctcagggcgatgtcggtgggggcgcgcaagttcatgaccgccacctccgaaagcgcgatcaacgcgcggcatgggtttcacctgtccagcggcaccctggcctcgattccggacccgatcatggaagcctccggcggctggctgacggaccagtcgcagaacctggtgttttttgaacgcaaggtgggcaaggccgagttcgactacatcgtcagcaaagggctgtacgacgcggccaaccagctgaaagtcgcgcagaacctcgacaaccagaaccccggcgggctgtccttgcccatcggtgaacccatgcgctcgctgccgcccaacccggtgccgcaggagcaactgggagctctggaggtcaaggcagcatggcgaatcctcaccggtaaacccgagctctacggacgttacctgaccaccgtcgcctggctcaaaaacccggccaccttgcagtgcacccagcaggtggtgggcctggtgggcctgcatatcatcaacaagacccaggcctcgcccaacttcatctggaccaccttcgagcaagtggacaacgtgccggaacccaaccaggtgccgccacaacaaacgccgcccgacagctttgccttcaacaacccgaactgcggcaccggccccgaatgcacgccgaacgtggcgcgtatccagtgcaagcagcagcatccggaccgcgactgcaccgagccgtttccacgggaccaacccgtgcagaccacccgggaacatccgctgcccactgaactgcaggcgcttaacggcgcggtgcaggccaattttgcccagcagagccagggcaagtcggtgttccagtactacaaactgatcaacgtactctggaccctcacccccaacccgcccacccagccggaaccgggtgtcagtgcgcaagtgccgctgtcctacgggccatttatcagccagggcaacgtaccggtggccaacaccaccctggagacctacgtccagggcgacaactgcaatgcctgtcatcagtacgcgaccatcgccggcagctcgaccctggcctcggacttttcgttcctgttcaacagtgccgattcggccagcaagaaaagcctggtcaagcgcgtaaaagccttccagaccctcaaggacggttcaccctga

SEQ ID NO: 118 - DNA, 1737 bp, Pseudomonas sp. PAMC 26793
atgagcacacccttcaaacaattcacctctcccgccgggcaagcacccaaggactacaacaagctgggcctggaaaaccagctgccgcagtttgaaaccgactggaacaacgacctcaccggctggacccagtccgcaatcatcggcaacccgtggtcgggcctcaatgacgcaccgcgctcgggctattacaacccgctggtggaaggctacggccccagcacgccgccggcgattacctgggcgcccttccccaatcggctgtggacgttcttctacaacaacggcacggcggtgattccgcaattgggcggcaaggccatgtccatgcaacaggtgatggaactgaccgacaacggccagattacgatcaacaacaccctgtacatgctctacgacccgaacaagcaaggcaccctgctgcaactgcccgtcacccgctgcccgaccatcgactggcaaggcaagtacaaggatttctcgccctcggggccccgtggctggcttgacgaatactgcgagtggtccatcgtgcgtgacgccaatggcaacatgcgcaagatcaccttcacctgcgaaaacccggcgtatttcctggccatgtggcgcattgatccaaatgcagtgctgggcctgtaccgcgactacatcgacccgcaggtgcaactcgaagacctgtacttgcgctacaccgccgactgcccgaccggcaaagccggcgatccggtcatcgaccctaccaccggccaaccggcctacgacacggtcaacaaatggaacgccggcaccgcctgcgtacccggccaatacggcggggcgatgcacctgacctccggccccaacaccttgagcgccgaggtgtacctggccgccgcagcgaccatcctgcgtccactggccagcagccagaattcccaggcattgatctgctgcgcgcaatacgggcagaactaccgcaactctgacccgcatatcggtttctcggccaacagcgtggcggtgaataaccggctgtccctgaccaaccccatcggcctttacctgcaacaacccaccgatttctcggcgtggaaaggccctcaaggccaggacgtcagccagtactggaaaatcacccgtggcaccgccaagtccgccgccaacggctccgaccagattctgcaagcggtgtttgaagtgccggtcagcgccgggttttcgatcaacgacatcaccatcagtggccagccgatcaactatgtgtgggtgattgcccagcagttgctggtgggcctgagtgtgacaaccacgcccatcagcccgacgccggattcctgcccctgcgtgacggatcgggtcaacggcgtgcaaccctggccggtgcaactgctgcccctggatctgttctacgggcagtcgcctaccgacctgccggcgtggctggcacccggcaccagcgggcagttcgctctggtggtgcaaggcgccgacctcaagaccaccgccgagacggcgcgggtgcagttttccaatcctagcgtgacggcgcaggtcacccagttcctgccggatgcctccgccatcccagggcaaaccaactccggtggcacccagggctacctgctgaccatcaccgtaagccccactgccgctccgggactggtgacggtgcgcgcgctcaacccgggcgaagccgataaccccagcgcgacggaacatccatgggagtccggattggcgctggtgcctggcgcctga

SEQ ID NO: 119 - DNA, 1608 bp, Pseudomonas sp. PAMC 26793
atgtccaggttacgcttaagtgttttatcgctgctgaccagtgtggtgctgagcctgttcgccatgcaggccgcctacgcatcccccacttccgacgccgacgcttgcgtgcagcaacagttggtgttcaacccgaaaagcggcgggttcctgccgatcaacaacttcaacgccaccggccagagctttatgaattgctttggctggcagttgttcattgccctgaactggccggtgaatcccggttggccagccacgcccgccctcgcgggtgagccggacatgaacagtaccctggcgcaattcggtgtgccgcccgcctccgggcagccaatgagcgtcgcgccggtatgggccagctacaaggacgccaacgatatcttcctgcccggcgcccccgcgcccaccggctggggcgtgcaaaccctggtgccgtccaattgcagcacccagggcagcctcagggcgatgtcggtgggggcgcgcaagttcatgaccgccacctccgaaagcgcgatcaacgcccgccatggttttcacctgtccagcggcaccttggcctcgattccagacccgatcatggaagcctccggcggctggctgacggaccagtcgcagaacctggtgttttttgaacgcaaggtgggcaaggccgagttcgactacatcgtcagcaaagggctgtacgacgcagccaaccagctgaaagtcgcgcagaacatcgacaaccagaacccgggcgggctgtccttgcccatcggtgagcccatgcgctcgctgccgcccaacccggtgccgcaggagcaactgggagccctggaggtcaaggcggcgtggcggatcctcaccggcaaacccgagctctacgggcgttacctgaccaccgtcgcctggctcaaaaacccggccaccttgcagtgcacccagcaagtggtgggcctggtgggcctgcatatcatcaacaagacccaagcctcgcccaacttcatctggaccaccttcgagcaggtggacaacgtgccggaacccaaccaggtgccgccacaacagacgccgcccgacagctttgccttcaacaacccgaactgcggcaccggccccgaatgcacgccgaacgtggcgcgtatccagtgcaaacagcaccatcccgaccgcgactgcaccgagccgtttccacgggaccaacccgtgcagaccacccgggaacatccgctgcccactgaactgcaggcgcttaacggcgcggtgcaggccaacttcgcccagcagagccagggcaagtcggtgttccaatactacaaattgatcaacgtactctggaccctcacccccaacccgcccacccagccggaaccgggtgtcagtgcgcaagtgccactgtcctacgggccgtttatcagccagggcaacgtaccggtggccaacaccaccctggagacctacgtccagggcgataactgcaatgcctgtcatcagtacgcaaccatcgccggcagctccaccctggcttcggacttttcgttcctcttcaacagcgccgactcggccagcaagaaaagcctggtcaagcgcgtgaaagccttccagaccctcaaggatcaaccgtga

SEQ ID NO: 120 - DNA, 1737 bp, Pseudomonas putida
atgagcacgcccttcaagcagttcacctctcccgccggccaagcccccaaggactacaacaagctgggcctggaagaccagttgccgcagtttgaaaccgactggaacaacaacctcaccggctggaccgaatcgtcgatcatcggcaacccctggtcgggcctgaacgacgccccccgctcgggttactacaacccgctggtggaaggtttcggcgacgtgaccgccccggcgatcacctgggcgcccttccccaaccggctctggacgttcttctacaacaacggtgcggcggtcattccccagctgggtggcaaggccatgaccctggaccaggtgatggaattgaccgaccacggccagatcaccctcgacaacaccctctacatgctctacgaccccaacaagcaaggtaccgtgctgcaactgccggccaagcgctgcccgagcatcgactggaacggcaaatacacggcgttctcgccttccggcccgcggggctggctcgacgagtactgcgagtggtcgatcgtacgcgatgccaacggcaacatgcgcaagatcaccttcacctgcgaaaaccccgcgtacttcctgaccatgtggcgcatcgacccgaacgcagtactggggctgtaccgcgactacatcgacccgaacgtgcaactcgaagacctgtacctgcgctacaccgtcgactgcccgaccggcaaggccggcgacccggtcatcgaccccaccaccggcaagccggcctatgacaccgtcaacaaatggaacgccggaacggcctgtgtacccggccagtacggcggtgcgatgcacctgacctccggccccaataccctcagcgccgaggtgtacctggccgccgccgccaccattctgcgcccggtgagcagcagccagaacgcccagtcgttgatctgctgcgcgcagtacgggcaaaactatcgcaactctgatccgcacatcggtttcatggccaataccacggcagtgaacaaccgactgtcgctgaccaaccccattggcctgtacttgcagcagcccaccgatttcagcgcctggaagggcccgcaaggccaggacgtgagccagtattggcgcatcacgcgcggtacggccaagtcggctgccaatggttccgaccagatcctgcaggcggtgttcgaggtgccggaaagcgccggcttctcgatcaatgacatcaccatcaacaaccagaaggtcaactatgtgtgggtcatcgcccaacaactgctggtcggcctgagtgtcaccgtcaagccgctcagcgccacgcttcaagcattcccatgcgtgcaggaccgggtggccggcctgcaaccctggccagtgcaactgctgccgctggacctgttctacgggcaatccccaaccgacctgcccgcctggcttgcaccgggtagcagcaaccagttcgtgctggtggtgcaaggggccgacccgactaccacggcgcagaatgcaagggtgcaattctccaaccccggggtgacggcgcaggtcacccagtacctgcccgacgcgtcggccattcccggccagaccaactcgggcggcacccaggcctacattctgaccatcacggtcagcccctccgcagcacccggcctggtgacagtgcgtgccctcaacccgggtgaagatgtgaacgtgagcgcgacagaccacccttgggaatctggcctggcgctggtgccgggggcctga

SEQ ID NO: 121 - DNA, 1608 bp, Pseudomonas putida
atgatgtccaggtcacgcttgagtcctctgtcgctgctgtgcggcattctactgtgcctgtcgaccctgcaacccgccacggcggccacgctgtcggacgccgatacctgtgtacagcagcaattggtgttcaacccggccagcgggggattcctgccggtcaacaacttcaatgccaccagccaggcgttcatgaactgctttggctggcaattgttcattgccttgaactggccggtgaaccccggttggccggccaccgccagcctggcgggtgaacccgacatgcaaagcacgctggcgcagttcggggtcccctccgcaccgggtcagcccatgagcgtggccccggtatgggccagctacaaggacgccaacgacatcttcctgcccggcgcacccacgcccaccggctggggtgtgcaaaccctggtgccgtccggctgcagcacccagggtagcctcaaggcgctcaaggtgggcgcacgcaagttcatgaacgccacctccgaaggcgcgatcaatgccttgcacggtttccacctgtcgaccgggacacttgcgtccattcccgacccggtcatggaggcgtccggcggctggctgacggaccaggcgggcaaactggtattttttgagcgcaaggtgggcaaggccgagttcgactacatcgtcgacaaggggctctacgacgccgccaaccagttgaaggtcgcgcaaaacctcgacggccagacaccggagggcctgtcgttgcccatcggcgaaccgatgcgctcactgccaacctccccagtgccacaggaacaactgggcgcgatcgagctcaaggccgcctggcgggtgctgaccggcaaacccgagctgttcggccgctacctgactaccgtcgcctggctcaaacgccccgacacgctggagtgcacccaggaggtggtggggctggtgggcctgcatatcatcaacaagacccaggcttcgcccaacttcatctggaccaccttcgagcaggtggacaacgtgcccgaaccggcccaggtcccgccgcaacaaaccccgccgaacgggttcgccttcaacaaccctgactgtggcgacggccccgagtgcacaccgaaccaagcccgtatccagtgcaagcaaacgcatcccgacaaggactgcaccgatctcttcccacgcgaccagccggtacagaccacccgcgaacaccccgtgcccggcgacctgcaagccctcaacagcgcggtacaagccaacttcgcgcagcacagccaaggcaagtcggtgttccagtactacaagctgatcaacgtactctggaccctcgctcccaatccgcccagcccggaaccgggcgccaacgcgcaagtgccgctgtcgtacgggcccttcatcagccagggcaacgtgccggtggccaacaccaccatggagacctacgtgcagggtgatgactgcaatcagtgccatcagtacgcgacgattgccggcagcccgtcattggcctcggatttctctttcctgttcaacagtgccggttccgccagcaacaaaagcctgatcaaaagcgtcaaagccttcgaaaccctcaaggaccgtccctga

SEQ ID NO: 122 - DNA, 1737 bp, unknown
  Fungus garden combined
atgagcacgcccttcaagcagttcacctctcccgccggccaagcccccaaggactacaacaagctgggcctggaagaccagttgccgcagtttgaaaccgactggaacaacaacctcaccggctggaccgaatcgtcgatcatcggcaacccctggtcaggcctgaacgacgccccccgctcgggttactacaacccgctggtggaaggtttcggcgacgtgaccgccccggcgatcacctgggcgcccttccccaaccggctctggacgttcttctacaacaacggtgcggcggtcattccccagctaggtggcaaggccatgaccctggaccaggtaatggcgttgaccgaccacggccagatcaccctcgacaacaccctctacatgctctacgaccccaacaagcaaggtactgtgctgcaactgccggccaagcgctgcccgagcatcgactggaacggcaagtacacggcgttctcgccttccgggcctcggggctggctcgacgagtactgcgagtggtcgatcgtacgcgatgccaacggcaacatgcgcaagatcaccttcacctgcgaaaaccccgcgtacttcctgaccatgtggcgcatcgacccgaacgcagtactgggcctgtaccgcgactacatcgacccgaacgtgcaactcgaagacctgtacctgcgctacaccgtcgactgcccgaccggcaaagccggcgacccggtcatcgaccccaccaccggcaagccggcctatgacaccgtcaacaaatggaacgccggaacggcctgtgtgcccggccagtacggcggtgcgatgcacctgacctccggccccaataccctcagcgccgaggtgtacctggccgccgccgccaccatcctgcgcccggtgagcagcagccagaacgcccagtcgttgatctgctgcgcgcagtacgggcaaaactatcgcaactctgatccgcacatcggtttcatggccaataccacggcagtgaacaaccgactgtcgctgaccaaccccattggcctgtacttgcaacagcccaccgatttcagcgcctggaagggcccgcaaggccaggacgtgagccagtactggcgcatcacgcgcggtacggccaagtcggctgccaacggttccgaccagatcctccaggcggtgttcgaggtgccggaaagcgctggtttctcgatcaatgacatcaccatcaacaaccagaaggtcaactatgtgtgggtcatcgcccaacaactgctagtcggcctgagcgtcaccgtcaagccgctcagcaccacgcctcaagcgttcccatgcgtgcaggaccgggtggccggccggcaaccctggccagtgcaactgctgccgctggacctgttctacgggcaatcccccaccgacctgcccgcctggcttgcaccgggtagcagcaaccagttcgtgctggtggtgcaaggtgccgacccgactaccacggcgcagaatgcaagggtgcaattctccaaccctggggtgacggcgcaggtcacccagtacctgcccgacgcatcggccattcctggccagaccaactcgggcggcacccaggcctacattctgaccatcacggtcagcccctccgcagcacccggcttggtggcagtgcgtgccctcaatccgggtgaagacgttaacgtgagcgcgacagaccacccttgggagtctggcctggcgctggtgcctggcgcctga

SEQ ID NO: 123 - DNA, 1605 bp, unknown
  Fungus garden combined
atgtccaggtcacgcttgagtcttctgtcgctgctgtgcggcattctactgtgcctgtcgaccccgcaacccgccacggcggccacgctgtcggacgccgatacctgtgtacagcagcaattggtgttcaacccggccagcgggggattcctgccggtcaacaacttcaatgccaccagccaggcgttcatgaactgctttggctggcaattgttcattgccttgaactggccggtgaaccccggttggccagccaccgccagcctggcgggtgaacccgacatgcaaagcacgctggcgcagttcggggtcccctccgcaccgggtcagcccatgagcgtggccccggtatgggccagctacaaggacgccaacgacatcttcctgcccggcgcacccacgcctaccggttggggcgtgcaaaccctggtgccgtccggctgcagcacccagggtaacctcaaggcgctcaaggtgggcgcacgcaagttcatgaacgccacctccgaaggcgcgatcaatgccttgcacggtttccacctgtcgaccgggacacttgcgtccattcccgacccggtcatggaggcgtccggcggctggctgacggaccaggcgggcaagctggtgtttttcgaacgcaaggtgggcaaggccgagttcgactacatcgtcgacaaggggctctacgacgcagccaaccagttgaaggtcgcgcaaaacctcgacggccagacaccggagggcctgtcgctgcccatcggcgaaccgatgcgctcactgccgacctccccagtgccacaggagcaacttggcgcgatcgagctcaaggccgcctggcgggtgctgaccggcaaacccgagctgttcgggcgctacctgactaccgtcgcctggctcaaacgccccgacacgctggagtgtacccaggaggtggtggggctggtgggcctgcatatcatcaacaagacccaggcttcgcccaacttcatctggaccaccttcgagcaggtggacaacgtgcccgaaccggcccaggtcccgccgcaacaaaccccgccgaacgggttcgccttcaacaaccctgactgtggcgacggccccgagtgcacaccgaaccaagcccgtatccagtgcaagcaaacgcatcccgacaaggactgcaccgatctcttcccacgcgaccagccggtacagaccacccgcgaacaccccgtgcccggcgacctgcaagccctcaacagcgcggtacaagccaacttcgcgcagcacagccaaggcaagtcggtgttccagtactacaagctgatcaacgtactctggaccctcgcccccaatccgcccagcccggaaccgggcgccaacgcgcaagtgccgttgtcgtacgggccgttcatcagccagggcaacgtaccggtggccaacaccaccatggagacctacgtgcagggtgatgactgcaatcagtgccatcagtacgcgacgattgccggcagcccgtcattggcctcggatttctctttcctgttcaacagtgccggctccgccagcaacaaaagcctgatcaaaagcgtcaaagccttcgaaaccctcaaggaccgcccctga

SEQ ID NO: 124 - DNA, 1734 bp, Pseudomonas monteilii
atgagcacgcccttcaagcagttcacatctcccgccggccaagcccccaaggactacaacaagctgggcctggaagaccagttgccgcagtttgaaaccgactggaacaacaacctcaccggctggaccgaatcgtcgatcatcggcaacccctggtcgggcctgaacgacgccccccgctcgggttactacaacccgctggtggaaggtttcggcgacgtgaccgccccggcgatcacctgggcgcccttccccaaccggctctggacgttcttctacaacaacggtgcagcggtcattccccagctgggtggcaaggccatgaccctggaccaggtgatggagttgaccgaccacggccagatcaccctcgataacaccctctacatgctctacgaccccaacaagcaaggtaccgtgttgcaactgccggccaagcgctgcccgagcatcgactggaacggcaagtacacggcgttctcgccttccgggcctcggggctggctcgacgagtactgcgagtggtcgatcgtacgcgatgccaacggcaacatgcgcaagatcaccttcacctgcgaaaaccccgcgtacttcctgaccatgtggcgcatcgacccgaacgcagtactggggctgtaccgcgactacatcgacccgaacgtgcaactcgaagacctgtacctgcgctacaccgtcgactgcccgaccggcaaagccggcgacccggtcatcgaccccaccaccggcaagccggcctatgacaccgtcaacaaatggaacgccggaacggcctgtgtgcccggccagtatggcggtgcgatgcacctgacctccggccccaataccctcagcgccgaggtgtacctggccgccgccgccaccatcctgcgcccggtgagcagcagccagaacgcccagtcgttgatctgctgcgcgcagtacgggcaaaactatcgcaactctgatccgcacatcggtttcatggccaataccacggcggtgaacaaccgactgtcgctgaccaaccccattggcctgtacttgcaacagcccaccgatttcagcgcctggaagggcccacaaggccaggacgtgagccagtactggcgcatcacgcgcggtacggccaagtcggctgccaacggttccgaccagatcctgcaggcggtgttcgaggtgccggaaagcgctggtttctcgatcaatgacatcaccatcaacaaccagaaggtcaactatgtgtgggtcatcgcccaacaactgttggtcggcctgagcgtcaccgccaagccgctcagcgccacgccccaagcattcccatgcgtgcaggaccgggtggccggcctgcaaccctggccagtgcaactgctgccgctggacctgttctacgggcaatcccccaccgacctgcccgcctggcttgcaccgggtagcagcaaccagttcgtgctggtggtgcaaggtgccgacccgactaccacggcgcagaatgccagggtgcaattctccaaccccggggtgacggcgcaggtaacccagtacctgcccgacgcgtcggccattcccggccagaccaactcgggcggcacccaggcctacattctgaccatcacggtcagcccctccgcagcacccggcctggtggcattgcgtgccctcaacccgggtgaagatgtgaacgtgagcgcgacagaccacccttgggaatctggcctggcgctggtgcctggcgcc

SEQ ID NO: 125 - DNA, 1605 bp, Pseudomonas monteilii
atgatgtccaggtcacgcttgagtcttctgtcgctgctgtgcggcattctactgtgcctgtcgaccccgcaacccgccacggcggccacgctgtcggacgccgatacctgtgtacagcagcaattggtgttcaacccggccagcgggggattcctgccggtcaacaacttcaatgccaccagccaggcgttcatgaactgctttggctggcagttgttcattgccttgaactggccggtgaaccccggttggccggccaccgccagcctggcgggcgaacccgacatgcaaagcacgctggcgcagttcggggtcccctccacaccgggtcaacccatgagcgtggccccggtatgggccagctacaaggacgccaacgacatcttcctgcccggcgcccccacgcccaccggctggggcgtgcaaaccctggtaccgtccgactgcagcacccaaggtagcctcaagacactcaaggtgggcgcgcgcaagttcatgaacgccacctccgaaggcgcgatcaatgccttgcacggtttccacctgtcgaccgggacacttgcctccattcccgacccggtcatggaagcgtccggcggctggctgacggaccaggcgggcaaactggtgttttttgaacgcaaggtgggcaaggccgagttcgactacatcgtcgacaaggggctctacgacgccgccaaccaattgaaggtcgcgcgaaacctcgacggccagacaccggagggtctgtcactgcccatcggcgaaccgatgcgctcactgcctacctccccagtgccacaggagcaactgggcgcgatcgagctcaaggccgcctggcgggtactgactggcaaacccgagctgttcgggcgctacctgactaccgtcgcctggctcaaacgtcccgacacgctggagtgcacccaggaggtggtggggctggtgggcctgcatatcatcaacaagacccaggcttcgcccaacttcatctggaccaccttcgagcaggtggacaacgtgcccgaaccggcccaggttccgccgcaacaaaccccgccaaacgggtttgccttcaacaaccctgactgtggcaacggccccgagtgcacaccaaaccaagcccgtatccagtgcaagcaaacgcatcccgacaaggactgcaccgatctcttcccgcgcgaccagccggtacagaccacccgcgaacaccccgtgcccggcgacctgcaagccctcaacagcgcggtacaagccaacttcgcgcagcacagccaaggcaagtcggtgttccagtactacaagctggtcaacgtactctggaccctcgctcccaacccgcccagcccggaaccgggcgccaacgcgcaagtgccgctgtcgtacgggccgttcatcagccaggggaacgtgccggtggccaacaccaccatggagacctacgtgcagggtgataactgcaatcagtgccatcagtacgcgacgattgccggcagcccgtcattggcctcggatttctcttttctgttcaacagtgccggctccgccagcaacaaaagcctgatcaaaagcgtcaaagccttcgaaaccctcaaggaccgcccc

SEQ ID NO: 126 - DNA, 1738 bp, Pseudomonas monteilii
atgagcacacccttcaaacaattcacctctcccgccggacaagcccccaaggactacaacaagctgggcctggaagaccagttgccgcagtttgaaaccgactggaacaacaacctcaccggctggacccaatcgtccatcatcggcaacccttggtcgggcctgaacgacgctccccgctcgggctactacaacccgctcgtagagggcttcggcgacgtgaccccacccgcgatcacctgggcgcccttccccaaccgcctgtggacgttcttctacaacaacggtgcggcggtcattccccagttgggcggcaaggccatgaccctggaccaggtgatggaattggccgaccacggccagatcaccctcgacaacaccctctacacgctttacgacccgaacaaaaagggcactgtgctgcaactgccggtcaagcgctgccccagcatcgcctggaatggcacgtacaaggatttcacgccttccggcccacggggctggctcgacgagtactgcgagtggtcgatcgtgcgcgatgccaacggcaacatgcgcaagatcaccttcacctgtgaaaaccccgcgtacttcctggccatgtggcgcatcgacccgaacgcggtcctgggcctgtaccgcgaatacatcgacccgagcgtgcagctcgaagacctgtacctgcgctatgccgaagactgcccgaccggcaaggccggcgatccggtcatggaccccaccaccggcaagccggcctatgacaccgtcaacaaatggaacgccggaaccgcctgtgtgcccggccagtacggcggagcgatgcacctgacatccggccccaataccctcagtgccgaggtgtacctggccgccgccgccaccatcctgcgcccggtgagcagcagccagaatgcccagtcgctgatctgctgcgcgcagtacgggcagaactatcgcaactccgacccgcacatcggcttcatggccaataccacggcggtcaacaaccgactgtcgctgaccaaccctattggcctgtacttgcaacaacccaccgacttcagcgcctggaagggcccgcaaggccaggacgtgagccagtactggcgcatcacccgcggtacggccaagtcggccgccaacggctccgaccagatcctgcaggcggtgttcgaggtgccggaaagcgccggcttctcgatcaatgacatcaccatcaacaaccagaaggtcaactatgtgtgggtcatcgcccaacaactgttggtgggcctgagcgtcaccgtcaaaccgctcagcgtcacacctcaatccttcccatgcgtgcaggaccgggtggccggcctgcaaccctggccggtgcaactgctgccgctggacctgttctacgggaactcccccaccgacctgcccgcctggcttgcaccgggcagcagcaatcagttcgtgctggtggtgcaaggcgccgacaagaccaccacggcgcagaatgccagggtgcaattctccaaccccggggttaccgcgcaggtcacccagtacctgcccgacgcgtcggccattcccggccagaccaacgccggcggcacacaggcctacatcctgaccatcacggtcagccccaccgcagcccccggcctggtgacggtgcgtgcgctcaatccggatgaagacgtgaacgtgagcgcggcagaccacccttgggaatccggcctggcgctggtgcctggcgcctgaa

SEQ ID NO: 127 - DNA, 1605 bp, Pseudomonas monteilii
atgtccaggtcacgcttgagtcttctgtcgctgctgtgcggcattttactgtgcctgtcgaccccgcaacccgccatggcagccacgctgtcggatgccgacgcctgtgtgcagcagcagttggtgttcaacccggccagcgggggattcctgccggtcaacaacttcaatgccaccagccaggcgttcatgaactgctttggctggcagctgttcattgccttgaactggccggtgaaccccggctggccggccaccgccagcctggcgggcgaacccgacatgaacagcacgctggcgcagttcggtgtcccctccgcaccgggccaacccatgagcgtggccccggtatgggccagctacaaggacgccaatgacatcttcctgcccggcgcgcccacgcccactggctggggcgtacaaaccctggtgccgtccggttgcagcactcagggtagcctcaagtcactcaaggtaggcgcacgcaagttcatgaacgccacctccgaaggcgcgatcaatgccttgcaccgattccacctgtctaccggaacactcgcgtccattcccgacccggtcatggaagcgtccggcggctggttgacggaccagtctggcaacctggtgttttttgagcgcaaggtaggcaaggccgagttcgactacatcgtcgacaaggggctctacgacgccgccaaccagttgaaggtggcgcaaaaccaggacggcaagacaccggaggggctgtcgctgccaatcggcgaaccgatgcgctcgctgcctccgtcccctgtcccgcaggagcagctgggcgcgatcgagctcaaggccgcctggcgggtgctgaccggcaaacccgaactgttcgggcgctacctgaccaccgtcgcctggctcaaacgccccgataccctgaactgcacccaggaagtggtggggctggtgggcctgcatatcatcaacaagacccaggcttcgcccaacttcatctggaccactttcgagcaggtcgacaacgtgcctgaaccggcccaggccccgccgcaacaaaccccaccgaacggttttgccttcaacaaccctgactgtggcagtggccccgagtgcacaccgaaccaagcccgtatccagtgcaagcaacaccatcccgataagcaatgcaccgatctcttcccacgcgaccagccggtacagaccacccgcgaacaccccatacccagcgacctgcaggccctcaacagcgcggtgcaagccaacttcgcgcagcacagtcaaggccagtcggtgttccagtactacaagctgatcaacgtactctggaccctcgcccccaatccgcccagcccggaaccgggcgccaacgcgcaagtgccgctgtcgtacgggccattcatcagccagggcaacgtgccggtggccaacaccaccatggagacttacgtacagggtgatgactgcaaccagtgccatcagtacgcgacgattgccggcagcccttcgttggcctcggacttctctttcctgttcaacagtgccggttctgccagcaccaaaagcctgatcaaaagcgtcaaagccttccagaccctcaaggatcaaccgtga

SEQ ID NO: 128 - DNA, 1746 bp, Pseudomonas brenneri
atgagcacgcccttcaagcaattcacctcccccgctgggcaagcgccaaaggactacaacaagctgggcctggaagaccagttgccacaattcgaaaccgactggaacaacgacataaccggctggaccgaagcggcgatcatcggcaacccctggtcgggcctgtatgacgcgccccgctcggcctattacaacccgctggtcgaaggctatggcgacaccaccctgccggcgattacctggcaaccctttcccaaccggctgtggacctttttctacaacaacggcacggcggtgattccccaactgggcaacaaggccatgaccctgcaacaggtcatggagctgaccgacaacggccagatcaccatcaacggcaccctgtacaccctgtacgacccggacaagaaaggcaccctgctgcaactgcccgtaacccgctgcccgactatcgactggaacggcaaatacaaagacttctcaccctcggggccacggggctggctggacgaatactgcgagtggtcgatcgtgcgcgataccaacggcaacatgcgcaagatcacctttaccagtgaaaacccggcgtacttcctggccatgtggcgcatcgatccgaatgccgtgctgggcttgtatcgcgactacatcgacccgaatgtgcaactgcaagatctctatctgcgctacaccgccgactgcaagaccggcaaggccggtgacccggtgattgacccgaccacgggcctgccggcctacgacacggtcaacaaatggaactccggcactgcctgcacccccggccagttcggcggcgcgatgcacctgacctctgggcccaacactctcagcgccgaggtgtacctggcggcggcggccactatcatgcggcccctgaaaagcagccagagcgcccaggcgctgatctgctgcgcgcaatatgggcagaactatcgcaactccgacccgcatatcggctttgcagccaacggggcgacaaatgatggggccacccccagccggatttccctgaccaaccccatcgccctgtacctgcaacagccgaccaacttcaatgcctggaaaggcccccaaggccaggatgtgagccagtactggcgcatcacccgcggtaccgccaaatcggcgatcaacggctccgaccagatcctgcaggcggtgttcgaggtaccggaaagtgccgggttctcgatcaacgacatcaccatcaatggccaggcggtggactatgtgtgggtgattgcccagcaattgctggtgggcctgagtgtcaccaccatgccgagcaccgcgcagcagcaatcgccttgcgtgcaggatcgggtcaatggcctgcagccctggccggtgcagttgttgccgctggacctgttctacggccagtcgcccaccgacctgccggcctggctggccccaggtaccagcgggcaattcgcgctggtggtacaaggcgcggacctcaagaccaccgccgccaccgcacggatccagttcaacaaccccggggtcacggcgcaggtcacggagttcctgcccgacgcctcggccattcccggccagaccaatgcgggcggcacccagggctacatcatgaccatcaccgtcgcaaaagacgcggcgccgggactggtgacagtgcgcgcgctcaatccgggcgaggcggataacgtcagcgcggcggaccacccttgggagtccgggctggcgctggtgccatccacttaa

SEQ ID NO: 129 - DNA, 1602 bp, Pseudomonas brenneri
atgatgtacagatttcgcttacgtggtctgctgctggtcggcacgctgctgtcgctgtttctcctgcccacggcccaggcatcggatgccgatacctgcgtccagcagcagttggtgttcgaccccaacagcggcggttttctacccgtcaacaatttcaacaccactggccagagcttcatgaactgttttggctggcagctgtttattgccctgaactggcccgtggatcccggatggccagccaatgcagccctcgcgggcgagccgaaccgcaagatcagcatggcgcaatttggcgtgccccaggtcgccgggcaacccatgaccaccgcgccggtgtgggcaagctttaaagacgctaacgatatattcctgcccggcgcccgaccgcccacaggctggggcgtgcagacattggtgccgtccaattgcagcagcgagggcagcctcaaagcgttgtcggtgggggcgcgcaagttcatgaacgccacctcggaaagcgcgaccaacgccaagcatcgcttccacttgtccagcggtaccctggcgtcgattcccgacccgatcatggaagccgccggtggctggctgacggaccagaccggcaacctggtgtatttcgagcgcaaggtgggcaaggccgagtttgactatatcgtcaagtacgggctgtacgatgccgccaatcaaatggtcgttgcacaaaacagcgatggcaatcatccggccgggctgtccctgcccgccggcgagctgatgcgctcgatgccggcgcaacccctgccccaggagcaactgggcgccctggaactcaaggccgcctggcgtatcctcaccggcaagccccagctctacgggcgctacctgaccaccgtggcctggctcaagaaccccgccaccctgcagtgcacccaacaggtggtgggcctggtgggcctgcatatcatcaacaagacccagagttcaccgaactttatctggaccacattcgagcaagtagacaacgtacaagagccaggccaggtgcccgcgcaacagacaccgcccgacggttttaccttctacaaccccaattgcaccggtggccctgacgtgtgcacgcccaacgtggcccgtatccagtgccagcagcaccaccctgatcgcgaatgcaccgagccctatccacgcaaccaaccggtccagaccactcgcgaacaccccctgccttcggacatgcaggccctcaacggcgccgtgcaggctaacttcgcccagcagaccaacggccagtcggtgttccagtactacaaactggtcaatgtgctgtggatcaccgccccgaccgcaccggacccggagccgggcgcgggtgcgaaggtgcccctgtcctatggcgcctttatcagcgatagcaacgtaccggtggccaataccaccatggagacctacgtccagagcatggactgcaatgcctgccatcagcaggcgacgattgccggcagcagcagcctggcctcggacttctcgttcctgttcaacaacgccgattcggccaagcaaaaaagcctgatcaaacgcgtaaatgccttcgaaaccctcaaggatggcccaccatga

SEQ ID NO: 130 - DNA, 1851 bp, Pseudomonas gessardii
atgcccgctgcctggctttatcgcccaactggtgtgggacgacccgcgccagaccgttgccgaccctccctcgagtgccggttgctgctccgtttctaccccccatggagatctgacatgagcacgcccttcaagcaattcacctcccccgccgggcaagcgccaaaggactacaacaagctgggcctggaagaccagttgccgcaatttgaaaccgactggaacaacgacgtcaccggctggaccgaagcggcgatcatcggcaacccatggtcgggcctgtacgacgcgccacgctcgggctattacaacccgctggtcgagggctatggcgacaccaccccgccggcgattacctggcaaccctttcccaaccggctgtggacgtttttttatagcaacggcacggcggtgattccgcaactgggcggcaaggccatgaccctgcaacaggtcatggaactgaccgacaatggccagatcaccatcaacgacaccctgtacaccctgtacgacccggacaagaaaggcaccctgctgcaactgccggtgacccgttgcccgagtatcgactggaacggcaagtacaaggatttctcaccctcgggcccacggggctggctggacgagtattgcgagtggtcgattgtccgcgatgccaatggcgacatgcgcaaaatcaccttcaccagtgaaaacccggcgtatttcctggccatgtggcgcatcgacccgaatgccgtgctggggctgtatcgcgactacatcgacccgaacgtccaactcgaagacctctacctgcgctatgccaccgactgcccgaccggcaatgccggggatccggtgattgacccgaccacgggcctgcccgcctacgacactgtcaacaaatggaacgccggcaccgcctgtacgcccggccagttcggcggcgcgatgcacctgacgtccggccccaacaccctcagcgccgaggtgtacctggcggcggcggccacgatcatgcggcccctgaaaagcagccagaaccctcagtcgctgatctgctgcgcgcaatatgggcagaactatcgcaactccgacccgcatatcggttttgcggccaatgaggcggccatcagcaaccgtatctccctgaccaatcccatcgccctgtacctgcagcaaccgaccaacttcagcgcgtggaaaggcccgcagggccaggatgtgagtcagtactggcgcattacccgcggcaccgccaaatcggcgatcaacggctccgaccagatcctccaggcggtgttcgaggtgccgcaaagcgcggggttctcgatcaatgacatcaccatcaacggccaggccgtggactatgtgtgggtgattgcccagcaactgctggtgggcctgagtgtgaccgtcatgccgagcaccacggcggcgccgtctccttgcgtacaagaccgggtcaatggcctgcaaccctggccggtgcagttattgccgctggacctgttctacggccagtcgcctaccgacctgccggcctggctggcccctggcagcagcgggcagtttgtcctggtggtgcaaggcgccgatctgcagaccaccgccgccacggcgaggatccagttcagcaatcccggggtgacggcacaggtcacgaagttcatgcccgacgcctcggccattcccggccagaccaacgcgggcggcacccagggttacatcatgaccatcagcgtcgcggcgaacgcggcgccgggactggtgacggtacgcgcgctcaacccgggcgaggcggataacgtcagcgcggcggaccacccgtgggaatccgggctggcgctggtgccatccacctaa

SEQ ID NO: 131 - DNA, 1602 bp, Pseudomonas gessardii
atgatgtccaggtttcgcttgagtcgtctgctgctggtcagcaccctgctgtcactgtttatcctgcccttggcccacgcgtccgatgccgataactgcgtccagcagcaactggtgttcaaccccaagagcggcgggtttatgccggtcaacaacttcaacaccaccggccagagctttatgaattgctttggctggcaattgttcatcgccctgaactggccggtggaccccggctggccggccaatgccagcctggcgggcgagccggacagaaccatcaccgtcgcgcaattcggcgtgcccaccaccgccgggcagcccatgagcgtggcgccggtatgggccagctacaaagacgccaatgagattttcctgcccggtgcacccaagcccagcggttggggggtgcaaaccctggtgccgcccaattgcagcagccaggacagcctccaggccctgtcggtaggggcgcgtaaattcatgaatgccacctcggaaagcgcgaccaacgccaagcatcgcttccacttgtccagcggcaccctggcgtcgattcccgacccgatcatggaagccgccggtggctggctcacggaccagaccggcaacctggtgtatttcgaacgcaaggtgggcaaggccgagttcgactacatcgtcgacaacggtctgtacgatgccgccaatcaactgatcgtcgcgcaaaacagcgatggcaaacacccggccggcctgtcgctgcccgccggtgagctgatgcgctcgatgcccaccaccccgctgccccaggagcaactgggcgccctggaactcaaggccgcctggcgcatcctcaccggccagccccagctctacgggcgctacctgaccactgtggcctggctcaagaaccccgccaccctgcaatgcacccaacaggtggtgggcctggtgggcctgcatatcatcaacaagacccagagctcaccgaactttatctggaccaccttcgagcacgtggacaacgtaccggaaccgggccaggtgcccgcgcaacagctgcccccggacggctacaccttcaacaatcccaactgcaccggcggccccgatgtgtgtacgccgaacgtggcgcgcatccagtgcaaacagcaccacccggatcgcgaatgcaccgaaccctatccacgggaccaaccggtgcagaccacccgcgaacacccactgtcgtcggacatgcaggcgctcaacggcgcagtgcaggcaagcttcgcccaacagaccaacggccagtcggtgttccagtactacaagctgatcaatgtgctgtggatcaccgccccgacgccgcccgaccccgagccgggcccgaatgcgaaggttcccctgtcctacggtgcttttatcagcgacagcaacgtacccgtggccaataccaccctggagacgtacgtccagggcatgaactgcaatgactgccatcagcaagcgaccattgccggcagcgccaccctggcctcggacttctcgttcctgttcaacaacgccgattcggccaagcatacaagcctgatcaaacgcgtacatgccttcgaaaccctcaaggacggccaaccatga

SEQ ID NO: 132 - DNA, 1737 bp, Pseudomonas putida
atgagcgcgcccttcaagcagttcacctctcccgccggccaagcccccaaggactacaacaagctgggcctggaagaccagttgccgcagtttgaaaccgactggaacaacaacctcaccggctggaccgaatcgtcgatcatcggcaacccctggtcgggcctgaacgacgccccccgctcgggttactacaacccgctggtggaaggtttcggcgacgtgaccgccccggcgatcacctgggcgcccttccccaaccggctctggacgttcttctacaacaacggtgcggcggtcattccccagctgggtggcaaggccatgaccctggaccaggtgatggcgttgaccgaccacggccagatcacgctcgacaacaccctctacatgctctacgaccccaacaagcaaggtactgtgctgcaactgccggccaagcgctgcccgagcatcgactggaacggcaagtacacggcgttctcgccttccggcccgcggggctggctcgacgagtactgcgagtggtcgatcgtacgcgatgccaacggcaacatgcgcaagatcaccttcacctgcgaaaaccccgcgtacttcctgaccatgtggcgcatcgacccgaacgcagtgctgggcctgtaccgcgactacatcgacccgaacgtgcaactcgaagacctgtacctgcgctacaccgtcgactgcccgaccggcaaggccggcgacccggtcatcgaccccaccaccggcaagccggcctatgacaccgtcaacaaatggaacgccggaacggcctgtgtgcccggccagtacggcggtgcgatgcacctgacctccggccccaataccctcagcgccgaggtgtacctggccgccgccgccaccatcctgggcccggtgagcagcagtcagaacgcccagtcgttgatctgctgcgcgcagtacgggcaaaactatcgcaactctgatccgcacatcggtttcatggccaataccacggcagtgaacaaccgactgtcgctgaccaaccccattggcctgtacttgcagcagcccaccgatttcagcgcctggaagggcccgcaaggccaggacgtgagccagtactggcgcatcacgcgcggtacggcgaagtcggccgccaatggttccgaccagatcctgcaggcggtgttcgaggtgccggaaagcgccggcttctcgatcaacgacatcaccatcaacaaccagaaggtcaactatgtgtgggtcatcgcccaacaactgctggtcggcctgagcgtcaccgtcaagccgctcagcactgcgcctcaagcgttcccatgcgtgcaggaccgggtggccggcctgcaaccctggccagtgcaactgctgccgctggatctgttctacgggcaatcccccaccgacctgcccgcctggcttgcaccgggtagcagcaaccagttcgtgctggtggtgcaaggtgccgacccgactaccacggcgcagaatgcaagggtgcaattctccaaccctggggtgacggcgcaggtcacccagtacctgcccgacgcatcggccattcctagccagaccaactcgggcggcacccaggcctacattctgaccatcacggtcagcccctccgcagcacccggcctggtggcagtgcgtgccctcaacccgggtgaagatgtgaacgtgagcgcgacagaccacccttgggaatctggcctggcgctggtgcctggcgcctga

SEQ ID NO: 133 - DNA, 1605 bp, Pseudomonas putida
atgtccaggtcacgcttgagtcttctgtcgctgctgtgcggcattctactgtgcctgtcgaccccgcaacccgccacggcggccacgctgtcggacgccgatacctgtgtacagaagcaattggtgttcaacccggccagcgggggattcctgccggtcaacaacttcaatgccaccagccaggcgttcatgaactgctttggctggcagttgttcattgccttgaactggccggtgaaccccggttggccagccaccgccagcctggcgggtgaacccgacatgcaaagcacgctggcgcagttcggggtcccctctgcaccgggtcagcccatgagcgtggccccggtatgggccagctacaaggacgccaacgacatcttcctgcccggcgcacccacgcctaccggctggggcgtggaaaccctggtgccgtccggctgcagcacccagggtagcctcaaggcgctcaaggtgggcgcacgcaagttcatgaacgccacctccgaaggcgcgatcaatgccttgcacggtttccacctgtcgaccgggacacttgcgtccattcccgacccggtcatggaggcgtccggcggctggctgacggaccaggcgggcaaactggtattttttgagcgcaaggtgggcaaggccgagttcgactacatcgtcgacaaggggctctacgacgctgccaaccagttgaaggtcgcgcaaaacctcgacggccagacaccggagggcctgtcgctgcccatcggcgaaccgatgcgctcactgccgacctccccagtgccacaggagcaactgggcgcgatcgagctcaaggccgcctggcgggtgctgaccggcaaacccgagctgttcgggcgctacctgactaccgtcgcctggctcaaacgccccgacacgctggagtgcacccaggaggtggtggggctggtgggcctgcatatcatcaacaagacccaggcttcgcccaacttcatctggaccaccttcgagcaggtggacaacgtgcccgaaccggcccaggtcccgccgcaacaaaccccgccaaacgggtttgccttcaacaaccctgactgtggcgacggccccgagtgcacaccgaaccaagcccgtatccagtgcaagcaaacgcatcccgacaaggactgcaccgatctcttcccacgcgaccagccggtacagaccacccgcgtacaccccgtgcccggcgacctgcaagccctcaacagcgcggtacaagccaacttcgcgcagcacagccaaggcaagtcggtgtttcagtactacaagctgatcaacgtactctggaccctcgcccccaatccgcccagcccggaaccgggcgccaacgcgcaagtgccgctgtcgtacgggccgttcatcagccagggcaacgtgccggtggccaacaccaccatggagacctacgtgcagggtgatgactgcaatcagtgccatcagtacgcgacgattgccggcagcccgtcattggcctcggatttctctttcctgttcaacagtgccggctccgccagcaacaaaagcctgatcaaaagcgtcaaagccttcgaaaccctcaaggaccgcccctga

SEQ ID NO: 134 - DNA, 1737 bp, Pseudomonas plecoglossicida
atgagcacgcccttcaagcagttcacctctcccgccggccaagcccccaaggactacaacaagctgggcctggaagaccagttgccgcagtttgaaaccgactggaacaacaacctcaccggctggaccgaatcgtccatcatcggcaacccttggtcgggcctgaacgacgccccccgctcgggttactacaacccgctggtggaaggcttcggcgacgtgaccgccccggcgatcacctgggcgcccttccccaaccggctctggaccttcttctacaacaacggtgcggcggtcattccccagttgggtggcaaggccatgaccctggaccaggtgatggagttgaccgaccacggccagatcaccctcgacaacaccctctacatgctctacgaccccaacaaacgaggtaccgtgctgcaactgccggccaagcgctgcccgagcatcgactggaacggcaagtacacggcgttctcgccttccggcccacggggctggctcgacgagtactgcgagtggtcgatcgtgcgcgatgccaacggcaacatgcgcaagatcaccttcacctgcgaaaaccccgcgtacttcctgaccatgtggcgtatcgacccgaacgcagtattgggcctgtaccgcgactacatcgacccgaacgtgcaactcgaagacctgtacctgcgctacaccgccgacggcccgaccggcaaggccggtgacccggtcatcgaccccaccaccggcaagccggcctatgacaccgtcaacaaatggaacgccggaacggcctgtgtgcccggccagttcggcggtgcgatgcacctgacctccggccccaataccctcagcgccgaggtgtacctggccgccgccgccaccatcctgcgcccggtgagcagcagccagaacgcccagtcgttgatctgctgcgcgcagtacgggcagaactatcgcaactctgatccgcacatcggtttcatggccaataccacggcggtgaacaaccgactgtcgctgaccaaccccattggcctgtacttgcaacagcccaccgacttcagcgcctggaagggcccgcaaggccaggacgtgagccagtactggcgcatcacgcgtggtacggccaagtcggctgccaacggttccgaccagatcctgcaggcggtgttcgaggtgccggaaagcgccggcttctcgatcaatgacatcaccatcaacaaccagaaggtcaactatgtgtgggtcatcgcccaacaactgctggtcggcctgagcgtcaccgtcaagccgctcagcaccacgcctcaagcgttcccatgcgtgcaggaccgggtggccggcctgcaaccctggccagtgcagctgctgccgctggacctgttctacgggcaatccccaaccgacctgcccgcctggcttgcaccgggcagcagcaaccagttcgtgctggtggtgcaaggcgccgacccgactaccacggcgcagaatgccagggtgcaattctccaaccctggggtgacggcgcaggtcacccagtacctgcccgacgcgtcggccattcccggccagaccaactcgggcggcacccaggcctacattctgaccatcacggtcagcccctccgcagcacccggcctggtgacagtgcgtgccctcaacccgggtgaagatgtgaacgtgagcgcgacagaccatccttgggaatctggcctggcgctggtgccgggggcctga

SEQ ID NO: 135 - DNA, 1605 bp, Pseudomonas plecoglossicida
atgtccaggtcacgcttgagtcttctgtcgctgctgtgcggcattctgctgtgcctgtcgaccctgcaacccgccacggcggccacgctgtcggacgccgatacctgtgtgcagcagcaattggtgttcaacccggccagcgggggattcctgccggtcaacaacttcaatgccaccagccaggcgttcatgaactgctttggctggcagctgttcattgccttgaactggccggtgaaccccggttggccggccaccgccagcctggcgggcgaacccgacatgcaaagcacgctggcgcagttcggggtcccctccgcaccgggtcaacccatgagcgtggccccggtatgggccagctacaaggacgccaacgacatcttcctgcccggcgcacccacgcccaccggctggggcgtgcaaaccctggtgccatccggctgcagcacccagggtagcctcaaggcactcaaggtcggcgcacgcaagttcatgaacgccacctccgaaggcgcgatcaatgccttgcacggtttccacctgtcgaccgggacacttgcgtccattcccgacccggtcatggaggcgtccggcggctggctgacggaccaggcgggcaaactggtgtttttcgaacgcaaggtgggcaaggccgagttcgactacatcgtcgacaaggggctctacgacgccgccaaccagttgaaggtcgcgcaaaacctcgacggccagacaccggagggcctgtcgctgcccatcggcgaaccgatgcgctcactgccgacctccccagtgccacaggagcaactgggcgcgatcgagctcaaggctgcctggcgggtactgaccgacaaacccgagctgttcgggcgctacctgactaccgtcgcctggctcaaacgccccgacacgctggagtgtacccaggaggtggtggggctggtgggcctgcatatcatcaacaagacccaggcttcgcccaacttcatctggaccaccttcgagcaggtggacaacgtgcccgaaccggcccaggtcccgccgcaacaaaccccgccgaacgggtttgccttcaacaaccctgactgtggcaacggccccgagtgcacaccaaaccaagcccgtatccagtgcaagcaaacgcatcccgacaaggactgcaccgatctcttcccacgcgaccagccggtacagaccacccgcgaacaccccgtgcccggcgacctgcaagccctcaacagcgcggtacaagccaacttcgcgcagcacagccaaggcaagtcggtgttccagtactacaagctgatcaacgtactctggaccctcgcccccaatccgcccagcccggaaccgggcgccaacgcgcaagtgccgttgtcgtacgggccgttcatcagccagggcaatgtgccggtggccaacaccaccatggagacctacgtgcagggtgacgactgcaaccagtgccatcagtacgcgacgattgccggcagcccctcgttggcctcggacttctccttcctgttcaacagtgccggctccgccagcaacaaaagcctgatcaaaagcgtcaaagccttcgaaaccctcaaggaccgcccctga

SEQ ID NO: 136 - DNA, 1737 bp, Pseudomonas putida
atgagcacgcccttcaagcagttcacctctcccgccggccaagcccccaaggactacaacaagctgggcctggaagaccagttgccgcagtttgaaaccgactggaacaacaacctcaccggctggaccgaatcgtcgatcatcggcaacccctggtcgggcctgaacgacgccccccgctcgggttactacaacccgctggtggaaggtttcggcgacgtgaccgccccggcgatcacctgggcgcccttccccaaccggctctggacgttcttctacaacaacggtgcggcggtcattccccagctgggtggcaaggccatgaccctggaccaggtgatggcgttgaccgaccacggccagatcacgctcgacaacaccctctacatgctctacgaccccaacaagcaaggtactgtgctgcaactgccggccaagcgctgcccgagcatcgactggaacggcaagtacacggcgttctcgccttccggcccgcggggctggctcgacgagtactgcgagtggtcgatcgtacgcgatgccaacggcaacatgcgcaagatcaccttcacctgcgaaaaccccgcgtacttcctgaccatgtggcgcatcgacccgaacgcagtgctgggcctgtaccgcgactacatcgacccgaacgtgcaactcgaagacctgtacctgcgctacaccgtcgactgcccgaccggcaaggccggcgacccggtcatcgaccccaccaccggcaagccggcctatgacaccgtcaacaaatggaacgccggaacggcctgtgtgcccggccagtacggcggtgcgatgcacctgacctccggccccaataccctcagcgccgaggtgtacctggccgccgccgccaccatcctgcgcccggtgagcagcagtcagaacgcccagtcgttgatctgctgcgcgcagtacgggcaaaactatcgcaactctgatccgcacatcggtttcatggccaataccacggcagtgaacaaccgactgtcgctgaccaaccccattggcctgtacttgcagcagcccaccgatttcagcgcctggaagggcccgcaaggccaggacgtgagccagtactggcgcatcacgcgcggtacggcgaagtcggccgccaatggttccgaccagatcctgcaggcggtgttcgaggtgccggaaagcgccggcttctcgatcaacgacatcaccatcaacaaccagaaggtcaactatgtgtgggtcatcgcccaacaactgctggtcggcctgagcgtcaccgtcaagccgctcagcactgcgcctcaagcgttcccatgcgtgcaggaccgggtggccggcctgcaaccctggccagtgcaactgctgccgctggatctgttctacgggcaatcccccaccgacctgcccgcctggcttgcaccgggtagcagcaaccagttcgtgctggtggtgcaaggtgccgacccgactaccacggcgcagaatgcaagggtgcaattctccaaccctggggtgacggcgcaggtcacccagtacctgcccgacgcatcggccattcctggccagaccaactcgggcggcacccaggcctacattctgaccatcacggtcagcccctccgcagcacccggcctggtggcagtgcgtgccctcaacccgggtgaagatgtgaacgtgagcgcgacagaccacccttgggaatctggcctggcgctggtgcctggcgcctga

SEQ ID NO: 137 - DNA, 1605 bp, Pseudomonas putida
atgtccaggtcacgcttgagtcttctgtcgctgctgtgcggcattctactgtgcctgtcgaccccgcaacccgccacggcggccacgctgtcggacgccgatacctgtgtacagaagcaattggtgttcaacccggccagcgggggattcctgccggtcaacaacttcaatgccaccagccaggcgttcatgaactgctttggctggcagttgttcattgccttgaactggccggtgaaccccggttggccggccaccgccagcctggcgggcgaacccgacatgcaaagcacgctggcgcagttcggggtcccctccacaccgggtcaacccatgagcgtggccccggtatgggccagctacaaggacgccaacgacatcttcctgcccggcgcccccacgcccaccggctggggcgtgcaaaccctggtaccgtccgactgcagcacccaaggtagcctcaagacactcaaggtgggcgcgcgcaagttcatgaacgccacctccgaaggcgcgatcaatgccttgcacggtttccacctgtcgaccgggacacttgcctccattcccgacccggtcatggaagcgtccggcggctggctgacggaccaggcgggcaaactggtgttttttgaacgcaaggtgggcaaggccgagttcgactacatcgtcgacaaggggctctacgacgccgccaaccaattgaaggtcgcgcgaaacctcgacggccagacaccggagggtctgtcactgcccatcggcgaaccgatgcgctcactgcctacctccccagtgccacaggagcaactgggcgcgatcgagctcaaggccgcctggcgggtactgactggcaaacccgagctgttcgggcgctacctgactaccgtcgcctggctcaaacgtcccgacacgctggagtgcacccaggaggtggtggggctggtgggcctgcatatcatcaacaagacccaggcttcgcccaacttcatctggaccaccttcgagcaggtggacaacgtgcccgaaccggcccaggttccgccgcaacaaaccccgccaaacgggtttgccttcaacaaccctgactgtggcaacggccccgagtgcacaccaaaccaagcccgtatccagtgcaagcaaacgcatcccgacaaggactgcaccgatctcttcccgcgcgaccagccggtacagaccacccgcgaacaccccgtgcccggcgacctgcaagccctcaacagcgcggtacaagccaacttcgcgcagcacagccaaggcaagtcggtgttccagtactacaagctggtcaacgtactctggaccctcgctcccaacccgcccagcccggaaccgggcgccaacgcgcaagtgccgctgtcgtacgggccgttcatcagccaggggaacgtgccggtggccaacaccaccatggagacctacgtgcagggtgataactgcaatcagtgccatcagtacgcgacgattgccggcagcccgtcattggcctcggatttctcttttctgttcaacagtgccggctccgccagcaacaaaagtctgatcaaaagcgtcaaagccttcgaaaccctcaaggaccgcccctga

SEQ ID NO: 138 - DNA, 1737 bp, Pseudomonas putida
atgagcacgcccttcaagcagttcacctcgcccgccggccaagcccccaaggactacaacaagctgggcctagaagaccagctgccgcagttcgaaaccgactggaacaacaacctcaccggctggaccgagtcgtcgatcatcggcaacccctggtcgggcctgaacgatgcgccccgctcgggttactacaacccgctggtggaaggcttcggcgacgtgaccccgccggcaatcacctgggcgcctttccccaaccgactgtggacgttcttctacaacaatggcacggcggtcattccgcagctgggtggcaaggccatgaccctggaccaggtgatggagttggccgaccatggccagatcagcctcgacaacaccgtctacaggctctatgacccgaacaagcaaggcaacctgctgcaactgccggccaagcgctgcccgagcatcgcctggaacggcccgtacaaggatttctcgccttccggcccacggggctggctcgacgaatactgcgagtggtccatcgtgcgcgatggcaacggcaaaatgcgcaagatcaccttcacctgtgaaaacccggcgtatttcctgaccatgtggcgcatcgacccgaatgcggtgctgggcctgtaccgcgaatacatcgacccgaacgtgcagctcgaagacctgtacctgcgctataccgaagacggcccgaccggcaaggccggtgagccggtcatcgatcccaccaccggcaagccggcgtacgacaccgtcaacaaatggaatgccggcacggtcagtgtgcccggccagtatggcggggcaatgcacctgacctccggccccaataccctcagtgccgaggtgtacctcgccgccgccgccaccatcctgcgaccggtcagcagcagccagaacgcccagtcgctgatctgctgcgcgcagtacgggcagaactaccgcaactccgacccgcacatcggtttcatggccaacagcacggcggtgaacaaccgcctgtcgctgaccaacccgattggcctgtacttgcaacaacccaccgacttcagtacctggaagggcccgcaaggccaggatgtgagccagtactggcatatcacgcgcggcgcggccaagtccgcggccaacggttccgaccagatccttcaggcggtgttcgaaataccggaaagcgccggtttctcgatcaacgaggtcaccatcaacaaacaaccggtcaaccatgtgtgggtcatcgcccaacagttgctggtgggcctgagcgtcaccgtcaagccactcgccgccacgcctgcttcctacccctgcgtgcaggaccgggtggcaggcctgcaaccctggccggtgcagctgctgccgttggacctgttctacggcaactcacccaccgacctgcccgcctggcttgccccgggcagcagcaaccaattcgtgctggtggtgcaaggcgccgacgagaacaccaccgcagagaacgcccgggtgcaattctccaaccccggggttaccgcgcaggtcacccagtacctgcccgacgcaacggccatacccggccagaccaataccggcggcacccaggcttacatcctgacgatcacggtcagccccactgccgcacccggcctggtgacggtacgtgcgctcaacccggacgaagacgccaacgtgagcgcggcagaccacccttgggaatccggcctggcgctggtgcctggcgcctga

SEQ ID NO: 139 - DNA, 1605 bp, Pseudomonas putida
atgtccagcctacgcttgagtcttctgtcgctgctaagcggcattctcctgtgcctgtccgcccagcaaacagccacggcggccacgcagtccgacgccgatagctgtgtgcagcagcaactggtgttcaacccggccagtggcgggttcctgccggtcaacaacttcaatgccaccagccaggcgttcatgaactgctttgcctggcagttgttcattgccctgaactggccggtgaacctcggttggccaggcactgccagcctggccggggaacccgacctgaacagcagcctggcgcagttcggggtacctgccacaccgggtcaacccatgagcgtggcgccggtgtgggccagctacaaggacgccaacgacatcttcctgcccggcgcacccacgcccagcggctggggcgtgcaaaccctggtaccggccaattgcagcacccagggcagcctcaaggcactcaaggtcggcgcgcgcaagttcatgaacgcaacctccaagagcgcgatcaacgtcttgcacggtttccacctgtccagcgggacgctggcatccagccccgacccgttcatggaggcgtctggcggctggctgacagaccagtcgggcaacctggtgtttttcgaacgcaaggtgggcaaggccgaattcgactacatcgtcgacaacggcctctacgacgcggccaaccagctgaaggtcgcgcaaaaccaggacggcaagtccccggcggggctgtcgctgcccgccggcgaaccgatgcgctccctgcctgccgccccggtcccgcaggagcaactgggggcgatcgaagtcaaagccgcctggcgggtgctgaccggcaaacccgagctgttcgggcgctacctgaccaccgtcgcctggctcaaacgccccgacacgctggcctgcacccaggaagtggttggcctggtgggcctgcatatcatcaacaagacccaggcttcgcccaacttcatctggaccaccttcgagcaggtggacaacgtgcccgaaccggcccaggccccgccgcaacaaaccccgccgaacgggtttgccttcaacaaccccgactgtggcagcggccccgagtgcacaccgaaccaggcccgtatccagtgcaagcaacaccaccccgacaaggactgcaccgatcgcttcccacgcgaccagccggtacagaccacccgcgaacaccccgtgcccggcgacctgcaagcgctcaacagcgcggtacaagccaacttcgcgcagcacagccaaggccagtcggtgttccagtactacaagctgatcaacgtactctggaccctcgcccccaatccgcccagcccggaaccgggcgccaacgcgcaagtgccgctgtcatacgggccgttcataagccagggcaacgtgccggtggccaataccaccctggagacctatgtacagggtgatgactgcaaccagtgccaccagtacgcgacgattgccggcagcccgtcgttggcctcggacttctctttcctgttcaacagtgccgattccgccagcaacaaaagcctgatcaaaagcgtcaaagccttcgaaaccctcaaggacctcccctga

SEQ ID NO: 140 - DNA, 1737 bp, Pseudomonas monteilii
atgagcacgcccttcaaccagttcacttctcccgccgaacaagcacccaaggactacaacaagctgggcctggaaaaccagctgccgcagttcgagagcgactggaacaactacctcaccggctggaccgaatcgtccatcatcggcaacccgtggtcgagcctgtacgacgcgccgcgctcgggctactacaacccgctggtggaaggtttcggtgatgtggttgtgccggcgatcacctgggcgcccttccccaaccggctatggacgttcttttacaacaacggtgccgcagtcattccccagctgggtggcaaagccatgaccctgcaacaggtgatggagctggccgactacggccagatcaccctcaacgacaccctctacacgctgtacgacccggacaacaaaggcaccctgctgcaactgccggccaaacgctgccccagcatcgactggaacggcaagtacaccgcgttctcgccctccggcccacgcggctggcttgatgaatactgcgagtggtcgatcgtgcgcgacgccaacggcaacatgcgcaagattaccttcacctgcgaaaacccggcgtactacctggccatgtggcgcatcgacccgaacgccgtgctgggcctgtaccgtgaatacatcgaccccaacgtgcagctcgaagacctgtacctgcgctacaccgtcgattgcccgaccggcaaggctggcgacccggtcatcgaccccaccaccggcctgccggcctatgacacggtgaacaagtggaatgccggcacggcctgtgtgcccggccaatttggcggggccatgcacctgacctcaggccccaacaccctcagcgccgaggtgtacctggccgccgccgctaccatcctgcgcccggtgaccagcagccagaacgcccagtcgctgatctgctgcgcccagtatgggcagaactatcgcaactccgacccgcacatcggtttcatggccaattccaaggcagtgaacaaccgcttgtcactgaccaatccgattggcctgtacctgcagcagcccaccgacttcagcacctggaaaggcccgcaaggccaggatgtgagccagtattggcgggttacgcgcggcactgccaagtcggccgccaacggctccgaccaaatcctccaggccgtgttcgaagtgccggaaagcgcaggcttctcgatcaacgagatcacgatcaacaagcaaccggttgactatgtgtgggtcatcgcccaacaactgctggtgggcctgagcgtcagtgctctaccgcccgccaccacccctccatccttcccctgcgtgcaggaccgggtgacgggcctgcagccctggccggtgcagttgctgccgctggacctgttctacggccagtcacccaccgacctgccggcctgtcttgcgccgggcagcagcaaccagttcgtgctggtggtacaaggcgccgacccgaacaccacggcgcagagtgccagggtgcagttctccaaccctggcatcagcgcgcaggtcacccagttcctgcctgacgcctcagccattcccgggcagaccaatgcgggcggcacccaggcctacatcctgaccatcacggtcagccccagcgccgcccccggcctggtgacggtgcgtgccctcaatccgggcgaagacgggaacgtgagcgcagcagaccacccgtgggaatccggcctggcgctggtacctggcgcctga

SEQ ID NO: 141 - DNA, 1605 bp, Pseudomonas monteilii
atgtccaggttacgcttgagtcttctgtcgctactaagcggcatgctgctgtgcctgtcgaccctgccagccgccacggcggcgccaatgacggaggccgacgcctgtgtacagcaacagttggtgttcaacccggccagcggcgggttcctgccggtcaacaacttcaatgccagcaaccaggcgttcatgaactgttttgcctggcagctgttcattgccctgaactggccggtgaatcccggctggccagccaccgccagcctggccggcgaacccgacatgaacagcaccctggcgcagttcggtgtgccctccgacccggggcaaccgatgagcgtggcgccggtgtgggccagctacaaggacgccaacgacatcttcctgcccggcgcccccaagcccagcggctggggcgtgcaaaccctggtgccatccggttgcggcacccagggcagcctcaaggcgctcaaggtgggggcacgcaagttcatgaacgccacctccgaaagcgcgatcaacgccgtgcacggtttccacctgtccagcgggacgctcgcatcccttcccgactcgatcatggaagcatccggtggctggctgaccgaccaggcgggcaacctggtgttcttcgagcgcaaggtgggcaaggccgagttcgactacatcgtcggcaaggggctgtacgacgccgccaaccagttgaaggtcgcgcaaaacgccgacggcactacaccggaggggttgtcgttgcccattggcgagccgatgcgctcgctgccgccatccccggtgccgcaggaacaactcggcgcgatcgaactcaaggccgcctggcgcatactgaccggcaaacccgaactgttcgggcgctacctgaccaccgtcgcctggctcaagcgccccgacacgctgacgtgtacccaggaagtggtggggctggtgggcctgcatatcatcaacaagacccaggcctcgccgaacttcatctggaccactttcgagcaggtcgacaacgtgcccgagccgggtcaggtaccgccgcaacaaaccccgccgaacggcttcgccttcaacaacccggactgcggcagcggccctgagtgtgaaccgaaccagccccgtatccaatgcaagcaacaccaccccgaccgggactgcaccgatctgttcccacgcgaccagccagtgcagaccacgcgcgagcatcctgtgccgagcgacctgcaagcgctgaacggcgcagtgcaagccaccttcgcgcagcacagccagggcaagtcggtgttccagtactacaaactgatcaacgtactctggaccctcgcgcccaacccgcccagcccggaaccaggagccaacgcgccggtgccgttgtcgtacggggcgtacatcagccagggcaatgtgccggtggccaacaccaccctggaaacctatgtgcagggtgatgactgcaaccagtgccatcagtacgcgacgattgccggcagcagttcgctggcctcggacttctcgttcctgttcaacagtgccagctcagccagcaagcacagcctgatcaagcgtgtccaagccttcgaaacgctgaaggaccgtcgctga

SEQ ID NO: 142 - DNA, 1734 bp, Pseudomonas poae
atgagcacacccttcacccaattcacctcccctgccgaacaagcgcccaaggactacaacaagttgggcctggaggaccagttgccggcgttcgaaaccgactggaacaacaacgtcaccggctggacccagatgtcgatcatcggcaacccctggtccaacctcaacgatgcaccgcgctcgggctattacaacccgctggagagcggctacggcacgctgacgccaaagaccatcacctggcagcccttccccaatcggctgtggacgtttttctataacgagggcgctgccgtggtcccgcaactgggcggcaaggccatgaccctggaccaggtgatgcaactgaccgaccacggccagatcaccctcaacgacaccctctattcgctgtacccggaccccaaggccacccaactgcagatccccagcgtgctgtgcaaatccatcaactggaacggcccctacgccgacttttcgccctcgggtccacggggctggctggacgaatactgcgagtggtcgatcacccgcgaccccgacggcaacatgcgcagcatcatgttcaccagcgagaacccggcgtatttcctgaccatgtggaacatcgacccgggtgccgtgctgggcctgtaccaggcgtatgtcgacccgcaggtgaaactcgaagacctgtacctgcgctacaccgccgacggcccgaccggcaaggccggcgaaccggtactcgaccccaccaccggccagcccgcctacgacaccgtgaacaaatggaacagcggcaccgtgcgcataccgggcgtatcgggcggcgcgatgcacctgacttccggccccaataccctgagtgccgagatctacctggcggcggcggccaccatcctgcggccactcaccagcagccagaaccagcagagcctgatctgctgcgcgcaatacgggcagaactaccgcaactccgacccgcatatcgggttctccgcgaaccaggcggcggtcaacaacctgatctcgttgaccaaccctatcggcctgtacctgcagcaacccaagtccttcagcacctggaagggcccgcaaggccaggatgtcagcagctactggcgcgttacccgtggcaccgccggcaccggcccgaacaactccgaccagattctccaggcggtcttcgaggtgccggccagcgcggggttctcgatcaatgagatcaccatcaacggcacgccgatcgactacgtgtgggtgatcgccaacgaactgaacgtggccctcagcgtgacccctgcgccgctcacggcccagcccaaggagtgtgcctgcgtggcggccaacaccaccgatgcgcaaccctggcccgtgcagttgctgccgattgacctgttctacggccaatcccccagcgacttgccggccagttttgcccccggcagctcaggccagttcgtattggtggtacaaggcgccgacccgaacaccacggcggcggatgcacgggtgcagttctccaacccgggcatcacggcccaggtcacgcagttcctgccggatgcctcggcgattcccggccagaccgacggcggcggcacccagggctacatcatgaccatcaccgtcagcagcaacgcggcgccggggctggtcagtgtgcgtgcgctgaaccccagcgaagcggccaacccgagtgcctccgagcacccctgggaaagcggcctggccctggtgcccagcgcctga

SEQ ID NO: 143 - DNA, 1587 bp, Pseudomonas poae
atgaacggatggcttcgcccgctgcgccgggcacgcttgcgtattgcctgcgcaatcacctgcacccttctcccactgctggccgccacaccggccaatgccgcctcggacgcccagagctgcgtcagccagctggtgttcgatcccaccagcggcggcttcctgccggtgaacaatttcggcaccgagcaggcttttctcaattgtttcggctggcagttgttcatcgccatgaactggccggtcaatcccggctggccggccaacccaagcctggccggtgagccggacacccaaagcagcgcggcccagttcggcgtgccgccaacccccggccaaccgatgagcaatgccccggtgtgggccagctacaaggatgccagcgaaatcttcctgcccggcgcggccaagccgtccggctggggcgtggaaaccctggtgccgtccaattgcaccgccaccggcaacctcaaggcgtttgccacgggggcgcgtaaattcatcaccgccacctcggaaagcgcgatcaaccgcaagcaccgcttccacctgtccagcggcacccaggtgaccctgccggattcgatcatggaagcgtccggcggctggctcacggaccagtcgggcaacctggtgtttttcgagcgcaaggtgggcaaggccgagttcgactacatcgtcgacaacggtttgtacgacgccgccaaccaactgatcgtggcgcaaaacagcgacaaccgacaccccgccggcctgtcactgccggccggcaagccggtgcgcgagctgccagccaaggcgctaccccaggaggagctgggtgccctggaactcaaggcggcctggcgcgtgctcaccaacaagcccgacttgtacgggcgctacctgaccaccgtggcctggctgcaacgcccggacacgctgcaatgcacccaggaagtgataggcctggtagggctgcatatcatcaacaagacccagacccagccgaacttcatctggaccaccttcgagcagatcgacaacgtgcccgatggcggcgccgccccaccccagggctacagcttcaacaaccccgagtgcaccggcgatgcctgcgcgccaaacgtcgcccgcgtgcagtgcgacgccacccacacgccgcccgactgcacgcccctggaccagccggtgcaggccacccggctcaacgccacgccccaggacatgcaggcgctgaacacggcggtgcagcagaccttcgcccagcagacccagggccagtcggtgttccagtactacaaactggtgaacgtgctgtggtccaagacgcccaacgcccccaacgatccaggccctgggccgaacgtgaaggtgccgctgtcctatgggccgtttgtcagcgaccagagtgtcgtggtcgccaacaccacgatggaaacctacgtgcagacagacaactgcaatgactgccaccagtacgcggcgattgccggcaaatccgggctggcgtcggacttctcgttcctgttcggcaatgccgactcggcgaaaaatacgcggctgatcaaacgcatcgagtcgttcaagaccctcaaggacaacccg

SEQ ID NO: 144 - DNA, 1734 bp, unknown
  Mountain Pine Beetle microbial communities
atgagcacgcccttcacccaattcacctcccctgccgaacaagcccccaaggactacaacaagctgggcctggagaaccaactgcccaccttcgaaaccaactggaacaacaacgtcaccggctggacccagatgtcggtgatcggcaacccgtggtccaacctcaacgacgcaccgcgctcgggctactacaacccgctggagagcggctacggcacgcagacgccagtgaccatcacctggcagcccttccccaatcggctgtggacgttcttctacaacaacggcgccgccgtggtcccgcaactgggcggcaaggccatgaccctggaccaggtgatgcagttgactgaccatggccagatcaccctgaacaacaccctctattcgctgtacccggaccccaaggcaacccaactgcagatccccagcgtgctgtgcaagtccatcaactggaacggtccttacgccgacttttcaccctcgggcccacggggctggctggatgaatactgcgagtggtcgatcacccgcgatcccgacggcaacatgcgcagcatcatgttcaccagcgagaacccggcgtacttcctgaccatgtggaacatcgatccgcaggccgtgctggggttgtacaaggcgtatgtcgacccgcaagtgaagatcgaagacctgtacctgcgctacaccgccaacggcccgaccggccaggccggcgaaccggtgctcgaccccaccaccggccagcccgcctatgacacggtgaacaaatggaacagcggcaccgtgcgtatcccaggggtgtcgggcggcgccatgcacctgacctccgggcccaataccctgagtgctgagatctacctggcggcggccgccactatcctgcggccgctcaacagcagccgtaaccagcagagcctgatctgctgcgcgcagtacgggcagaactatcgcaactccgacccgcatatcggcttttccgccaaccaggcggcggtcaacaacctgatctcattgaccaaccccatcggcctgtacctgcaacagccgaaatccttcagcacctggaaaggcccgcaaggccaggatgtcagcagctactggcgcgtcacccgtggcacggccggcaccggtccaaacaactccgaccagatcctgcaggcggtgttcgaggtgccacaaagcgcggggttctcgatcaatgacattaccatcaacggcacgccgatcgactacgtgtgggtgatcgccaatgaattgaatgtggccctgagcgtcaccccggcgccgctccccgcaccgcccaaggaatgcgattgcgtggcggccaacaacaccgatgcgcaaccctggccggtgcagttgctgccgatcgacctgttctacggccagtctcccagcgacttgccggccagctttgcccccggcagttccggccagttcgtgctggtggtgcaaggcgccgacccgaacaccacggcggcggatgcgcgggtgcagttttccaacccagggattaccgcccaggtcacccagttcttgccggatgcgtcggccattccagggcagaccgacagcggcggcacccagggctacatcatgacggtcaccgtcagcagcaacgcggcaccggggctggtcagcgtgcgtgcgctgaaccccagcgaaggcgccaacccgagtgccacccagcacccatgggaaagcggcctggccctggtgcccgacgcctga

SEQ ID NO: 145 - DNA, 1590 bp, unknown
  Mountain Pine Beetle microbial communities
atgaacggatggcttcgcccgctgcgtcgggcacgcttgcgtgtgttctgctggatcacctgcgcccttctcccactgctggccccgtcaccggccaatgcggctaccgatgcccagagctgcgtcagccagctggtgttcgaccccaccagcggcggcttcctgccggtgaataacttcggcaccgagcaggactttctcaattgtttcggctggcagctgttcatcgccatgaactggcccgtcaaccctggctggccggccaacgcgagcctggccggcgagccggacacccaaagcagcgtggcccaattcggcgtgccggcaacacccggccagccaatgagcaacgccccggtgtgggccagctataaggatgccagcgagatcttcctgcctggtgcgcccaaaccctctggctggggcttggaaaccctggtgccgtccaattgcaccgccagcggcaacctcaaggcctatgccaccggcgcacgtaagttcatcaccgccacctcggaaagcgcgatcaaccgcaagcaccgtttccacctgtccagcggcacccaggtgaccctgccggactcgatcatggaagcctccggcggctggctgacggaccagtcgggcaacctggtgtttttcgagcgcaaggtcggcaaagccgagttcgactacatcgtcgataacgggctgtacgacgctgccaaccaattgatcgtggcgcagaacagcgacaaccggcaccccgccgggctgtccttgcccgccggcaaactggtgcgtgaactgccagcccaggcactgccccaagaggaattgggcgccctggagctgaaggcggcctggcgcgtactcaccaacaagcccgaattgtacgggcgctacctgaccaccgtcgcgtggctgcaacgcccggacacgctgcagtgcacccaggaagtggtgggcctggtgggcctgcatatcatcaacaagacccagacccagccgaacttcatctggaccaccttcgagcaggtcgacaacgtgcccgacgccggcccgacaccgccccaaggctacagcttcaacaacccggcatgcagcggcactgcctgcacgcccaacgtcgcccgcgtgcagtgcgacgccacccacgccccgcccaactgcacgcccctggatcagccggtgcaggccacgcgggtcaatgccacgccccaggacctgcaggccttgaatacggctgtacagcaaaccttcgcccagaaaacccagggccagtcggtgttccagtactacaaactggtgaatgtgctgtggtccaagacgcccaatgcgcccaacgatccaggccctgggcccaacgtgaaaacgccgctgtcctacgggccgtttgtcagcgaccagagcgtcgtcgtcgccaataccacgatggaaacctacgtgcaggcagacaactgcaacgactgtcaccagtacgcggcgattgccggcaagtcgggcctggcatcagacttttcgttcctgttcggcaatgccgattcggcgaagaacacccgcctgatcaaacgcatcgaggggttcaagaccctcaaggatgatcaatag

SEQ ID NO: 146 - DNA, 1734 bp, Pseudomonas trivialis
atgagcacgcccttcacccaattcacctcccctgccgaacaagcgcccaaggactacaacaagctgggcctggaggaccagctatcgaccttcgaaaccaattggaacaacaacgtcaccggctggacccaaatgtcggtcatcggcaacccctggtcgaacctcaatgacgcaccgcgttcgggctactacaacccgctggaaagcggctacggcacgcagacaccgctgaccattacctggcagcccttccccaatcgactgtggacgtttttctacaacaatggcgccgccgtggttccgcaactgggcggcacggccatgaccctggaccaggtgatgcagttgaccgatcacggccagatcacccttaacaacacgctttattcgctgtacccggacccggcggcaacccaactgcagatccccaaagtgttgtgcaagtccatcaactggcacggcccctatgccgatttttcgccctcgggtccacggggctggctggatgagtattgcgagtggtccatcacccgcgaccccgacggcaacatgcgcagcatcatgttcaccagcgagaacccggcctacttcctgaccatgtggaacatcgacccaaatgccgtgctggggctgtaccaggcgtacgtcgacccgcaggtgaaactcgaagacctgtacctgcgctacaccgccaacggcccgaccggcaatgccggtgacccggtgatcgatgaaaccaccgggcggcccgcctatgacaccgtcaacaaatggaacgccggcaccgtgcgtataccgggcgtctcaggcggcgcgatgcacctgacctccgggcccaacaccctgagtgccgagatctacctggcggccgcggctaccatccttcggccgatccaaagcagcggcaaccaacagaacctgatctgttgcgctcaatacgggcagaactatcgcaactccgacccgcatatcggcttttccgccaaccaggctgcggttaaaaacctgatctcgttgaccaatcccatcggcctgtacctgcaacagccgaaatccttcagcacctggaaaggccctcaaggccaggatgtgagcagctactggcgcgtcacccgtggcactgccggcaccggcccgaacaactccgaccagatcttgcaggcggtgttcgaggtgccgcaaagcgcggggttctcgatcaatgacatcaccatcaacggcacaccgatcgactacgtgtgggtgattgccaacgaattgaatgtcgccttgagcgtgacgccagcaccgttgaccgccacgcccaaggaatgcgattgcgtggccgccaataacaccgatgcccaaccctggcccgtgcaactgctgccattggacctgttctacggccagtcacccagtgacttgccggccagttttgcacccggcagctcagctcagttcgtgctggtggtgcaaggggcagacccgaacaccaccgtggcggatgcgcgggtgcagttttccaacccggggatcagcgcccaggtcacgcagttcttgccggatgcctcggcgattcccgggcagaccgacagtggcggcacgcaaggctacgtcatgaccgtcaacgtcagcggcaacgctgcgccggggctggtcagcgtgcgggcgctgaaccccagcgaagccgccaaccccagcgcggcccaacacccatgggaaagcggccttgcgctggtgccaggcgcctga

SEQ ID NO: 147 - DNA, 1587 bp, Pseudomonas trivialis
atgtacggatggcctcgcccgctgtgtcgggctcgcttgaatgttttctcgttactggccggcgccctgctgtcactggtggcgccgccaccggccagcgcttcggacgcgcagacctgcgtccagcaactggtgttcgaccccgcaagtgggggcttcctgccggtgaacaatttcggcaccgagcaggactttctcaattgtttcggctggcaactgttcatcgccatgaactggccggtcaatcccggctggccggccgacccgaccctggcgggcgagccagacacgcaaagcagcgctgcacagttcggcgtgccgcaaacgcccggcaagccgatgagcaacgcgccggtgtgggccagctacaaggacgccaacgacattttcctgcccggtgcacccaaaccgaccggctggggcgtggaaaccctggtgccgtccaattgcaccgccaccggcaacctgaaagcgctctccaccggcgcgcgcaaattcattaccgccacgtcggaaagcgcgatcaaccgcaagcaccgcttccacctgtccagcggcacccaggtgaccctgcccgattcgatcatggaagccgccggcggctggctgacggaccagtcgggcaacctggtgtttttcgagcgcaaggtcggcaaggccgagttcgactacatcgtcaataacggcttgtacgacgccgccaatcaattgatcgtggcgcagaacagcgacaaccgacaccccgccggcctgtcgttgcctgcgggcaagctggtgcgtgagctgccggccaaggcgctgccccaggaagagttgggcgccctggaactcaaggcggcctggcgcgtcctcacccacaaacccgagctgtacgcacgctacctgaccaccgtcgcctggctgcaacgccctgacacgctgcaatgcacccaggaagtcgtgggtctggtgggcctgcatatcatcaacaagacccagacccagccgaacttcatctggaccacgttcgagcaggtcgacaacgtgcctgacggcggcgctacaccgccgcagggctacagcttcaacaacccggcctgcaccggtgatgcctgcacacccaacgtcgcccgcgtgcaatgtgacgccacccacacgccgcccaactgcacgccatttaaccaaccggtacaggccacacgggccaatgccacgcctgaggacatgcaagcgttaaacacggcggtgcagcagaccttcgcccagcagacccagggccaatcagtgttccagtactacaaactggtgaacgtgctgtggtctaaaacgcccaacgcacctaacgatccaggccctgggccgaacgtgaagacgccgctgtcctatgggccgtttgtcagcgatcaaagtgttgccgtcgccaataccaccctggaaacctatgtgcagacagagaactgcaacgactgccaccagtacgcggccattgccggtggttccaaattggcgtcggacttctccttcctgttcggcagcgccgactccgcgaagaacactcgcctgatcaaacgcatcgaggcgttcaagaccctcaaggatgatcattag

SEQ ID NO: 148 - DNA, 1734 bp, Pseudomonas sp. R81
atgagcacgcccttcacccaattcacctcgcctgccgagcaagcccccaaggactacaacaagctgggcctggaaaaccagctgccgaccttcgaaaccgactggaacaacaacgtcaccggctggacccagatgtcggtgatcggcaacccctggtccaacctcaatgacgcaccgcgttcgggctattacaacccgctggacagcggatacggcacgcagacgccagtgaccatcacctggcagcccttccccaaccggctgtggacgtttttctacaacgacggcgccgccgtggtcccacaattgggcggcaaggccatgacccttgaccaggtgatgcagttgaccgaccacggtcagatcacgctcaacaacaccctgtattcgctgtacccggacccgaaagcgacccagctgcagatccccagcgtgctgtgcaagtccatcaactggaacggcccctacgctgacttttcaccctcgggcccacggggctggctggatgaatattgcgagtggtcgatcacccgcgaccccgacggcaacatgcgcagcatcatgttcaccagcgagaacccggcctatttcctgaccatgtggaacatcgacccgcaggccgtgctcgggctgtacaaagcgtacgtcgacccgcaagtgaagatcgaagacctgtacctgcgctacaccgccaacggcccgaccggcaaggccggcgagccggtgcttgacccgaccaccggccagcccgcctacgacaccgtgaacaaatggaacagcggcactgtgcgtataccgggcgtgtcgggcggcgcgatgcacctgacctccggccccaataccttgagtgccgagatctacctcgcggccgcggccaccatcctgcggccgatcaagagcagcgccaaccaacagagcctgatctgctgcgcccaatacgggcagaactaccgcaactccgatccgcatatcggtttctccgctaaccaggaagccgtcaaagccctgatttcactgaccaaccccatcggcctgtacctgcaacaaccgaaatccttcagcacctggaaaggccctcaaggccaggatgtcagcagctactggcatgtcacccgaggcactgctggcaccgggccgaacaagtccgaccagatcctgcaagccgtcttcgaggtgccccaaagcgcggggttctcgatcaacgaaatcaccatcaacggcacgccgattgattacgtgtgggtgatcgccaacgagctgagtgtggccctcagcgtcaccccggcaccgctcaccgccacgcccgaggaatgcgattgcgtagcggcgaacaccaccgatgcgcaaccctggccggtgcagttgctgccgattgacctgttctacggacagtcccccagcgacttgccggccagctttgcccccggcagctcaggccagttcgtgctggtggtgcaaggggccgatccgaataccactgcggcggatgcgcgggtgcagttttccaatccagggatcactgcccaggtcacggaattcctgccggatgcctcggcgattccagggcagaccgacagcggcggcacccagggctacatcatgaccgtcaccgtcagcagcaacgcggtgccggggctggtcagcgtgcgcgcgcttaaccccagcgaagccgccaaccccagcgccacccagcacccgtgggaaagcggcctggcgctggtgcctggcgtctga

SEQ ID NO: 149 - DNA, 1587 bp, Pseudomonas sp. R81
atgaacaaatggcttcgcccgctgcgtcgggcacgcttgagtgtgttgtgctggataccctgcgcccttctccccctcgcccccgcaccggccattgcggcctcggacgcccagagctgcgtcagtcaactggtgttcgatcccaccagcggcggcttcctgccggtcaacaactttggcaccgagcaggactttctcaattgtttcggctggcagttgttcatcgccatgaactggccggtcaatcccggctggccagccgacccgagcctggccggtgagccggacacgcaaagcaccgcggcccagttcggcgtaccgccaacgtccggccagcccatgggcaatgccccggtgtgggccagctacaaggatgccagcgagatcttcctgcccggcgcccccaaaccctcgggttggggcgtggaaaccctggtgccgtccaattgcaccgccaccggcaacctcaaggcgtttgccacgggcgcgcgtaaattcatggcggccacgtctgaaagcgcgatcaaccgcaagcaccgtttccatttgtccagcggcacccaggtgaccttgccggactcgatcatggaggcttccggtggctggcttacggaccagtcgggcaacctggtgtttttcgagcgcaaggtcggcaaggccgagttcgattacatcgtcgataacgggctgtacgacgccgccaaccaactgatcgtggcgcagaacagcgacaaccggcaccccgccggcctgtcattgcccgccggcaaactggtgcgcgagctgccggccaaagctctgccccaggaagaactcggcgccctggaactcaaggcggcctggcgcgtactcaccaacaaaccccagctgtacgggcgttatctgaccaccgtcgcctggctgcagcgccccgacacgctgcagtgcacccaggaagtggtggggctggtgggcttgcacatcatcaacaagacccagactcagccgaacttcatctggaccaccttcgagcaggtcgacaacgtgccggacaacggcacggctgcgcccgagggctacagtttcaacaacccgacctgcaccggtgatgcctgcacgcccaacgtcgcacgggtgcaatgcgatgccacccacacgccgcccgactgcacgccccttgatcagccggtgcaggccacgcgggtcaatgccacgccccaggacctgcagatgctgaacaccgctgtgcagcagaccttcgcccaaaagacccagggccaatcggtgttccagtactacaaactggtgaatgtgctgtggtccaaaacgcctaacgcgcccaacgatccgggccctgggcccaacgtgaaggtgccgctgtcctatggaccgtttgtcagcgaccagagtgtcgtcgtcgccaacaccaccctcgaaacctacgtgcaaaacaagaactgcaacgactgccaccagtacgcggcgattgccggcacctcccaactgacatcggacttctccttcctgtttggtaatgccgattcggcgaagaacgcgcgcctgatcaaacgcatcgaggcgttcaagaccctcaaggacagcccgtaa

SEQ ID NO: 150 - DNA, 1734 bp, Pseudomonas libanensis
atgagcacgcccttcacccaattcacctccccggccgaacaagcccccaaggactacaacaagctaggcctggaaaaccagttgccgaccttcgaaaccgactggaacaacaacgtcaccggctggacccagatgtcggtgatcggcaacccctggtccaacctcaacgacgcaccacgctcgggctactacaacccgatcgaaagcggctacggcacacagacgccagtgaccatcacctggcagcccttccccaaccggctgtggacgtttttctataacaatggcgccgccgtggtcccgcaactgggtggcaaggccatgaccctggaccaggtgatgcagttgaccgatcacggccagatcaccctcaacaacaccctgtattcgctctacccggacccgaaggcgacccaactgcagatccccagcgtgctgtgcaagtccatcaactggaacggcccctacgccgacttttcaccttcgggcccaaggggctggctggatgaatactgcgagtggtcgatcacccgcgaccccgacggcaacatgcgcagcatcatgttcaccagcgagaacccggcgtatttcctgaccatgtggaacatcgacccgcaggccgtgctggggctgtacaaagcctatgtcgacccacaagtgaagatcgaagacctgtacctgcgctacaccgccaacggcccgaccggcaaggccggtgacccggtgcttgaccccaccaccggccagcccgcctacgacaccgtgaacaaatggaattccggcaccgtgcgtattcccggcgtatcgggcggcgcgatgcacctgacctccggccccaataccttgagtgccgaaatctacctggcagcggcggcgactatcttgcgcccgctcaacagcagccgtaaccagcaaagcctgatctgctgcgcccagtacgggcagaactaccgcaactccgatccgcatatcggttattccgccaaccaggaagccgtgaaagccctgatttccttgaccaaccccatcggcctgtacctgcaacaacccaagtccttcagcacctggaaaggcccgcaaggccaggacgtgagcagctactggcgcatcacccgtggcaccgccggcaccgggccgaacaactccgaccagattctgcaggcggtgttcgaggtgccggccagcgcggggttctcgatcaatgacatcaccatcaacggcacgccgattgactacgtgtgggtgatcgccaacgagctgaatgtggccttgagcgtcaccccggcaccgctcagcggcacgcccaaggagtgcgattgcgtggcggccaacaataccgatgcgcaaccctggcccgtgcagttgctgccgattgacctgttctacggccaatcccccagcgacttgccggccagctttgcgcccggcagctcaggccagttcgtgctggtggtgcaaggcgccgacccgaacaccacggcggcggatgcacgggtgcagttctccaacccaggcatcacggcccaggtcacgcagtttctgccggatgcttcggcgattcctgggcagaccgacagcggcggcacccagggctacatcatgaccgtcaccgtcagcagcaacgcggcgccggggctggtcagcgtgcgcgcgctgaaccccagcgaagccgccaaccccagcgccacccagcacccatgggaaagtggcctggcgctggtgcccgtcgcctga

SEQ ID NO: 151 - DNA, 1587 bp, Pseudomonas libanensis
atgaacggatggcttcgcccgctgcgccgggcacgcttgaatgtgttgtgctggatcacctgcgcccttctccccttcgcacccgcaccggtcagcgcggcgtcagatgcccagagctgcgtcagtcagttggtgttcgaccccaccagcggcggcttcctgccggtgaacaacttcggcaccgagcaggactttctcaactgtttcggctggcagttgttcatcgccatgaactggccggtcaaccccggctggccagccaacccgagcctggccggggagccggacacgcaaagcaccgcggcccagttcggcgtgccgccaacgcccggccagcccatgagcaatgccccggtgtgggccagctacaaggatgccagcgagatcttcctgcccggggcgcccaagccctccggctggggcgtggaaacccgggtgccgtccaattgcaccgccaccggcaacctcaaggcgttttccacgggcgcgcgtaaattcatcacggccacttccgaaagcgcgatcaaccgcaaacaccgcttccacttgtccagcggcacccaggtgaccttgccggattcgatcatggaggcttccggcggctggctcacggaccagtcgggcaacctggtgtttttcgagcgcaaggtcggcaaggccgagttcgactacatcgtcgacaacgggctgtacgacgccgccaaccaactgatcgtggcgcagaacagcgacaaccggcacccggccggcctgtcactgccggccggcaaactggtgcgcgagctgccggcccaggcgctgccccaggaagaactcggcgccctggaactcaaggcggcctggcgcgtactcaccaacaaacccgagctgtacgggcgttacctgaccaccgtcgcctggctgcaacgcccggatacgctgcaatgcacccaggaagtggtgggcctggtgggcctgcacatcatcaacaagacccagacccagccgaacttcatctggaccaccttcgagcaggtcgacaacgtgcccgacggcggcgccaccccgcccggcggctacagcttcaacaacccggcctgcaccggtgacacgtgcacgcccaacgtcgcacgggtgcagtgcgatgccacccacacaccgcccaactgcacgccccttgatcagccggtgcaggccacgcgggtcaatgccacgcctcaggacatgcaagcgctgaacacggcggtgcagcagactttcgcgcagaagacccagggccagtcggtgttccagtactacaaactggtgaatgtgctgtggtccaagacgcccaacgcgcccaacgatccaggccctgggcccaacgtgaaggtgccgctgtcctatgggccgtttgtcagcgaccagagtgtcgtcgtcgccaacaccacgatggaaacctatgtgcagagcgacaactgcaacgactgccatcagtacgcgacgattgccggcgggtccaaactggcgtcggatttctcgttcctgttcggcaatgccgactccgcgaaaaatacgcgcctgatcaaacgcatcgaggcgttcaagaccctcaaggacaatccgtag

SEQ ID NO: 152 - DNA, 1731 bp, Pseudomonas asplenii
atgagcatcccgttcacacgattcagcccacccgccaatcaggctcagaaggactaccagaaactgggcctggaacagcaacaagcgcaattcgataccgactggagcaacaatctagcaggctggaccgaagcagcaatcattggcaacccatggaccggcctgaacgacgcaccgcgcacgggatacttcaacccgctgatttcgggctttggtgatgcccctccagcggtcatcgactggacgccgttccccaatcgactgattacctacctcacgcaagccgactcggcaaaaaacccacaactgggtggcaagccactgaccatggaccaggtcatgcaactggccgataccggcgaaatcgatatcaatggtaccccgctcaaactctacgacccgctaggcagcaacaccctgcagttgccttccattcgctgcccccagatcgactggaccggcccctacgcggccttcaccccgtccggcccacgcggatggctggacgaatactgcgagtggtcgatcaccctcgacgccaacggcaacatgcgcagtgtgatgttcacctgcgagaacccggcctactacctgaccatgtggcgcatcgaccccaaggcggtgttaggcctgtaccgaatgtacatcgactcggccgtgcagttggaagacctgtacctgcgctacccggtcgaccagccgaccggcaagcagggcgaaccggtgatcgaccctaccactgggctgcccgcatacgacgtgaccaacaagtggaactcgggtaccgcgcgcaagcccggcctgtttggaggtgccctgcaccttacttccgcccccaacaccctcagcgccgagatctacctggcgggtgcttcgaccatccagcgctcggataagagtagtgaaaccccacagacgctgatctgctgcgctaagtacgggcggaactaccgtaactccgacccgcacatcggctacgtcgccaacgggatagcctacggcaaccgcatttccctgaccgacccagtcggtctgtacctgcaacagcccaagaacttcagcaaatggaaagacccgcagggcaatagcgtcagccagtactggcagatcacccgtggcaccgccggaaccgggccactgggctccgaccagatcctgcatgccgtattcgaagtgcctgagcaggcaggtttctcgatcaacgacattaccattgacggtcagaagatcacccatgtcggggtgatcgccaaccagatgaaggtcgccctatcggcctcgcctctggacgccatcaagcccgtcatccagccttgcgtgacagaccgcagcacggggctgcagccatgtccggttcaactactgccgctctcgctgttctacggtctctcgcccagcgatctacccgcctggctagcgccgagcagcagcaaccagttcatcctccttgtacagggttcggatgctgccaccaccgctgccaatgcgcgtatccagttctccaacccgggcgtgaaagcacaggtcattgagttccagaccaacgccacgccaattgcgggcacgaccgacaacagcggtacccagggctacatcatcaccatcactgtggcggccaatgctgcaccgggcctggtgcagctgcgggtgctcaaccccgacgagccggtcaatccaagcgataccgatcacccatgggccagttcactggcgatcgtgccagcgctttag

SEQ ID NO: 153 - DNA, 1557 bp, Pseudomonas asplenii
atgttctcactcgattgttcccgggggaatggccggttctgcctgcctcccttgttactgatcatttggctgctcggcagcctggtcgcccgaaacgcctatgcgctatccgaccccgaaacaccggcccaatgcgtgcagcagttggtgttcgacccaaccaacggcagcttcctgaccagcgacaccccctttgtagctcaacaggccaccttcaactgctatgcctggcagatgttcatcgccatgaactggccggtgaacccgggctggcccacccacccagagctggcgggcgaacccgataccaaaagcccggccgcccagttcggtgtgccgacgatagcggaccagcccatgagcgttgcaccggtctgggccagctacaaggacgccaacgacatcttcctgcacggcgcggccattcctaccgcctggggcatgcagccccctgagccggtcggctgccagacaaaaccctcgcttctgtccctgcgggtcggggcacgcaagttcatgaccgccacctcagagagcgcggtgaacgccaaacatcgtttccacctgtccagcagtaccctggtgaccgcctccgacccgaccctggaagccaccggcggctggctaaccgatcaggccggtaagctggtctatttcgagcgcaaggtgggaaaggccgagttcgactatatcgtaagcaatgaactgtatgacgcggctaaccagttgcaggtggcgaagaaccaggggctgtccctacccgccggggcgcattttcgcagcccgccgacgtcacccattgcgcaggaaaaactcggcgcatttgaacttaaggcagcgtggcgcatcctcaccgacaaaccccagctgtacgaccgttacctgaccaccgtcacctggctgaaacacccggaaaccggccagtgcacacaggaagtggtaggcctagtggggctgcatatcattcacaagaccgccagccaaccggacttcatatggaccacgtttgaacacgtggacaacgtgccagatggcggttctacacccaccgctggctatacgttcaacaaccccaagtgcaccggccctgattgcacgccaaatcaacggcgcatcacttgcacggccttgggctgcaaagacaactatccccgcaacgagccggtgcaggttacccgtgaagattcagtacccagcactatcaacgacctcaacactgtcgtgcagcaagccatctccaccaagaccgccggtaagtcggtgttccagtactacaaactggtcaatgtgctgtgggacgcctcaccacacataccggacccagaacccggcgccaatgcaacagtgccgctggtctacggcagcttcagcagcgacggcaacaacacacccgtgtccaataccaccatggagacctacatccagaacaggtcgtgcgacttctgccacaggaatgccaaggtagcggggagcaagagcctgacctcggacttttcgttcctgttcgagagtgccgactcgtccaagataccgacactgatcaagaagatgccctag

SEQ ID NO: 154 - DNA, 1743 bp, Thalassospira xiamenensis
atgagcacaccctttgccagatttacgtcgcccgcccatcaggcacccaaggattacaaaaagcttggtatggaaaacgaactgtcggcttttgaaaccgattggaacaataatgttgccggttggaccgagatggcgatcattggtgatccgtggtcgaacctgaatgatgcaccacgggcggattactataacccgctgaccgagggatttggtgaagccggtgacgcagtcatcagttggaccccgttcccgaaccgcttgatcgcctttctgaccccacccgaggcatccaacaacccgcaactgcatcgaccattgaccatggatgaggttatgagccttgccgatagtggcgagatcaccgtcgatggcacgctttacaagctctatgatccgagcggttcggctccgatcctgaaaatcccggccaaacggtgtccggagatcgactggaccggggaatacgttgatttctcgccatccggcccacgtggctggcttgatgaatattgtgaatggtcgattacctatgatgcgtcgggcagcaagatgcaaagcgtcatgtttacctgcgaaaacccggcctattacctgacgatgtggcggatcaatcccgaggcggtccttggcctttatcagatgtatgttgatccggcggtcaagcttgaagacctttatttgcgttacacggttgatcagccgaccggtaaaaaaggcgatcctgtcatggatccgaccaccggacgtccggcctatgacgtgaccaacaagtggaaccgcggcacggtgcgggttcccggccagtcgggcggggcgctgcatctgacgtcaggccccaatacgctgagtgctgaaatttaccttgccgcggcggcaaccattcagcgtccggatttaagcagccgcgatccgcaaagcctgatttgttgtgcgcaatacggtcagaactatcgtaattccgatccgcatatcggtttcatcgccaaccgggctgcggcacgttaccgtatttcactgaccgatccggtcgggctttatatccagcagccccagaacctttcgaactggaaggggccgaatggcgaggatatcagccagtattggaaaatcacccgtggcacggcgggaaccggtccgaacaattcggaccagatactgcatgcggtgtttgatattccgccaagtgccggtttcacgatcaatgactgcacgatcaatggtcagaagattgctcatattggcgatatcgccaaccagatgaaaattgccctttcggcaacgcagatgactccgaaccaaccgttgcagtcaccgatgaaatgcgtttcaagccgcagcagcggcagtatgcagccctggccggttcagtttgtgccgattgatctgttttatggggaatctccgaccgatcttccggcattgatggtaccgggaacggtgaatagctttgttctgatcgtgcagggagcggataaaaacaccacgatcgacaacgcgcggattgagttttccaaccccgggatcaaggccaaagtgaccaagttcctgccagatgcatcggcgattccgggccagaccgacggcggcggtacgcagggcttcattatggatgttgctgtatcgtcatcggcaaagccgggatccgtcagtctccgggttctgaacccgaatgaaccggccaatccatcggatgctgatcatccgtgggaaagtggtttggcggttattcccagtcattaa

SEQ ID NO: 155 - DNA, 1620 bp, Thalassospira xiamenensis
atgaaccgattacatttgggggcaggctgtgtgattgcggggttttgtatcctggcgattgcgggacttctttgggtgattgatgttccggctggcagggcggatgaaatcaatatcagccgggtgacggaaatagcccaatcggcacagcaatgcccggatcaactggttttcgatccgacaagcgggtcgttcatgaccagtgacaatctgttcctgccaacccagcagggtaacaattgttatgcgtggcaaatgttcatcgcgatgaactggccggtcagcagttcatggccgggaacaccatcggccgcaggtgagccagatcaaaacgtttcggtggaaaattggggggtaccggaaaatccgacctcacccttaaccagcgtaccggtctggggcagtttcaaggatgcgcaggcgatcttcctgcctgatgcggccaagccgaccgattggggcgtgccgcaagccgtgccgtcgggatgtaaaagtgacaagatgttgctgggttatccggctggttcggcaaagattttaacaacgctttcaaaaaatgcggtcaatactgcccatcggttccatctttcaagtggtacgcgtgatacccagtccgacgagatcatggaagccaccggcggatggttgacagatcagaacggcaatctggtgtttttcgaacgaaaggtcggcaaggccgagttcgattacatcatgaacaatgcgctttatgacgctgcctatcagatgcgggtcgcaaccaatgctgatggtcgacatccggcgggattgtccctgccaagtggcaagttcctgcgtgttccaccgacggaaccgcaaggtcaggatgcgcttggagcgttcgagatcaaggcagcgtggcgggtcctgacagggcaaagcgacatttatgaccggtatctgacatcggttgcatggctgaaacgtcctgataccggtgaatgcagccaagaagttgtcggtttggtcgggcttcatatcattcacaagaccgatacattccccgatctgatctgggcaaccttcgagcaggtcgacaatgtgcccgacgggcaggcaactttaccgcctggcggatattcctttaacaacccgaattgtaccggaccggattgcaaacccaatcagccgcgcattgactgtaacgatcagaaccagtgcaaggatctttatccccgcgatcagcccgtacaggttacgcgcgaacaggccctaaccagtgaaatggatacgctaaatgccggtgttgcccaaaagatcgcatcgcaaaccggcgggaaatcggtgtttcagtattacaagctggtcaatgtgttgtgggatggcagcccaagccccccagtcatggagcccggtgcgaatgcatcgataccgctgcgctatggcacctttgagtccgagggtaatctgaaagtcgccaatacaaccatggaaacctacatccaggatcaatcctgcgatttttgtcatgccaatgcgacgattgctggcagcgatacgctagcatcggatttctcattcattttccgcgatgccggatcggcgaaaaacccgtcactggtggaagaggtaaaacaattcatggagcaggcacaatga

SEQ ID NO: 156 - DNA, 1734 bp, Paracoccus denitrificans
atgaccatattcacggaattttcgacccccgcacagcagggcccgaaggattaccagcttctcggcctgccagccgccgatctggccgcgttcgaggcggactggagcgcgaatatcgccggctggacccagatgtcgatcatcggcaatccctggtccaacctgaacgacacaccgcgcgacaactactatgatccgctggtcgaggggatgggcgaggccacggcggccgtcatcagctggccgccctttccgaaccggctgatccagttcctaaccaatcccggcatcgtcaagggcgggcagttgacggcaccgcttagccaggatgcggtgcaggaactggccgatagcggccggatcacccagggcgggacgagtttcgtgctgttcgatccagaaccgggtcaggtattgctgaagatccccgccgaccgctgcccggccatcgattgggacggcaagtatgtcgacttctcgccctcggggccgcgcggctggcaggacgaatattgcgaatggtcgatcctgcgcaatgcccagggaaaaatgcagtccatcgccttcacctgcgagaatccggcctattacctgaccatgtggcggcagaacccgaaggcggtgctgggcatctatcagcgctatatcgacccggcggtgcagctggaggatctgttcctgcgctatgaatacgatcagccgacgggcaagaagggcgatccggtccttgatccgacaacgggcaatccggcctatgacccgacgaacaaatggaacaggggccccgcacgggtgcccggttcgttcgggggagcgatgcatctgacgtcgccgcccaatacgctgtcggcagagatctatcttgccgccgccgcgacgatccagcgcccctcctcggtcaatggcaatccgcaatcgctgatctgctgcgcgcaatacggccagaacttccgcaactcggatcccaatatcggctatggcgcgaatgtcgccgcgcggaccgccaggctgacgctgaccgatccggtcggcctctacatccagcagccgcagaactttcagggttggagcggtccgaatggcgaagatgtctcaggctattggcaaatcctgcgcgggacggcgggcaccgggccgaacgggtccgaccagatcctgcacgcggtctttgccatccccgaaagcgccggctattcgatcgaggattgcaccatctacggcctgccgatttcgcatgtcggcgtcattctggaccagatgaaggtcgcgctggcggtcacgccgaacaatgccgccccggacacgaccgcattcgcctgcgtgaccgaccgaaccgacggcacacaaccctggccggtgcagatggtgccggagagcctgttctatggtgaatcaccctcggatctgccggcgcttctgcggcccggaagcaagttccgctttgtcctgatcgtgcagggggcggatgagaacaccacgcccgcaaccgcaagggtcgaattctccgatccgaatatcaccgtcacggtcgagcagttcctgaaaaacgcctcggcagtgccggggcagaccaatggcggcggcacgcagggttatgtcatggacatcgccgttggcgcgaacgcgcaacccggtccggtctcggttcgggcgttgaacccgtccgaagggccggcgccgacgcccgagcagcacccctgggaagcgggccttgcggtcatctcgtctcggtaa

SEQ ID NO: 157 - DNA, 1509 bp, Paracoccus denitrificans
atgcgcacaggtcagatcctcatcgcactggtcgcaggcgtcatgcttgcctttgccgcatccggcggcaaggcccagaccgcctgcagcgccatgctcatcaccgatccgacctcggccgatttcctgaccggagacacgcccttcggccatacccaggacggaatgaactgctatggatggcagatgttcctgtcgctgaactggccggccgatcccggatggccgcaaacgcccgccatggccggcgagccggatcgcagcgcgacaatcgccgatttcggcctgcccggcccggcgggacagccgatgcagcgacccacggtctggcaaagcttcatgccggcgcccgagatattcaagccctttgcggccatgccgaccggctggggagaaacctcgccgccgcccgccagttgcggctccgcctcgctggcagcctcggccgggtcgatccgcatgctgaacgcggtctccaaatccgccgtgagcccgcgtcacggcttcaacctcgacaccggaacgatgtcatccatatcggacgaaatcgaagaggctacgggtggctggctgaccgatcagaagggcaagctggtgtttttcgaacggatgatcggcaaggccgaatacgactatatcgtcgcgaagggcctgtatgacgcggccaaccagttgaaagtggcgaccaatgccgacggagccacccccgaaggcctgtccctgcccaaaggcacgccaccgggatcggccgttcagaaccaggatgagcttggcgccttcgagctgaaggccgcctggcggaacctgaccgggctggatgacctttatggccgctatctgacctccacggtctatctgctgtatcccgacggctcttgcgaaaaggctgtcgtcgggctggtcggtctccatatcattcacaagaccgcctccatgccagatttcgtctggtccaccttcgagcagatcgacaatgttccgggcgcgtccgcgccggaagtggatttcagtttcaacaacccggcctcgaatgcgaagccgaaccagatgccgcactgtgtgaatggtgtctgcgactattccctccccatccaggtcacgcgcgaagtcgcgatcccggccggtgtggcgcagaccaaccgcgacgtgcagcagttgcttgcggaccggacggggggcaagtcggtgttccagtactaccagctcgtgaacgtgctgtgggacggcgcaccgaccccgccgtcaccggaacccggcgcgaatgcccaggttccgctggtctatggcaccttccagacggatggcagcgtgccggtcgccaatacgacgatggagacctatgcgcagcaattcacccccggtctggggccgtcctgcaccgcctgccacaagggcgccaccatcgccaacagcgcaacgctggcgtcggatttttccttcctgttctcgaccgcgtccagcgccacgaaactgccgggcctgttcatatcccgcgactttgttccatga

SEQ ID NO: 158 - DNA, 1743 bp, Cellvibrio japonicus
atgtcagcgtttacattttccactcctgcattaattcaggatttcagcgacaacccctccctgcagcagcaactcaaccaaaattgggatttggcaattgatgcgtatacccaggctgccctggttagcaatccctggactgtggattaccaggctccctgcgattggtatgtgaatcccaaacaggcggatattaccgcagctaatccggttgaacctattttttggacggcttttcccaaccgcttgaaaatttatttttcggcggctgaaaaaagtccttatcaaatggcgaatgcgcaggtttttgcgctggcggattttggcaatgttccgcaatcgaaggcgtttcccacaggtttgccgtttattattcccagcaagcgctgccctaatttgaattggcagcagtcgattgctgagtgggtacagtacgatcctaaagggccgcgcggttggttggatgaatattgtgagtggtccgtgacgcgcaatgccgatggaaaaattaccaagattgcgtttacctgcgagaatccggagtactggtttaccctgtggcaggtttcaccggaaaaagtattggcgctttaccagcaattggtgagcccgaatgtggtgctggaggatttgcaattgccatcagccgatggcaagggatttgttatcgatccgacaacagggcgccctgcctataaccccttgaataaatggaattccggtacggtggcgacagaaacctatggcggtgctgtgcatctcaccagcccaccgaacaccatcggtgcggaaattatgttggcggcacaggcaaccctgttgcgcgatttgccgccggaccagtacaacatgcagcgtatggtatgcgccggtgcctatggacgcgcttatcgcaacagtgatccgcatatcggtttgcaggcaaaccagttggtgaaaaacctgggtgtgaaaatcaccttaaccaacccggtgggtttgtatttgcagcgcccggatttcagcagctataagacacccgatggtaaggatgccggccaattctataaggtcattcgcggtcgcaccgcccaacaggcaggtacgacttacgaccagatattgcatgcggaattttcagtaccggaagaactgggttataccgtcagtgatattttgattggcaacgccgtgcccggcagttcccaggtgcctgtgccgattctctatgcgggtcaaattgcagaaacattccatgtatgcctggcgggaacagcgattgcccccgctacaggtgaaccttcgcaagcatttttaccaccggtgactgataaaaccggtaataccaacggccaggtgagcatgctgttggcaaacccggtattgctggccatgcaggcagtgaacccctttcccccgtttgtgcaattgccggtacaaattgcccagggtcaaacactcaccaatatggctttgcaggtcagttacgccaatgacaatttccaggaggcgcaaattgcattctgggatgcacagggcaatagcgagccgggcatcagtgtgacagtaacggccatagagactgctgatgggacaccggcgggaaaaagcgccggtggtgatggactgtttaattacattatcagcatcagtgtcgcgccgggggtaagtcccggctttaaaggtgtgacggtgcgcaaccccgcatgtgatatgcccttgccgttgccgggtgtgttgtttgtgactgcaaaaggaaactaa

SEQ ID NO: 159 - DNA, 1521 bp, Cellvibrio japonicus
atgaagcatacattactgataggggttaccaccggtttgctggtggctgcctgccagcaaccggtacaggagtcatccgcagcggttgacgctcccgccgtgagcacggtgtccagcagcagtgcgccaatcagctttccctgcctgaataaaccggcggttaattacaacacaccgggggatacacccatcacttcgcaagatggtgtgaattgttttgcctggcaaacgtttattggcctgaactggccggtcgatgccagccatccgggtgagccggataagacggcgtctgcgtctgtgtttggtgagccgggtttgcaccaaacctcggtgtgggaaacctatgccaatagcaagagtgtatttcgtgcaaacgcccaaccacccctgccctggggacatacgcccgatgtgccatccagctgtcaaaaaatatcccagacactgggcttgcgcgttatgcaggcgagccgcatgccgggcagttttaatatgagtaaggaggcctcgcaggcatttcccggcaacaatcccaattggctggcggataagagtggcaacctggtgtattacgaaatcctgattggcaaggacgagtacgattacatcaataataatggtttgtataacgccaatacccaggctgcccatatccagcagaacaagaatattgccatgcccctgggccacgacaaggtgctgggtgggttggagattaaagcggcctggctgagcgtgagcgatccacaaaatcccaagtggaaaaattacaagctcagtaccagtgtgatttacgatccggtttccaaggattgccacgcgagcacgattgcgttagtgggcatgcacattatccgcaagaccgcatcgcaaccgcagtggatctgggccacgtttgagcacaaggacaatgcgccggatactgccagtattaaaagtgatggcacggtggatggcgattacaccttctatagcaacagctgcacggtcaaaccggtgccggcgggttgcaaggccaaggttgaaaatggcacatcggttacccaaacctcctgccacgtgaatgtatcgcccgcgtattatctggatactagcggcaactgtccggcctatcccatccaggtgagccgcgattttgcgatcaaggattccaccgataaccacgtggcctcgctcaaccgcgcagtacaacaactgattgccagcagcaatgccgattcggtgtatacccattaccagctggtgaatgtgctctggtcatcggcggcggtgaatgacaatgcaccaccgggcaatccgccgctgacgcccttatcgatcagcggtgaaacgccatcgctcaataccgtgccggttgccaataccatgctggaaacctacgcacagggttttaactgtttgtcctgccatgcctatgccagtgtcgcgcgcgatgccagggcacagctgggcggtaaggcttacgcaacggattacagttttatttttagttttgcgacgtcacccgctgccaaatag

SEQ ID NO: 160 - DNA, 771 bp, Pseudomonas brenneri
atgggttccattactgatcataatcaactgctggcctgggtagcatccttggatattcccgaagcttccggagtaaaaacccgttcgcgtaatgtggttgcgcgtgctaatgccgaggacgaaggcgcggcagtagtacgcggtagtattacttcgtttgtgaccggcctgagtcaacaagcgcgtgatgacgtgcaaaacagcacgttgttgatgcagttggctgcggataaaaaattcaatccggaaaaacaacgggaagagtggttcaagttctataccgatggccttgctaacctgggctgggggcgtgttagctcgtattatcagagctatcagccgcgtaataccaatgtcaccatggaccaggtcgtacttgaggtgattgctgcagtcgtgggcgctgacagcgctgtgtacaaggtgactgaaaaaaccttctcgtcactccaagacaatccgaagaaccaggccccgctgaaactgttcgacagtagcagcactcgggacagcgtgggcacgttccagatactcccagtgatgcaggatagggacggaaacgtggtaatggtactgactaccgtcaacgccagtaccacggtacagcgaggcagcttcctgttctggagttggagcaagaccaccgcgtggatgtatcgggctgcacagcagactgtgctcaatgagtcggtatatgcgactgttcgccaatctgtcatcaagaagctgggcaaaaacgccgaagaattcatcgatgatctggaaatttaa

SEQ ID NO: 161 - DNA, 783 bp, Pseudomonas brenneri
atgaaattgtctgccgacgaagtttatgtgatttcgggtaacttgctatccgcgacgccttcgctcaccgatcctacggtacttgaagatatcgccaattcaaaccttttgtgccagttggcagccgataagaatcaaggcacgcggtttatcgatccagctgcgtggctggacttctatcgaagctcactaggtaggttgttctggcgcatcagtaattcaggcacggttagttatgctataccgcaactcgtgcataaaattaccgtgaaagaagttttggaaaaaacgttctacaagactctggatcgcccccagcgcatccgggttgaagaaagtattgaattgttgggtgagcaatcagccgatagcccgtcggcgacattgtacagcctcaagacccaggtcaatttcaatgagacgacatcatctccaggtctcttgccccactctatatcgtccgttaacttgcaactcagtgtggtgcacagtgagacgtgcatttcggtgtgcagtgtttacttcaaaacgtcgacccggatcggtgatgatgtattcaatcagaagttcccggtaaaagaactgctgggcaatgttagtgtgagtacgttcgaagccaagctgctggaatcgagttatgccggcataaggcagagcatcatcgataagttgggtgaggacaatattcgcgagaacattctgcttgtccccgccgtttcaccgtcgttgtccaacacgcgccacgcgggggcgctgcagttcgtgcaggaactggatatttag

SEQ ID NO: 162 - DNA, 783 bp, Pseudomonas gessardii
atgaaattgtctaccgacgaagtttatgtgatttcgggtaacttgctttccgcgacgccttcgctcaccgatcctgcggtacttgaagatatcgccaattcaaaccttttgtgccagttggcagccgataagaatcaaggcacgcggtttatcgacccagctgcgtggctggacttctatagaaactcactaggtaagttgttctggcgaatcagtaattcaggcacggttagttatgctataccgcaactcgtgcataaaattaccgtgaaagaagttctggaaaaaacgttctacaagaatctggaccgcccccagcgcatccgggttgaagatagtattgaattattgggtgagcaatcagtcgacagtccgtcggcgacattgtacagcctcaagacccaggtcaatttcaatgagacgacatcatctccaggtctcttgccccactctgtatcgtccgttaacttgcaactcagtgtggtgcacagtgagacgtgcatttcggtgtgcagtgtttacttcaaaacgtcgacccggatcggtgatgatgtattcaatcagaagttcccggtaaaagaactgctgggcaatgttagtgtgagtacgttcgaagccaagctgctggaatcgagttatgccagcataaggcagagcatcatcgataagttgggtgaggacaatattcgcgagaacattctgcttgtccccgccgtttcaccgtcgttgtccaactcgcgccacgcgggggcgcggcagttcgtgcaggaactggatatttag

SEQ ID NO: 163 - DNA, 783 bp, Pseudomonas fluorescens
atggggtcaattactgatcatggaaaactgttggcttgggtcgagtcgctggatgtacccaagtcgaccggcaatgccaacctcaagcgcgcttcggctgtgctgcgcagtgccgcgcagaacagtgatgaagatggcgccgcagtcgtgcgcggcagtatcacttcgtttgtgaccggcctgacgccccaggcacgggatgacgtgcaaaacagcacgttgttgatgcaattggcggcggacaagaaatacaacccggatacacaacgggaagagtggttcaagttctacaccgatggtttggccaacctgggttggggacgtgtgtcttcggcgtaccagaaatacaagccgaccaacaccaatgccaccatggaccaggttgtgcttgaaatcatcagctccgtggtcagcccggaaagcgcgctgtacaaggtgactgaaaaaaccttcctggcactcaagaacaacccgaacaacaaagatgcgctgaagctgttcgatgtcagcagcacccgcaacgacctgggcaccttccagatcttgccggtgatgcaggacaaggacggcaacgtggtcacggtgctgacctgcatcaacgcccataccgaggtacaaaagggtagcttcctgttctggcactggagctcgaccagtgcggaaatgtaccgcgccgcgcaacaagttgtactcaatcagaatgtgtacgccaccgtgcgccagtcggtattgaagaagcttgggaaaaatgccgaagacttcattgatggtctggacatctaa

SEQ ID NO: 164 - DNA, 780 bp, Pseudomonas fluorescens
atgagttttactgcccctgaagttcatgtggtttcaggcaacctgatatcggcgatgccgtcggtcaacagccctcaggtacttgaagatattcttgaatcgaatttgttgtgccagatggcggcggataaaagtttgggttcgcgattcaataatccggctgcctggctggatttttatcgcaactcgctgggcaagctgttctggaaaatcaccaacttcaacacggtcagttatcccgtgccgtcacctacgcgttccgtgagcgtcatgggcatactggagcacactttcttcaaggtgttggcgcagccacttcgtcatcagatagaagcggatatcgagttgctgatggagctgccgctgacgagcccagcatcgcagctatacacctcaaagacccatgtggaaatgagcacgcgtgcgcgctcaagttttgatgggcgctctgagtcggtgatcagcctgcaaatcagcgttgtccacagcgggtcgctgatttcggtgtgcagtgtctacttcaagaccgcagagccggtggcagctgatgtgttcagtcagaagttcaaggtgagggatttgctgggcaacatcagcgtcaactcgttcgaggctgatttgttggagggtagttacgaaggcgttcgacagcaaatcaagacgaagctgggtgaagccaatatccgcgagaatatcctgttgatcgctgacaaccccatcccggtggacgaattgccccacgcaaatgcccatcagtttctcaaagggttggatatctga

SEQ ID NO: 165 - DNA, 768 bp, Alcaligenes faecalis
atgagcacgattactgaccacaagcaggtattggcatggattaacgccctggacattcccgacgccccggccggcggcaaccgtgtagccgcacgagcgaccagcagtgccgacgaagatggtgccgtcgttgccaaagccagcatcccttgctttgtcagcggactgaccgaacaatcccgcgccgacgtgcaaaacagcaccttgttgatgcaactggccgctgacaagaaataccccaacgaaaatgatcgcgaaaaatggttcaagttttactccgatgggctgaccaacctgggctggggtagcagcagcagcttctttgaacgcttccaacccaagaatacggacgtcaccatggaccaggtcgtactggaggtgatactgacagtggttaacaacgtcaataatccgctatacaaaatcgcccaggaaacattcggcgccttgaacaagcctgccaatcaaaagcccatgaagctgtttgaccacagcagcaccaaagaagaccgcggcaaattccagattctgcctgctggccaggaccagcacggcaccgtcagcatggtgctgaccgccatcaatgcacggaccgacatccaatccggcagcttcctgttctggaaatggagcaaatccaccgcttggctctaccgcgcagccaacctgattgtgctcaatgaatcggtgtactcgaaggtacgccaggcagtcatcgacaagctcggcgataacgctgtgaactttgtgctggatctggatatttaa

SEQ ID NO: 166 - DNA, 807 bp, Alcaligenes faecalis
atggctttttctactgagcaaacctatgtggtgtcaggcaatctgatttctgccaccacagaagacaccaatacgctgagctatgaagactttatccattccaaccttttggcccagatgggcgccgacaaaaaactgggctcccgctttgttgaccccgcaggctggctgagttttttcaagaatacagtaggcaatctgttctggaacctgagcgagcagggaaccagcacgttgaaaatctcagccggtaccgcaagcatcaccgtgcagcaaatactggagcagagttttttcaaacggctcaaccaagcgcaaatcgatagcgccacggcaagtgttgatctgtttagtcaactctctgaagatgatcctgccttcatcctctataacgcgaaatcacatgcccagatctctacggctaccaaggtgatcaagccaccccaaaaagagacttatagcgtcaacttgcaaatcagcattgcccatacagggtcggaaatcgcactgtgcaatattttcttccaaaccagccaggcagtcagcgacgaattattcacacagaaattcgcaatcaaagatctgattggaaacattaatgtgttttatttaaaggctctactctccgagaccaattacggccacatcaggcaacaggttatcgaaaagctgggtgagaacatcaacaccaatattgtgctggtagccgataacagcgataagccctccccccccttctcccacagaggcgcgcagtttcatacgcagcctgaaaatctaatccagcaacgcacaggcccaccatga

SEQ ID NO: 167 - DNA, 768 bp, Alcaligenes faecalis
atgagcacgattactgatcacaagcaggtattggcatggattaacgccctggacattcccgacgctccggccggcggcaaccgcgtcgccgcacgagcaagcagcagtgccgacgaagatggtgccgtcgtcgccaaggccagcatcccgtgctttgtcagcggactgaccgaacaatcccgcgccgacgtgcaaaacagcaccttgttgatgcaactggccgctgacaagaaataccccgacgaaaatgatcgggaaaaatggttcaagttttactccgatgggctgaccaacctgggctggggtagcagcagcagcttctttgagcgcttccaacccaagaacacggacgtcaccatggaccaggtcgtactggaggtgatattgacggtcgttaacaacgtcaataatccgctgtacaaaatcgcccaggaaacatttggcgccctgaacaagcctgccaatcaaaagcccatgaagctgtttgaccacagcagcaccaaagaagaccgcggcaaattccagattctgcctgcaggccaggaccagcacggcaccgtcagcatggtgctgaccgccatcaatgcacggaccgacatccaatccggcagcttcctgttctggaaatggagcaaatccaccgcttggctctatcgcgccgccaacctgattgtgctcaatgaatcggtgtactcgaaggtacgtcaggcagtcatcgacaagctcggcgataacgccgtgaactttgtgctggatctggatatttaa

SEQ ID NO: 168 - DNA, 780 bp, Alcaligenes faecalis
atggctttttctactgagcaaacctatgtggtgtcaggcaacctgatttctgccaccacgaaagataccaatacgctgagctatgaagactttattcattccaatcttttggctcagatgggcgccgataaaaaactgggttcccgctttgttgaccccgcaggctggctgagttttttcaagaatacagtaggcaatctgttctggaacctgagcgagcaaggaaccagcacgctgaaaatctcagccggtaccgcaagcatcaccgtgctgcaaatactggagcagagttttttcaaacgactaaaccaagcacaaatcgatagcgccacggcaagtattgatctgtttgatcaactccctgaagatgatcctgccttcatcctctataacgtgaaatcacatgcccagatctctgcggctgccaaggcaatcaagccgccccaaaaagcgacatatagcgtcaacttgcaaatcagcattgcccataccgggtctgaaattgcactgtgcaacgttttcttccaaaccagccaagccgtcagcgatgaactgttcactcagaaattcgcaatcaaagatctgattggcaacatcaatatcttttatttaaaggctcagctctccgagaccaactacggccaaatcaggcagcaggttatcgagaagctgggtgagaacatcaacaccaatattttgctggtagccgataacagcgaaacgccctcccctccttctcctgcagaagcgcgcagtttcatacgcagcctgaaaatctaa

SEQ ID NO: 169 - DNA, 768 bp, Alcaligenes sp. HPC1271
atgagcacgattactgaccacaagcaggtattggcatggattaacgccctggacattcccgacgccccggccggcggcaaccgtgtaaccgcacgagcgaccagcagtgccgacgaagatggtgccgtcgttgccaaagccagcatcccttgctttgtcagcggactgaccgaacaatcccgcgccgacgtgcaaaacagcaccttgttgatgcaactggccgctgacaagaaataccccaacgaaaatgatcgcgaaaaatggttcaagttttactcggatgggctgaccaacctgggctggggtagcagcagtagcttctttgaacgcttccaacccaagaatacggacgtcaccatggaccaggtcgtactggaggtgatactgacagtggttaacaacgtcaataatccgctatacaaaatcgcccaggaaacattcggcgccttgaacaagcctgccaatcaaaaacccatgaagctgtttgaccacagcagcaccaaagaagaccgcggcaaattccagattctgcctgctggccaggaccagcacggcaccgtcagcatggtgctgaccgccatcaatgcacggaccgacatccaatccggcagcttcctgttctggaaatggagcaaatccaccgcttggctctaccgcgcagccaacctgattgtgctcaatgaatcggtgtactcgaaagtacgccaggcagtcatcgacaagctcggcgataacgccgtgaactttgtgctggatctggatatttaa

SEQ ID NO: 170 - DNA, 780 bp, Alcaligenes sp. HPC1271
atggctttttctactgagcaaacctatgtggtgtcaggcaatctgatttctgccaccacggaagacaccaatacgctgagctatgaagactttatccattccaaccttttggcccagatgggcgccgataaaaaactgggctcccgctttgttgaccccgcaggctggctgagttttttcaaaaatacagtaggcaatctgttctggaacctgagcgagcagggaaccagcacgctgaaaatctcagccggtaccgcaagcatcaccgtgctgcaaatactggagcagagttttttcaaacggctcaaccaagcgcaaatcgatagcgccacggcaagtgttgatctgtttagtcaactctctgaagatgatcctgccttcatcctctataacgcgaaatcacatgcccagatctctgcggctaccaaggtgatcaaaccgccccaaaaagagacttatagcgtcaacttgcaaatcagtattgcccatacagggtcggaaatcgcactgtgcaatattttcttccaaaccagccaggcagtcagcgacgaattattcacacagaaattcgcaatcaaaaatctgattggaaacattaatgtgttttatttaaaggctctactctccgagaccaattacggccacatcaggcaacaagttatcgaaaagctgggtgagaacatcaacaccaatattgtgctggtagccgataacagcgataagccctcccccccttcccccacagaggcgcgcagtttcatacgcagcctgaaaatttaa

SEQ ID NO: 171 - DNA, 783 bp, Enterobacter sp.
atgaatactaacgctttggattttgtgcttaaaacaccgattgaaaccactgccgatctggcaccgttactggaacgtctaaagggggtaccggatcatggtcagtcaaaaagaaaaaccatgctgactgataataaagtatctgcacaagtcaatgccggcagcctcatctcatttaccgaacgtttggatgggcagaataaacaagatgtgcagaactcaacactgttcgctcaactggcggcggataaacactgcaaccgttatactgcgcccatggattggtatcgtttttatgtcaatgtactgggccaaattggctggaaccaacctgctttcgcgtttgatacctatacgtcaggtgccagtaccgtaaaactggatgaggctgtgttggggatcattgcgcaaatcgctactgtcggtgaggttgcattagtggcagcggcaatgaaggcgttatccagcctgagcgatacctcaaagcaaatgcttatctgggacgcgaaatcaaattcggaaaacaccggtaattttcaaattttcccggcagatctgttaccaaatggcgatgtggtaatgatgcttgatggtatgcaatttgatgcaaagcgcaatgaggggcgttttctgtgggtaacctggcaatccacctcgatcaaaattcaacgcgcggcaaataaattcgtcttaaacgaaggtgtttataagggggtgcgccaggccgttattgataaactgggtgatcgggcaatcgatatgattgcaaatattgaaatctga

SEQ ID NO: 172 - DNA, 777 bp, Pseudomonas fluorescens
atgagttttgaagtgtgtgacagcagcgtggccgcctgtgtggcgcgtctggaaagttatgatatctatccagatatcagtccccgctcgttgtattcgggtgatatcgagcctccggcgaaggggtcggttgtcggtgaaggtatcctggccttcgccggtggtctttcttcgcaacaccaggaagatgcgcagcatgcctttctctttgcgtccctggtcgccaacaggcagtaccctctcgaatcccaggggcgagagtggtactacaagtttgttgaagtcatgacgaacgccggttgggtcgccacgcagcgcttctacgatgatctgagcatcgccggcaacaccgtgcgaatggacaagctggtgttggacatcctcgcttccgtagtgtcggggattgccctcggaagcgcgacttcggcgttgctattgagggtcgccgacagtgcaatcacggccctgcagaagaaggaaaagaccctgacccttttcgagcgaaacctgctggaacatggtgtgggcggaatggcggccgggacctgtgttgaaatcgacggtgaggtcagcatgctgcttggcactgtgcgctttatccggcgcaacagcgcgacccaggtcttgtttgcagattggaacagtcgcgaagtgaagttgtataaaggtgagtcggttttcaggaaagtgccgagtattgtcgagcgaacccgaggcatcattattggtcggctgggtaatcatgccgtcagcaagatcgaagagtacgaaatctaa

SEQ ID NO: 173 - DNA, 729 bp, Pseudomonas fluorescens
atggacaaggcatattcgatttttgttaacgcggcggcgattgttttagtttcctccactgtgcggggaacaggggttgaagacctgatgaattcggtcttgctcgcgcaattggtggctaacaagaatctgcagcgcataccaagcgctgattggtacgctagttatatggacgtcctgagtgtcgcctgggtagcgggtgccaaacgccgaaaggacctgctaccgaaacaagacgctgccagctcgccagtggagtgggttacagcaatacctttggacgatcggccggaccagcaacagcagatcatggcggtgttggaccgtgtcgccgcgttacccggctcgctgccggcgctgagtatcctgcgcaagcatatgcaaaaaccaaacgaacctgagccgacgcagagcccttcagcgtccagccccgtgcgcttgttggtgatcgtagcgcacagccccgtttcgatgaccggtatctgtttgcaattcaacacagggaaagcgatcaatgccaacccttgggggcaatgctttgatggaaaggacatcgacggttgtgtgtcggcgcgttatttgcgcatgcaactgagcgaaacattgttcgcgccggcccgtgaggttatcgcccgtaaggtagggactgtcgtgggcgacaacgtggtggatatcaccggggctatcgaggattcggttgttcgtcctgccgaggaggtcgggcgatga

SEQ ID NO: 174 - DNA, 777 bp, Pseudomonas brassicacearum
atgagttttgaaatgtgtgatagcgctgtagccgcctgtgtggcgcggttggaaagttatgatatttaccctgatgtcagtcctcgttcgttgtatgtggacgatgttgagccaccggcgaagggatcggttgtcggtgaaggcatcctggcgttcgccggtggtctttctccccagcatcaagaggatgcgcagcatgcttttctctttgcttccctggtcgccaacaggcaataccctctcgaatcccaaggacgagagtggtactacaagtttgttgaagtcatgacgaacgccggttgggtcgctacgcagcgcttctatgatgacctgagcgtcggcggtaacaccgtgcggatggacaagctggtgttggacatcctcgcctccgtagtgtcgggtattgccctcggaagcgcgacttcggcgttgctgttgagggtcgtcgacagtgcaatcactgccttgcagaagaaggaagagaccctgaccctttttgagcgaaacctgctggagcatggggtaggcggaatggcagcgggtacctgtgtcgaaattgacggtgaagtcagcatgatgcttggcaccgtgcgctttatccggcgcaacagcgcaacccaggtcttgtttgcggattggaatagccgcgaagtgaagttatataaaggcgagtcggtttttcgaaaagttccaagtgttgtcgagcgaactcgagatatcattattgggcggctgggtaatcatgccgtaagcaagatcgaagagtacgaaatctaa

SEQ ID NO: 175 - DNA, 729 bp, Pseudomonas brassicacearum
atggataaggaatattcggtttttgttaacgctgcggcgattgttttagcgccctgcgcactacggcgcacggaagttgacgacctgatgaattcggtcttgctcgcacaactggttgctgataagagtctgctgcgtgcaccagcggttgattggtacgccacttatttggaggtcttgagtgtcgcctggatatcagctgccaaaaggcgaaaggatctgcagccgcaaaaagaagatacccattcgccattggagtgggtggcggccatccccttggatgatcaggtggatcagcaacagcggatcatggcggtgatggagcgtatcgcagcgttacccggctcgctgcctgcgatggggattgtgcgcaagcatgtgcaaaaacaatacgagcctgacgcggcacagagcccgtcatcttccagccccgtgcgcttgctggtgatcgtggcgcaaagccctgtttcgatggctggtgtctatttgcaattcaacacagcgaaagtgatcgaggccaatccttggaggcagtgctttgatggcaaagacatcgacggttgtgtgacggcacgttatttccgcacgcaactgagcgaaacattgttcgcgcctgcccgtgaggttatcgcccgtaaggtcgcggctgccgtgggtgacaacattgtcgatatcaccaaggctatcgatgattcaggtgttcttcctgccgaagaggtctgcagatga

SEQ ID NO: 176 - DNA, 792 bp, unknown
  Switchgrass rhizosphere microbial community from Michigan
atgagtgtaaatatgatcgatagtgctactgttgctgcctgtgtaaggcgtctggaaagttacgaaattgatgaagtgccagttgtacgttctcgtgcatttgctgcaagtgggattgttgttgaggagccttcgaagggggctgtcgttggcgaaggcattttgtccttcgtaggcaacctgtccgagcaaaatcaagtagatgcgatgcacgcctttctttttgccagccttgttgcgaataagcaatttccttacgagtatcagggcaaggaatggtactacaagtttgtcgaagttatgacctccgccggttggctgacgagccaaaaatattacaacgacattgaaattagcggaaataccgttcggatggaccagttggtactggaaatccttggctcggtggtcgctggcctcgctataccaggcactgcttctgcactgatgctgaaggttgccggtgatgccattaccgccttgaaaaagaaagaaacggctttaacgctgtatgaacggaatttgttggaacatggcgtaggcggtatggctgcaggaacctgtaccgaagtcaatggtgaggtaaccctggcactagggactgtacgttttattcgcaaaaatacagcaacccaagtcctgttcatggattgggatagtcgtgatgtgcagctgtataaaggtgaatctgttttcagaaaggttccttatatcgctgaccaaacccgagacctgattcggacaaaacttgggacgaatgcagtcagtaaaatcgaaggctacgagatctga

SEQ ID NO: 177 - DNA, 729 bp, unknown
  Switchgrass rhizosphere microbial community from Michigan
atggcaagggaatattcggtatttgttaatgccgctgctatcgttttattgccgagcaatcccgtggagtcagcaactaacgacctgatgaattcagtcctgcttgcacaactggtcgccaataagcgtgccgaagccacgagcgcggtcgattggtatgagacctatgtgggggtgctgggtgatttctggttaacgagggccagaagcaggcaagatatccagccgggaaaagacgataccgcttcaccgcttgaatggatcgctgcggtgctggcaagtagcactgaggatgaggcgcggctggtgacggcgttgttgaagggtatcgcacgactatccgattctttgcccgcgatgagtttgctgcgcaagcatgtgcaaaaagagtccgatgatgaaccggcagaaatctccttgcagtccaagcctgttcgcttggtcgtgatcgtggcccaagacaacgcttcgatgaccagcgtctgcctccaattcaaaacacggcaaatgcttgaccccaatccctgggggcagcgcttccatgtcgaggatatggagggctgcgtttcggcccattttttccatgcgcacctgtccgagacattgtacgcgcccgcccgtgaagcggtcgcccgcaaggttgagggcgttttgagcgacaacatcgtggatatcacggaggccatcgatgctttggcctttctgcccactgaggaggctggcacatga

SEQ ID NO: 178 - DNA, 786 bp, unknown
  Miscanthus rhizosphere microbial communities from Kellogg
atgaatgttcatgatgtcgaagattgcactgtagccgaatgtattcatcgtttggaaagttatgagctggacggcgctgaagttatgcgccctcgcagtttctcggtaccggttgtcaatgaacccggcaaaggttccatcgtgggtgagggcatcttgtcctttaccggcaacctgagtgagcaaaatcgggaagatgttcaacacgcttttctattcgcgagtctggtcgcaaacaaaaagtacccgtatgagtatcagggtaaggaatggtattaccagttcctggaagtcatgacccatgcaggctggctgccgaccagtaagtactacaacgacatgaacatcagcggtaacaccgtacggatggatcaattggtgctggagatcctcggcagtgtggttgccgggcttgccgtgcctggctccgcctccgtcctgatgctgaaggtggcaggcgatgcaatcaccgcattgaaaaaacgtgaaaccgcgttgaccctgtatgagcgcaacatgctggagcacggtgtgggtggtatggcggccggcacctgcaccgaagtcaacggtgaagtcaccatggcattgggtactgttcgtttcatccgcaagaacaccgcaaagcaagtgctgttcatggattgggactcccgcgaggtgaaactgtatcgcggtgactctgtcttcaggaaagtgccttatatcgtcgagcaaacccgcgacacgattcgtgcaaaacttggtttgaatgcgaaaccaaagatcgaagattacgacatctga

SEQ ID NO: 179 - DNA, 723 bp, unknown
  Miscanthus rhizosphere microbial communities from Kellogg
atgagttacgaatattctgtattgatcgttggggcttgtgtcgtgattattccggccgcggatggggcggcccaatatacggatctggtcaattccgtgttgctggcgcaactgattgccaataagaagatcgaaaaagctccggaaattgactggtacaacgcttatgtagaatttctggatgattactggctgcgacgtacaagagcgcgacaggattggtctatcgcccaagacagagtcgagtctgtcagcgactgggtcattgcagcgatttcacaagatgctgtggataaaggaagcgctactgcggcaacattgcagcggctggcaaggttgtccggcaacgagcctgcaatgggtttgctgcgcggtcacatgcagaaaatatccactgacgagtcgggtgatgtacttgcgcccgcaaaggctgtgcgtttgctggtggttatcgcgcagacgccgacatcggtcgcaagcgtctacatcgagcttaagacccgccagatcatcagtgccaatccgctggcccagcgacatctggctgaggatgtacaaggcagcgtttgcatgcgctacgccgctgctaacttgtccgaaactctctacagccctgtgcgcgacgccattgccttgaaggtcagggacaagtatcaggacaacgtagcgatgttgacattgagcgatgatgcttcggccatggagatctgtgcggtagattga

SEQ ID NO: 180 - DNA, 1668 bp, Pseudomonas rhodesiae
atggccaaactcacgcaattttccacccccgccgacatccaggacttcagtgacagccccgcccagcaagagcggatgaacgccgcctggagcggcaacatcaatcgctgggtcaacgcagcactggtgggcgacgtctgggacctgatcaactacggcccgcgcccggccttctacaaccctctggacaccgacaccccgagcacctcggtgaatgcccccatcacctggaacgccttccccgggcgcatccccgcgttgttccccaaccagtcggcgaactggctgcaatgggccgaccagggcgtgccggccaacgtcaccaccaacctctgcacccaacagagcgtccccccggcgccctactcgcccaccggcccccggggctggcaggacgaatactgtgaatggagcgtgacccgcaacgccgccgggcagatcaccagcgtgatgttcacctgtgagaacccggaatactggatgaccctgtggcaagtggacccgggcaaagtgctgcagcgctaccagcagttgatcaacccggcggtgcaactggccgacctgagcctcaaggacgcccagggccaaacggtgatcgacccggtgaccggagcgccgtgctacaacccgctgaacaagtggaacagcggcacccagaccctgcccggcagcggcggcgccatgcacctgaccagctcgcccaacaccctgggtgccgagtacgacctggcagcggccgcgaccatgccccgggagctgaacaacgaaccggtgacctcggcctcgcaactggtgtgctacgcccgttacgggcgcatcggccgccacagcgacccgaccatcggccagaacgtcaaccagtacgtcaactacacctccgggctgaccgaggtccgggcgaccctgaccaacccgccgggtctgtacatccagaccccggacttcagcggctacaccacccccgacggcagcccggcggcggcctgctggaccatcaaccgaggccacctggcgcagacctcggacgacatcgaccgcatcctccacgcgaccttcagcgtgcccgcgggcaaaaacttcaccgtcagcgacatcagcatcaacggtgcaaaaatccagtacgcctcgcagatcgccggcaccatcaccatgggcttgatggccacggtgtttggcaacagcggcgtgacccagcaaccggtggccggcaccctggacagcgacaaccccagcccgtcggtatcggcgctgcaaccgctgtcggtgttcaacgcctaccgggcccaggaactggccagcaacgagcaggcgctgtcgattccaatcctggccctggccatccgccccggacagcaagtggacaacatcgccttgctgctcaacaccagccagaccccgaacggcgccagcttcagcgtggtcgaaggcggcgtcagcatcagcatcaccggcacccaggacctgccggggttggacatgagcctgtacctggtgagcatcagcgccgacgccaacgccgccccgggggatcgcacggtcctcgccagcgtgcctggcatggccagcacccaacaggcggcgatcggcctgctgaccgtcggcggcccaaccctggtcacctcccagaccggcccgagcaagccgaacttccgtcgcggtcgcggctga

SEQ ID NO: 181 - DNA, 1356 bp, Pseudomonas rhodesiae
atgcgccgtcgtcccacggtgttactcggcctggccctgctactcggtttaccggccacccaggccatgggcgcgccgctgtgcggcagcccgttcgtcccctcgccgaccctgcaaccgacactcgccccccccaatttcagcgccagcgacagcgcggtggactgcttcatgtggcaaaccatggtctacctcaactggccggccaccccaggccaacggggcgtaccgaatgccgccgccagcctgggcagcccgggccccagcgtctggcagacctacaaggattacaacgagctgtacctgcccaatggccagcaaccgccagcctggaacgacaacttcctgtcggtgcagcgcttgcagacccgaggcgtggcacgggcgttgccgtcgatccgcctgcttaacagcaccagcaaggtctttcgcgccgccaatgccaacgaatccccggcgctacgggaaatcgagcaggtcggcggcggcgtgctctacgaccaggccggcagcccggtgtactacgaaatgctggtgaatgaggtcaacttcgacttcatctacaacaaccagctgtacaaccccgcccagcagaacctctatgccaagcaaaaaggcatcgtgctgccgaacaactccatcgagatcaaggccgcctggaaggtgctgagcgacccggataacccccagcgctttctcaccgcccaagcgttgctgcccggcagcagcacgccggtgaccgtgggcctggtcgggctgcatgtgttccagatgccttccagcgcgttcaaccaggggttctgggcgaccttccagcagctcgacaacgcccccacggtggccggcgccaccccaggggcgcactactcgttcaacaacccgcagtgcgcgccggcccagtgcccgcccaatgacaaaaccagcaatccgacccaggtggtgcagaacttcccgccgacgccagaggcgcagaacatcaaccactacatgcagaacctgatcgcccagcaggccccgggctccgcgttgcagtactaccagttggtggacgtgcaatggccgacttcgccacaagccatcggtcagcccggggccacggcgccggcgcccagtggcacgccgaaccacgacaccctgatcaacccggtgctggaaacctttctccaggccaatcacaagagctgcctgggttgccatgtgtacgccagcgtggcggcggacggcagcaacccgcccacccactaccaggccagcttcagcttcctgctgggccacgccaaaagcccggccctgggaagcaacctgaaaagcctggcgcaacagatcgaggacgcgtccctgagcctgcaacactga

SEQ ID NO: 182 - DNA, 1668 bp, Pseudomonas orientalis
atggccaaactcacgcaattttccacccccgccgacatccaggacttcagtgacagccccgcccagcaagagcggatgaacgccgcctggagcggcaacatcaatcgctgggtcaacgcggcactggtgggcgacgtctgggacttgatcaactacggcccgcgcccggccttctacaaccctctggacaccgacaccccgagcacttcggtgaatgcccccatcacctggaacgccttccccgggcgcatccccgcgctgttccccaaccagtcggcgaactggctgcaatgggccgaccagggcgtgccggccaacgtcaccaccaacctctgcacccagcagagcatccccgcggcgccctactcgcccaccggcccccggggctggcaggacgaatactgtgaatggagcgtgacccgcaacgccgccgggcagatcaccagcgtgatgttcacctgtgagaacccggaatactggatgaccctgtggcaagtggacccgggcaaagtgctgcagcgctaccagcagttgatcaacccggcggtgcagttggccgacctgagcctcaaggatgcccagggacaaacggtgatcgacccggtgaccggagcgccgtgctacaacccgctgaacaagtggaacagcggcacccagaccctgcccggcagcggcggcgccatgcacctgaccagctcgcccaacaccctgggtgccgagtacgacctggcagcggccgcgaccatgccccgggagctgaacaacgaaccggtgacctcggcctcgcaactggtgtgctacgcccgttacgggcgcatcggccgccacagcgacccgaccatcggccagaacgtcaaccagtacgtcaactacacctccgggctgaccgaggtccgggcgaccctgaccaacccgccggggctgtacatccagaccccggacttcagcggctacaccacccctgacggcagcccggcggcggcctgctggaccatcaaccgaggccacctggcgcagacctcggacgacatcgaccgcatcctccacgcgaccttcagcgtgcccgcgggcaaaaacttcaccgtcagcgacatcagcatcaacggtgcaaaaatccagtacgcctcgcagatcgccggcaccatcaccatgggcttgatggccacggtgtttggcaacagcggcgtgacccagcaaccggtggccggcaccctggacagcgacaaccccagcccgtcggtatcggcactgcaaccgctgtcggtgttcaacgcctaccgggcccaggaactggccagcaacgagcaggcactgtcgattccgatcctggccctggccatccgccccgggcagcaagtggacaacatcgccttgctgctcaacaccagccagaccccgaacggcgccagcttcagcgtggtcgaaggcggcgtcagcatcagcatcaccggcacccaggacctgccggggctggacatgagcctgtacctggtgagcatcagcgccgacgccaacgccgccccgggggatcgcacggttctcgccagcgtgcctggcatggccagcacccaacaggcggcgatcggcctgctgaccgtcggcggcccaaccctggtcacctcccagaccggcccgagcaagccgaacttccgtcgcggtcgcggctga

SEQ ID NO: 183 - DNA, 1356 bp, Pseudomonas orientalis
atgcgccgtcgtcctacggtgttactcggcctggccctgctactcggcttaccggccacccaggccatgggcgcgccgctatgcggcagcccgttcgtcccctcgccaaccctgcaaccgacactcgccaaccccaatttcagcgccagcgacagcgcggtggactgcttcatgtggcaaaccatggtctacctcaactggccggccaccccaggccaacggggcgtaccgaatgccgccgccagcctgggcagcccgggccccagcgtctggcagacctacaaggattacaacgagctgtacctgcccaatggccagcaaccgccagcctggaacgacaacttcctgtcggtgcagcgcttgcagacccgaggcgtggcacgggcgttgccgtcgatccgcctgcttaacagcaccagcaaggtctttcgcgccgccaatgccaacgaatccccggcgctacgggaaatcgagcaggtcggcggcggcgtgctctacgaccaggccggcagcccggtgtactacgaaatgctggtgaatgaggtcaacttcgacttcatctacaacaaccagctgtacaaccccgcccagcagaacctctatgccaagcaaaaaggcatcgtgctgccgaacaactccatcgagatcaaggccgcctggaaggtgctgagcgccccggataacccccagcgctttctcaccgcccaagcgttgctgcccggcagcagcacgccggtgaccgtgggcctggtcgggctgcatgtgttccagatgccttccagcgccttcaaccagggattctgggcgaccttccagcagctcgacaacgcccccacggtggccggcgccagcccaggggcacactactcgttcaacaacccgcagtgcgcgccggcccagtgcccgcccaatgacaaaaccagcaatccgacccaggtggtgcagaacttcccgccgacgccagaggcgcagaacatcaaccaatacatgcagaacctgatcgcccaacaggccccgggctccgccttgcagtactaccagttggtggacgtgcaatggccgacttcgccacaagccatcggtcagcccggggccacggcaccggcgcccagtggcacgccgaaccacgacaccctgatcaacccggtgctggaaaccttcctccagaccaatcacacgagctgcctgggttgccatgtgtacgccagcgtggcggcggacggcagcaagccggccaccgactaccaggccagcttcagcttcctgctgggccacgccaaaagcccggccctgggcagcaacctgaaaagcctggcgcaacagatcgaggacgcgtccctgagcctgcaacactga

SEQ ID NO: 184 - DNA, 1671 bp, Pseudomonas sp. PKRS11
atggccaaactcgcgcaattctcgcctcccgcccgtatccaggacttcagcaacgaccccgcccagcaggagtgtttgaacgctgcctggagcggcaacatcaatcgctgggtcaacgccgccctgctgggggacgtctgggatcgaatcaattacggaccgcgcccggcgttctacaatccgttggtgaccgatacccccgacaccgcgggcaatgtgccgatcacctggaacgccttccccggccgcctgcaagcgctgtttccgaaccagggcgcgtcgtggcaacagtgggccgaccagggcgtgccggataaagtcaccaccgacctctgcagcggcaagcccattgacccggccccctactcgcccaccggtccacggggctggcaggacgaatactgcgaatggagcgtgacccgcaacggtgccggacagatcaccagcgtgatgttcacctgcgaaaaccccgagtactggatgaccctgtggcaggtcgatccgggcaaggtgctgcagatctaccagcaggtgatcaacccggcggtgcaactgtcggacctgtgcctgaaagacagccatggccagacggtcaacgatccgctcaccggccagccgtgctacaacccgctgaacaaatggaacagcggcacccgcaccctggcgaacagcggtggcgccatgcacctgaccagctcccccaataccctcggcgcggaatacgacctggccgccgcggccaccatgccgcgcgaaaaggaccacgacccggtgacctcggccgcagccctggtgtgctttgcccgctatggccggatcggccgccacagcgatccgaccattggccagaacgtcaaccagtacgccaactacaccccgaccctaccgcatccccaggccaccctcgccgaccctccggggctgtacatgcagaccccgcagttcagcgactacgtcacccccgacaacaccccggcgcagactttctggaccgtggtgcgtggcagcctgaaagacccgaatacgtccgaggacatcgatcgcatcctgcacgccaccttcagtgtccctccggaactgggctacaccgtcagcgacatcaagatcggcaaccagccgatccggtacggctcgcagatcgccgccaccatcaccatggccctgctggccacggcctttcccaacagtggagtggtgcagaccccggtcggcgcgacgctcgacaactcgaaccccagcccctcggtcagcgccctgcaggcacttgcggtgttcaccgcgtaccgggcccaggagctggccagcaatgaacaaccgctgtcgataccggtactggctctggccgtcagtccggggcagcaggtgagcaatatcgccctgctgctcaacaccagcgacaccccggatggcgcggtgttcacggtgcccgaaggcggggtaagcatccgtatcgacggcacccaagcgctacccaatgcggagctgagcctgtatcaggtgacgctgtgcgtcgacgccaatgccgccatcggcgaccgcagcatcctggccagcgtgccgagcatgccagccacccaacaggcggccatcggcctgctgacggtcgtcgccccgccccaggtccggcttgccggcggaccgcgcaaacctcacgcccgtcacagtcgctaa

SEQ ID NO: 185 - DNA, 1350 bp, Pseudomonas sp. PKRS11
atgcgtgccattctcgccctcttgctgtacgccggattgtcgctggcgccggtcgcggcccgggccgccggcaatccctgtggcagccccttcagcccggaaccggtcatccagccggtcctggccaacccgcagataagcaacctggacccgtcggtggactgcttcatgtggcaaaccatggtctacctcaactggccggcccaggccggccagcgtggtctccccaataccgacgcgcacctgggcgaccccggccccacggtctggcaaaccttcaaggacttcaacgaactctacctgcccggtggccagcgcccggccccctggaacgacaacttcctcaccatgcaacgcctggaattgcgcggcgtggagcggccaaggccatcgatccgcctgctcaacagcaccagcaaggtgtttcgcaatgccgatgccagcgaacaaaaggccctggacgaattcaagcaagtgggcggcggcgtgctctacgaccagaacggccagccggtgtactacgagatgctgatcaaccagatcaacttcgattacatctacagcaatcagctgtacaacgctgcccagcagaatctccacgccgccaagcagggcatcgtcctgcccagcaactccatcgaactcaaggcggcctggaaagtcctcagcccccaggaagccgcgccgcccttgcgctttctcactgcccaggccctgctcccgggcagccaggtgccggttaccgtcggcctggtgggcctgcacgtgttccagatgccctccaaggacttcgcccagggcttctgggcgaccttttcccaggtggacaacgcccccaccctgaatacacctggccaggcccattactcgttcaataacccgcagtgcagccagtgtccggtcaacgaccttggcagcaagccgacgcaggtggtgcaggtccaggccaacgccgtctacgcccaggccgtcaaccagtacatgcaggcgctgatccagcagcaggcgccgaactcggccttgcagtattaccaactgatcaacgtgcagtggcccaactcatcggtacccatcggccagcccggccagccgacacctgcgccaaccggcagcccgagcaccgacaccctggtcaatccggtgctggaaacctttatgcaggtcagcaacatgagctgcctgggttgccacaagtccgccagcgttgccgacaatggcacgcagccgcccagcggctatcaggcaagctacagtttcctcctgggccacgcccagaacccgccgccgcaaggcagcctcaagagccttgcgcgacaggtggaagaagcctcgacagcccgtcaacggtag

SEQ ID NO: 186 - DNA, 291 bp, Pseudomonas Antarctica
atgaaattatcaaatgtcttactattgagtatcgtatttgcttggcaaggcatggccttcgccgatacacagaagtctaatgccgaaaccttgttatctaacgacaaaccaccgctaacacaggcggcgcaggagaaggaacaagaaaatgttgaggctgaccggaatgaatgttggtccgctaagaattgttctggaaagatcctaaacaataaagatgcgcacaactgtaaattatccggcggtaagtcatggcggagcaagactacagggcaatgcactaatctttaa

SEQ ID NO: 187 - DNA, 291 bp, Pseudomonas orientalis
atgaaaatgtccagcgtcttactgatgagtattgcgtttgtatgtcaaggcatggtcttcgctgatacacagaagtccaatactgaaaccttgttttccaacgacaagccaccgctgatacagacggcccaagagcaggaacaaaaagaggttgaggttgaccgcaatcaatgttggtccgccaagaattgctctggaaagatcctgaacaataaagatgcacataactgtaagttgtccggcggtaagtcttggcggagcaagactacagggcagtgcaccaatctgtag

SEQ ID NO: 188 - DNA, 288 bp, Enterobacter asburiae
atgaaaacactcgttatcgcaattctcaccgctgttctttgccagggcatggcgatggctgatacacagaaaccagcaaccggggctttgccagcaaatgaaaaaccccctctcgttcagccagctgacgaacataaaacgagcgaggcaaatgccaatcgtaatgaatgctggtcagcaaaaaattgtaccggaaaaatccttaataataaggatgcgcataattgcaaaaactccgggggtaaatcatggcggagtaaaaccaccggacagtgtaccaatctttga

SEQ ID NO: 189 - DNA, 288 bp, Enterobacter sp.
atgaaaacactcgttatcgcaattcttaccgctgttctgtgccagggcatggcgatggccgaaacgcagcaaccggcatccggggctttgcctgccaatgaaaagccgcccctggtgctgacggccgacgaaaaaaaagcgagtgaggctaatgccgacaggaatgaatgctggtcggccagaaattgtagcgggaaaatccttaataataaggatgcgcataactgcaaaaactccgggggtaaatcctggcggggtaaaaactccagccagtgcaccaatctttaa

SEQ ID NO: 190 - DNA, 318 bp, Acidovorax avenae
atgaaaaagctgttgctcatcgcttcgttactcgtttccatttccggtgcgaatgtgttcgcccaggcaccgtcatccggcgatgctcccgcagccgtcgcgggcaagcaggatggggcctcgcacaaagacacggaacaggcggccaatgtggaatgcgacgtcaatgcgaccgtccagcagtgctgctctgccgccaaatgccaggggaaagtgctcagcaatcgcgatgcccacaactgcaaggacaagtccaagggcaagagctggcatgcggcggcgcaagggggacagcccgctgcgtgccagcggatgtaa

SEQ ID NO: 191 - DNA, 285 bp, Serratia plymuthica
atgcagtgtaatggggctattttaaagttgttgtgcgcgcaacgaaaagaccaatttatgaacttacgcataaggacacatgctatgaaaaatttgtcgattttagttgttctatcttcctgcctcttacttcctttaaccgcgtctgcggctgctggtacgtgctatagtgcgaagaactgctccggtaaagtgttaagccatcgagatgcacataactgcaaggtcaaggataagggtaagtcttggcgcagtgatatcacaaatcaatgtaccaacctgtga

SEQ ID NO: 192 - DNA, 282 bp, Serratia liquefaciens
atgcgtgaggaggctattttaaagttgttgtgcgcgcaacgaaaagaccaatttatgaattcacgcataaggacacatgctatgaaaaatttgtcgattttagttgttctatcttcatgcctcttacttcctctaactgcgtcggcggcgtccggtaagtgctacagtgctaagaactgttctggaaaagttttaagcaaaagagacgcgcataactgcaaggtcaaggatcggggcaaatcttggcttagtgatgtcacaggcaaatgtaccaacctgtga

SEQ ID NO: 193 - DNA, 237 bp, Serratia sp.
atgaaacttaaatatgaacgaataaggatatatgttatgaaaagtctatcgattgttattactctcgcttcatgcttactgctacctctgactgcgtctgcggccgcaggcacatgttatagcgcaaagaactgttccgggaaggtgcttagccaccgggatgcccataactgcaaggttaaggacaaaggtaaatcctggcgcagtgatattacaggccaatgcacgaatctttga

SEQ ID NO: 194 - DNA, 228 bp, Serratia sp.
atgaattcacgcataaggacatatgctatgaaaaatttgtcgattttagttgtactatcttcatgcctcttactccctctaaccgcttctgcagctgctggcacatgctatagcgcaaagaactgctctggaaaagttttaagccatcgagacgcgcataactgcaaggtcaaggacaagggtaaatcttggcgcagtgatatcactggcaagtgtaccaatctgtaa

SEQ ID NO: 195 - DNA, 270 bp, Pseudomonas chlororaphis
atgtcggctcaagagaactttgttggcggatggactccttatcacaaactgaccccaaaggatcaggaagtattcaaagaagccctggccgggttcgtgggtgtgcagtacacacctgaactggtttcgacccaggtcgtcaacggcacgaactatcgctatcaatcgaaagcgacgctgcctggctcgtcggaaagttggcaagcggtagtggaaatctacgcgcctatcaaaggcaagccgcacatcacccagatccaccggatctaa

SEQ ID NO: 196 - DNA, 270 bp, Pseudomonas chlororaphis
atgtcggctcaagagaactttgttggcggatggactccttaccacaaactgactccaaaggatcaggaagtattcaaagaagccctggccggattcgtgggtgtgcactacacgcctgaacaggtttcaacccaggtcgtcaacggtacgaactaccgttatctgtcgaaagcaacggtgcctggctcgtcggacagctggcaagcggtcgtagaaatctacgcgcctatcaagggcaagccgcacatcacccagatccaccggatctaa

SEQ ID NO: 197 - DNA, 270 bp, Pseudomonas brassicacearum
atgtcggctcaagagaactttgttggcggatggactccttaccacgaactgactccaaaggatcgggaagtattcaaagaggccctggccgggttcgtgggtgtgcaatacacccctgaaaaagtttcgacccaagtcgtcaacggcacgaactatcgttatctgtcgaaagcaacggtgcctggctcgtcggacagctggcaagccgtagtggaaatctacgcgcctattaaaggcaagccgcacatcacccagatccaccggatctaa

SEQ ID NO: 198 - DNA, 270 bp, Pseudomonas chlororaphis
atgtcggctcaagagaactttgttggcggatggactccttaccacgaactgactccaaaggatcgggaagtattcaaagaggccctggccgggttcgtgggtgtgcactacacccctgaaaaagtttcgacccaagtcgtcaacggcacgaactatcgctatctgtcgaaagcaacggtgcctggctcgtcggacagctggcaggccgtagtggaaatctacgcgcctattaaaggcaagccgcacatcacccagatccaccggatctaa

SEQ ID NO: 199 - DNA, 270 bp, Pseudomonas chlororaphis
atgtcggctcaagaacattttgttggcggatggactccttaccacgaactgacgccaaaggataaagaagtattcaaggaagccctggccgggttcgtgggtgtgcactacacccctgaaaaggtttcgacccaggtcgtcaacggcactaactaccgttatctgtccaaagccacgctgcctggctcctctgacagctggcaggcggtagtggaaatctacgcgccgatcaaaggcaagccgcacatcacccagatccatcggatctaa

SEQ ID NO: 200 - DNA, 270 bp, Pseudomonas fluorescens
atgtcggctcaagaaaatcttgttggcggatggactccttaccacgaactgactccaaaggatcaggaagtattcgatgaagccctggccgggctcgtgggtgtgcactacaccgccgagctggtttcgacccaggtcgttaacggcaccaactatcgttatcagacgaaagcaacgcagccgggttcatcaaacagctggcaagcggtcgtggaaatttacgcgcctattaacggcaagccgcatatcacccagatcattcggatctaa

SEQ ID NO: 201 - DNA, 270 bp, Pseudomonas fluorescens
atgtcggctcaagaaaatcttgttggcggatggactccttaccacgaactgactccaaaggatcaggaagtattcgatgaagccctggccgggctcgtgggtgtgcactacaccgctgagctggtttcgacccaggtcgttaacggtaccaactatcgttatcaggctaaagcaacgcaacctggttcgccaaacagctggcaagcggtcgtggaaatttacgcgcctattaacggcaagccgcatatcacccagatcatccggatctaa

SEQ ID NO: 202 - DNA, 270 bp, Pseudomonas fluorescens
atgtcggctcaagagaatctcgttggcggatggactccttatcacgaactgactccaaaggatcaggaagtattcgatgaagccctggccgggctcgtgggtgtgcactacacggctgaactggtttccacccaggtcgtcaacggcaccaactatcgttatcaggcgcaagcaacgcagcctggttcgccaaacagctggcaagcggtcgtggaaatttacgcgcctattaacggcaaaccgcacatcacccagatcatccggatctaa

SEQ ID NO: 203 - DNA, 270 bp, Pseudomonas fluorescens
atgtcggctcaagaaaatctcgttggcggatggactccttatcacgaactgactccaaaggatcaggaagtattcgatgaagccctggccgggctcgtgggtgtgcactacaccgctgagctggtttcgacccaggtcgttaacggtaccaactatcgttatcaggcgaaagcaacgcagcctggttcaccaaacagctggcaagcggtcgtggaaatttacgcgccgattaacggcaagccgtatgtcacccagatcatccggatctaa

SEQ ID NO: 204 - DNA, 270 bp, Pseudomonas fluorescens
atgtcggctcaagaaaacctcgttggcggatggactggctaccacgaactgactccaaaagataaggaagtattcaaagaagctctggagggactcgtcggtgtgcattacacacctgaactggtttcgagccagatcgttaatggcactaattatcgctatcaaactaaagcgacccagccaggctcgtcaacgagctggcaagccatcgtggaaatttacgcgcctatcaagggcaagccgcatatcactcagatcatccggatctaa

SEQ ID NO: 205 - DNA, 270 bp, Pseudomonas rhodesiae
atgtcggctcaagaaaatctcgttggcggatggactccttatcacgaactgactccaaaggatcaggaagtattcgatgtagctctggccgggctcgtgggtgtgcactacaccgctgagctggtttcgacccaggtcgttaacggtaccaactatcgttatcaggcgaaagcaacgcagcctggttcaccaaacagctggcaagcggtcgtggaaatttacgcgcctatcaacggcaagccgtatgtcacccagatcatccggatctaa

SEQ ID NO: 206 - DNA, 270 bp, Pseudomonas sp.
atgacagctcaagaacatcttgttggtggatggaccccttaccacaaactgactcccaaggatcaggaagtcttcaaagaagcactggccggcttcgttggcgtgagctacacgcccgaagaggtttccagccaagtcgttaatggcaccaactatcgctacaagtcgaaagccacgcttccgggttcgccaaacggctggcaagcgatcgtagaaatctacgcgccaactaatggcaagccgcacatcactcagatccatcggatctaa

SEQ ID NO: 207 - DNA, 276 bp, Pseudomonas fluorescens
atgtcagctcaagaaaaccacgttggcgttggcggatggactgcttaccacgaactgaccccaaaggaccatgctgtattcaaagaggccttggaaggctttgtgggggtgcaatacacccctgagacggtttcgactcaggtcgtcgccggcacaaactatcgctatcactcgaaagcacagcagcctggttcgccagcaatctgggcagcaatcgtggaaatctacgcccccctcaaaggtaaaccgcacatcacccagatcatccgcatctaa

SEQ ID NO: 208 - DNA, 279 bp, Enterobacter-sp
atgtcggaacaacaaacgctgctgcctggcggctggacggcttatcatccgctgactgctcaggaccgaaaagtgttcgaagaggcgctcaacgggcatctgggcgtggattacgagccacaaaaggtaaaaacccaggtcgtggccggaacaaactaccgcttcctttgtgaggcttcggtcccgccgtctacggccgtctgggaagcgatagtggaaatttatgcgccattaccgggacagggcgccccgcatattactcaaattatcagaatttag

SEQ ID NO: 209 - DNA, 270 bp, Shewanella denitrificans
atgtcaaataatgaaactatcgttggtggttggacagcttacaacgcaatcacatctgctgaaagagaaattttcaataaagccatggagggttttgttggtgtaagttacatgccagagacggtttcaacccaggttgttgcgggaatgaattatcgttttaaatgcgaagcgtctatgccaccatcagaagtgttatgggaagcaattgttgaaatatatcagccattaaagggcatcccgcacatcacaaacatcacaaaaatataa

SEQ ID NO: 210 - DNA, 273 bp, Aeromonas diversa
atgtcggatcaagctgtgctggttggcggatggactgcatatcacaggctgactgcggaagaccaagcggtgtttcaggaagcgctgaaaggatttgttggggtggagtataagccctttgaagtttccacccaggtggtagcgggtatgaactaccgctacaagtgcaagaccacggtacccttgccgactccgatccatggcgaagccgtggtacagatcttccagtcgctggacggctctgcccatatcacctccatcactcccatctaa

SEQ ID NO: 211 - DNA, 273 bp, Aeromonas salmonicida
atgtcagaacaagcagtgttggtgggtggatggaccgcatatcacaagctgaccgccgaggatcaggcggtatttgaccaggcgctgaaaggatttgtcggggtgcagtacgtaccctttgaagtctgcacccaggtggtggccggcaccaactaccgcttcaagtgcaagagcacagtgccgcttgccaaaccgatccatggcgaagccgtggtgcagatcttccagtctctggatggctcggcccatatcacctccattaccccgatctga

SEQ ID NO: 212 - DNA, 273 bp, Aeromonas veronii
atgtcagaacaagcagtgttggtgggtggatggaccgcatatcacaagctgaccgccgaggatcaggcggtatttgatcaggcgctgaaaggatttgtcggggtgcagtacgtaccctttgaagtctccactcaagtggtggctggcaccaactaccgcttcaagtgcaagagcactgtgccgcttgccaaaccgatccatggcgaagccgtggtacagatcttcaaatcactggacggggatgcccatatcacctccattaccccgatctga

SEQ ID NO: 213 - DNA, 267 bp, Aeromonas molluscorum
atgtcagaacaagcagtgctgttgggcggatggactgcctaccacaagctgagcgccaaggatcaggcggtattcaaccaggcgctggaaggatttgtcggggtgcagtacacaccctttgaagtctccacccaggtcgtcgccggtaccaactaccgcttcaaatgcaagagcactgtgccgctgcccaaccccatccacggggaagccgtggtgcagatcttccaggcgttgtttcccaaatcgatgcagcttgaatggaactaa

SEQ ID NO: 214 - DNA, 273 bp, Aeromonas aquariorum
atgtcagaacaagcagtgttgttgggcggatggactgcctaccacaagctgagcgccaaagatcaggccgtattcaaccaggcgctggaaggatttgtcggggtgcagtacaccccctttgaagtctccacccaggtcgtcgccggcaccaactaccgtttcaaatgcaaaactactgtgccgctgcctaacccgatccacggagaagccgtagtgcagatcttccagtcgctggatggctcggcccatatcacctccattaccccgatctga

SEQ ID NO: 215 - protein, 5 aa, Artificial Sequence
  Cleavage linker
EEKKN

SEQ ID NO: 216 - DNA, 16 bp, Artificial Sequence
  16S riibosomal primer
taccttgttacgactt

SEQ ID NO: 217 - DNA, 20 bp, Artificial Sequence
  16S ribosomal primer
agagtttgatcmtggctcag

SEQ ID NO: 218 - DNA, 1737 bp, Pseudomonas sp. VLB120
atgagcacgtccttcacacagttcacctcgcccgccggccaagcccccaaggactacaacaagctgggcctggaagaccagttgccgcagtttgaaaccgactggaacaacaacctcaccggctggacccaatcgtccatcatcggcaacccctggtccaacctgaacgacgccccccgctcgggttactacaatccgctcgtcgaaggcttcggtgacgtgactgtccccgcgatcacctgggcgcccttccccaaccggctctggacgtttttctacaacaacggtgcggcgatcgttccccaactgggcggcaacgccatgactctggagcaggtgatggaattggccgatcacggccagatcaccctcaacaacaccctctacaaactctacgatcccgacaaccaagggaccttgctgcaactgccggccaagcgctgccccagcatcgactggaaaggccagtacacggcgttctcgccctccggcccacggggctggctcgacgagtactgcgagtggtccatcgtgcgcgataccgacggcaacatgcgcaagatcacattcacctgcgaaaaccccgcctatttcctggccatgtggcgcatcgatccgaacgcggtactgggcctgtaccgggactacatcgacccgaacgtacaactcgaagacctgtacctgcgctatgccgtcgattgcccgaccggcaaggccggagatccagtgatcgaccccaccaccggccagccggcctatgacacggtcaacaaatggaacgccggtacggcctgtgtacccggccagtacggcggcgcgatgcacctgacgtccggccccaacaccctcagtgccgaggtgtacctggctgccgccgccaccctcctgcgaccggtgagcagcagccagaacgcccagtcgctgatctgctgcgcgcagtacggacagaactatcgcaactccgacccgcacatcggcttcatggccaataccaaggcggtgaacaatcggctgtcgctgaccaaccccattggcctgtacctgcaacagcccaccgatttcagcgcctggaaaggcccgcagggccaggacgtgagccagtattggcgcatcacgcgcggcacggccaagtcggcggccaacggctccgaccagatcctgcaggcggtgttcgaggttccgcaaagcgcaggcttctcgatcaatgacatcaccatcaatggccaacgggtcgactatgtgtgggtcatcgcccaacaactgctggtgggcctgagcgtcaccgccaagccgatcaccgtcacacccccgtcgttcccttgcgtacaggcgcgggttgaggggctgcaaccctggccggttcaactgctgccagtagacctgttctacggacaatcacccaccgacctgcccgcctggcttgcaccgggaagcagcaactcgttcgtactggtggtgcagggcgccgacccgagcaccacgacgcagaatgcacgggtgcaattctccaaccccggcatcacggcgcaggtcacccactacctgccagacgcatccgccattcccggacagaccaactccggcggtacccaggcctacatcctcaccatcacggtgagcccgacggcagcacccggtctggtcatggtgcgcgcgctcaatccgggcgaagacgcgaacgtgagcgcggccgatcacccttgggaggccggcctggcgctggtgcccggcgcctga

SEQ ID NO: 219 - DNA, 1605 bp, Pseudomonas sp. VLB120
atgtccaggtcacgcttgagtctcatctcgctgttgagcggcatgttgctgtatctgtcggccctgcctcccgctgcggcagccacgatgtcggatgccgacagctgtgtgcagcagcaattggtgttcaatccggccagtggagggttcctgccggtcaacaacttcaatgccaccaaccaggcattcatgaactgttttgcctggcagttgttcatcgccctgaattggccggtcaatcccggctggcctgccaccgccagcctggcgggtgaacccgacatgaacagcaccctggcgcaattcggagtgccctcttccccggggcaacccatgagcgtggcgcccgtgtgggccagctacaaagatgccaacgacatcttcctgcccggcgcgcccacgcccaccggttggggcgtgcaaaccatggtaccgtccggttgcagcacccagggcagtctgaaggccctgaaggtaggtgcacgcaagttcatgaatgccacctcagaaggcgcgatcaacgccttgcatggtttccacctctcgaccgggacggtcgcttctattcccgaccccgtcatggaagcgtccggcggctggctgacggaccagtctggcaacttggtgttctttgaacgcaaagtgggcaaggccgagttcgactacatcgtcgagaaggggctctatgatgccgccaatcagttgaaggtcgcgcaaaacctcgatggcaatacaccggaaggcctgtcgctgcccctcggcgagccaatgcgttcgctgccgccgacccctgtgccacaggagcagctgggcgcgcttgagctcaaggccgcgtggcgtgtgctgaccggcaaacccgagctgttcgggcgctacctgaccaccgtcgcctggctcaaacgccccgacacactggagtgcacccaggaagtggtggggctggtgggcctgcatatcatcaacaagacccaggcgtcgcccaatttcatctggaccaccttcgagcaggtggacaacgtgcccgaaccggaccaggccccgccgcaaggaaccccgccgaacggtttctctttcaacaaccccgactgtgggagcggccctgcgtgtgaacccaatgtggctcgtatccagtgcaagcaataccaccccgacaaggactgcaccgatctctttccacgcgaccagccggtacagaccacccgtgagcaccccgtccccagcgacctgcaagccctgaacagcgcggtgcaatccaactttgcacagcagacccacggccagtcggtgttccagtactacaagctgatcaacgtactgtggaccctcgcgcccaatcctcccagcccggagccgggcgccaatgcccaggtgccgctgtcatacgggccgttcatcagtcagggcaacgtgccggtggccaacaccaccatggagacttacgtacagggcgatgactgcaacaaatgccatcagtacgcgacgattgccggcagcccctccttggcctcggacttctccttcctgttcaacagcgcgagttccgccggccataaaagcctgatcaagcgcgtcaaagccttcgaaacgctcaaggaccgcccctga

SEQ ID NO: 220 - DNA, 1734 bp, Pseudomonas putida
atgagcacgcccttcaagcagttcacctctcccgctggccaagcccccaaggactacaacaagctaggcctggaggaccagttgcagcagtttgaaaccgactggaacaacgacctcaccggctggaccgagtcgtcgatcatcggcaacccttggtcgggccagaacgacgcgcctcgctctggctattacaacccgctggtggagggtttcggtgaagtgaccccgcccgcgatcacctgggcgcccttccccaaccggctgtggacgttcttctacaacaacggtgcagcggtcgttccgcaacttggcagagccatgaccctgaaccaggtgatggagctggccgaccgcggccagatcaccctcgacaacaccctctacacgctatacgacccggacaaacagggcaccctgctgcaactaccggccaagcgctgcccaagtatcgactggaacggcaggtacacggcgttctcaccttccggcccgcggggctggctcgacgagtattgcgagtggtcgatcgtacgcgatgccaacggcaacatgcgcaagatcaccttcacctgcgaaaaccccgcctacttcctggccatgtggcgcatcgacccgcaggcagtattgggcctgtaccgcgactacatagaccccagcgtgcaactcgaggacctgtacctgcgctacaccgtcgactgcccgaccggcaaagccggcgatccggtcatcgacccgaccactggccagccggcctatgacaccgtcaacaaatggaacgccggcaccgcctgcgttcccgggcaatacggtggtgcgatgcacctgacctccggccccaacaccctcagtgccgaggtgtacctggccgccgccgccaccatcctgcgcccggtcagcagcagccagaatgcccagtcgctgatctgctgcgcgcagtatgggcagaactaccgcaactccgacccgcacatcggcttcatggccaattcgacggcagtgaaaaatcgcctgtcgctgaccaacccgattggcctctacctgcagcaacctaccgatttcagtggctggaaaggcccgcaaggccaggacgtaagccagtactggcgcatcacccgcggcaccgccaagtcggccgccaacgggtccgaccaaatcctgcaggcggtgttcgaagtcccagaaagcgccggtttctcgatcaacgacatcaccatcaacaaccagccggtcaactatgtgtgggtcatcgcccagcaactgttggtgggcctgagcgtcaccgtcaagccgcttgctaccacaccgccctccttcccgtgcgtgcaggaccggcagaccggccggcaaccctggccggtgcagctgctgccactggacttgttctacgggcagtcccccaccgacctgcccgcctggctggcaccgggtagcagcaactcgttcgtgcttgtggtgcaaggcgcagacgccaacaccacggcgcagaacgccagggtgcaattctccaaccctggggtgacggcacaggtcacccagtacctgcccgacgcgtcggcgattcctggccagaccaactctggtggcactcaagcctacatgctgaccatcacggtcagccccaacgcagcacccggcctggtgacggtgcgtgcactgaacccgggcgaagacgtgaacgtaagcgcggcagaccacccgtgggaatccggcctggcgctggtgcctggcgcctga

SEQ ID NO: 221 - DNA, 1590 bp, Pseudomonas putida
atgatgtccagcttacgcctgagccttctgtcgctgctcagcggcatcctgctttgcctgcagaccctgcaacccgctgctgcggccacgctgtcggacgccgatgcctgtgtgcagcaacagttggtgttcaaccctgcgagcggggggtttctgccggtcaataacttcaatgccaccagccaggcgttcatgaactgcttcggctggcaactgttcattgccttgaactggccagtaaaccccggctggccggccacccccagcctggcgggcgaacccgacaggcaaagcaccctggcgcagttcggtgtgccgaccacggcgggtgaaccgatgagcgtggccccggtgtgggccagctacaaggacgccaacgatatctttctgccaggcgcgcccgcgcccaccggttggggggtacaaaccctggtaccaagcagctgcaatagccagggtagcctgaaggcgctcaaggtgggtgcgcgcaaattcatgaacgctacctcagaaggcgcgatcaacgccctgcacgggttccacctgtctaccgggacactggcatccattcccgacccggtcatggaagcgtccggcggctggctgacggatcagtcgggcaacctggtatttttcgaacgcaaggtaggcaaggccgaattcgactacatcgtcgagcatgggctatatgacgcggccaaccagttgaagctcgcccaaaccgaggggctgtcgctgcccatcggtgaagcgatgcgcgaactgccgccgtcgcctgtgccgcaggagcaactgggcgcaatcgagctcaaggccgcctggcgggtgctgactggcaaacccgaactgttcggtcgctacctcaccaccgtcgcctggctcaagcgccccgacaccctggcatgcacccaggaagtggtgggcctggtgggcctgcacatcatcaacaagacccaggcttcgcccaacttcatctggaccacgttcgagcaggtggacaacgtgcccgaacctgcccaggtgccgccgcagcaaaccccgccgggcggttttgcgttcaacaaccccgaatgtggcaccggccccgagtgtaaaccgaacgtggcccgtatccagtgcaagcaacaccaccccgaccgcgactgcagcgacctcttcccgcgcgaccagccggtacagaccacccgtgaataccccgtgcccagtgccctgcaggccctgaacagcgcagtgcaagccaacttcgcgcagcaaagccagggccagtcggtgttccagtactacaagctgatcaatgtgctgtggacccttgcccccaacccacccagcccagaaccgggtgccaacgcacaggtgccgttgtcctacgggccgttcatcagcgagggccccgtgccagtggccaacaccaccatggaaacctacgtgcagggtgatgactgcaaccagtgccatcagtacgcgaccattgccggcagtccctcgctggcttcggacttctcgttcctgttcaacactgccagctcggccagccagaaaagcctgatcaagcgcgtcaaagccttcgagaccctcaaggaccggccctga

SEQ ID NO: 222 - DNA, 1734 bp, Pseudomonas poae
atgagcacacccttcacccaattcacctcccctgccgaacaagcgcccaaggactacaacaagctcggcctggaggaccaattgccgaccttcgagaccgactggaacaacaacgtcaccggctggacccagatgtcgatcatcggcaacccctggtccaacctcaacgatgcaccgcgctcgggctattacaacccgctggagagcggctacggcacgctgacgccgaagaccatcacctggcagccctttcccaatcgcctctggacgttcttctacaacaacggcgccgccgtggtcccgcaactgggcggcaaggccatgaccctggaccaggtgatgcaactgaccgaccacggccagatcaccctcaataacaccctgtattcgctgtacccggacccgcaggcgacccaactgcagatccccagcgtgctgtgcaaatccatcaactggaacggcccctacgccgacttttcgccctctggcccacggggctggctggatgaatactgcgagtggtcgatcacccgcgaccccgacggcaacatgcgcagcatcatgttcaccagcgagaacccggcgtacttcctgaccatgtggaacatcgacccgggtgccgtgctgggcctgtaccaggcgtatgtcgacccgcaggtgaaactcgaagacctgtacctgcgctacaccgccgacggcccgaccggcaaggccggcgaaccggtgctcgaccccaccaccggccagcccgcctacgacaccgtgaacaaatggaacagcggcaccgtgcgcataccgggcgtgtcgggcggcgcgatgcacctgacctccggccccaataccctgagtgccgagatctacctggcggcggccgccaccatcctgcggccgctcagcagcagccagaaccagcagagcctgatctgctgcgcgcagtacgggcagaactaccgcaactccgacccgcatatcgggttctccgccaaccaggcggcggtcaacaacctgatctcgttgaccaaccccatcggcctgtacctgcagcaacccaagtccttcagcacctggaaaggcccgcaaggcgaggatgtcagcagctactggcgcgtcacccgtggcaccgccggcaccggcccgaacaactccgaccagatcctccaggcggtcttcgaagtgccggccagtgcagggttctcgatcaatgacatcaccatcagcggcacgccgatcgactacgtgtgggtgatcgccaacgaactgaatgtggccctcagcgtgaccccggcaccgctcaccgcccagcccaaggagtgcgcctgcgtggcggccaacaccaccgatgcgcagccctggccggtgcagttgctgccgattgacctgttctacggccaatcccccagcgacttgccggccagctttgcgcccggcagctcaagccagttcgtgctggtggtgcaaggcgccgacccgaacaccacggcggcggatgcacgggtgcagttctccaacccgggcatcacggcccaggtcacgcagttcctgccggatgcctcggcgattcccgggcagaccgacggcggcggcacccagggctacatcatgaccattaccgtcagcagcaacgcggcgccggggctggtcagcgtgcgtgcgctcaaccccaacgaagcggccaacccgagtgccaccgagcacccatgggaaagcggcctggccctggtgcccagcgcctga

SEQ ID NO: 223 - DNA, 1590 bp, Pseudomonas poae
atgaacggatggcttcgcccgctgcgccgggcacgcttgcgtattgtctgcacaatcacctgcgcccttctcccgtggctggcccccgcaccggcaagtgccgcctcggatgcccagagctgcgtcagccagttggtgttcgaccccaccagcggcggcttcctgccggtgaacaatttcggcaccgagcaggcttttctcaattgtttcggctggcagttgttcatcgccatgaactggccggtcaaccccggctggcccgccaacccgagcctggccggtgagccggatacgcaaagcagcgcggcccagttcggcgtgccgccaaccccaggccaaccgatgagcaatgccccggtgtgggccagctacaaggatgccagcgagatcttcctgcccggcgcggccaagccgtccggctggggcgtggaaaccctggtgccgtccaattgcaccgccaccggcaatctcaaggcgtttgccacgggcgcgcgtaaattcatcaccgccacctcggaaagcgcgatcaaccgcaagcaccgcttccacctgtccagcggcacccaggtgaccctgcccgattcgatcatggaagcctccggcggttggctaacggaccagtccggcaacctggtgtttttcgagcgcaaggtgggcaaggccgagttcgactacatcgtcgacaacggcttgtacgacgccgccaaccagctgatcgtggcgcagaacagcgacaaccggcaccccgccggcctgtcactgccggccggcaagctggtgcgtgaactgccggccaaggcgctaccccaggaggaactcggcgccctggaactcaaggccgcctggcgcgtgctcaccaacaagcccgccctatacgggcgctacctgaccaccgtggcctggctgcaacgcccggacacgctgcaatgcacccaggaagtgattggcctggtgggcctgcatatcatcaacaagacccagacccagccgaatttcatctggaccaccttcgagcaggtcgacaacgtgcctgacggtggtgccgcgccgcccgagggctacagcttcaacaacccggcatgcaccggtgatgcctgcacgccgaatgtgccccgcgtgcagtgcgacgccacgcacacgccgcccaactgcacgcccctcgaccagccggtgcaggccacccgcgccaacgccacgccccaggacatgcaggcgctgaacaccgcggtgcagcagaccttcgcccagcagacccagggccagtcggtattccagtactacaaactggtgaatgtgctgtggtccaagacgcccaatgcgcccaacgacccaggcccagggccgaacgtgcaggtaccgctgtcctatgggccgtttgtcagcgaccagagtgtcgtcgtcgccaacaccaccatggaaacctacgtgcagaccgacaactgcaacgactgccaccagtacgcggcgattgccggaaaatccgggctggcgtcggacttctccttcctgttcagcaatgccgactcggcgaagaacacgcggctgatcaaacgcatcgagtcgttcaagaccctcaaggacaacccgtaa

SEQ ID NO: 224 - DNA, 771 bp, Pseudomonas entomophila
atgggttctattactgatcatgatcaactgatcgcttgggttcaatcgctggatattcctgagcccacgaaaagtattgcgcggtcacgcaatgcggtggttcgcgccagcagcgaagaagaaggagctgcggtggtgcgcggtagcgtgacatcgttcgttactggattgaaacagcaagcgcgcgatgatgtgcagaacagtacgctgctgatgcaactggcggccgacaagaaatataatcccgacacgcaacgggaggagtggttcaagttctacaccgatggcttagccaacctgggctgggggcgcgtcagttcgatttaccagaaatataacccgcgtaataccaatgtcaccatggatgaagtggtgctggaggtgatcgctgcggttgtcggtgctgacagtgccgtgtacaaggtcaccgagaagaccttcgcggcgctggaaagcaacccgaagaatcagggggcgctgaagctgttcgacagtaccaccactcgcgacgacatcggcacgttccagatccttccggtcatgcaggaccgggatggcaacgtggtcatggtactgaccacagtcaacgccagcaccactgtgcaaaagggtagcttcctgttctggagctggagcaagaccacggcctggatgtatcgggctgcgcagcagacggtgctcaacgaatcggtgtactcacgcgtgcgtgagtcggtgatccagaaattgggcaagaatgccgaagattttattgatggtctcgatatctaa

SEQ ID NO: 225 - DNA, 783 bp, Pseudomonas entomophila
atggcattatcagccgatgaagtttatgtggtttcgggcaacctgctgtctgcaatgcccaagcttgttgatcctgtgatgttcgaagattttgccaattccaatttgctctgccaattggcggcggacaagaaccaaggcacgcggtttgttgatccgcccgcctggctagacttctacaggaatgcattgggcaaggtgttctggaggatcagtaattccgggacggtcagttttaacataccgcctctggttcgcagcataacgataaaggaagtgctggagaagacgttctataaaacactggatcatgaagtctcgctgcaattagatagcagtatcgagcgtttggaagagcagccagaagagagtgctgctgcacgcttgtatcgtgcgaagacccaggtcacttacaagtccgccgtctcggacctggccgtccggccgcaccccatctcgaccattaatctgcagataagcgcggtgcagagtggaggtaaaatatcggtctgtagtgtctattttacaacgtcggctgatattgaaagtgatgtgttcaaccagaagtttctggtcagtcagctccggggcaatgtcagcgtgagtacgtttgatgcaaaattgctggagtcgagttacgcgggtatccgacagagcgttatcgaaaagttggggcctgaaaatatccgcgagaacatcatccaggtgtcagctgaggtgttctccctcgcgggcccgcgccatgccggtgccaagcagttcattcaggaactggaaatctag

SEQ ID NO: 226 - DNA, 270 bp, Pseudomonas chlororaphis
atgtcggctcaagaaaactttgttggcggatggactccttatcacgaactgactccaaaggatcgggaagtattcaaagaggccctggccgggttcgtgggtgtgaactacacccctgaaaaagtttcgacccaggtcgtcaacggcacgaactatcgttatctgtcgaaagcaacggtgcctggctcctcggacagctggcaagcggtagtggaaatctacgcgcctatcaaaggcaagccgcacatcacccagatccaccggatctaa

SEQ ID NO: 227 - DNA, 270 bp, Pseudomonas rhodesiae
atgtcggctcaagagaatctcgttggcggatggactccttatcacgaactgactccaaaggatcaggaagtattcgatgaagccctggccgggctcgtgggtgtgcactacaccgccgagttggtttcgacccaggtcgttaacggcaccaactatcgttatcagacgaaagcaacgcagccgggttcatcaaacagctggcaagcgatcgtggaaatttacgcgccgattaatggcaagccacatatcacccagatcatccggatctaa

SEQ ID NO: 228 - DNA, 270 bp, Pseudomonas rhodesiae
atgtcggctcaagaaaatctcgttggcggatggactccttatcacgtactgactccaaaggatcaggaagtattcgatgaagccctggccgggctcgtgggtgtgcactacaccgccgagctggtttcgacccaggtcgttaacggcaccaactatcgttatcaggcgaaagccacgcagcctggttcgccaaacagctggcaagcggtcgtggaaatttacgcgccgattaacggcaagccgtatgtcacccagatcatccggatctaa

SEQ ID NO: 229 - DNA, 273 bp, Aeromonas hydrophila
atgtcagaacaagcagtgttgttgggtggatggactgcctaccacaagctgagcgccaaggatcaggccgtattcaaccaggcgctggaaggatttgtcggggtgcagtacacaccctttgaagtctccacccaggtcgtcgccggcaccaactaccgtttcaaatgcaaaagcactgtgccgctgcccaacccgatccacggggaagccgtggtgcagatcttccaatccctggatgggtcggcccatatcacctccatcaccccgatttga

SEQ ID NO: 230 - DNA, 273 bp, Aeromonas veronii
atgtcagaacaagcagtgttggtgggtggatggaccgcatatcacaagctgaccgccgaggatcaggcagtgttcaaccaggcgatgaaaggatttgtcggggtgcagtacgtaccctttgaagtctccactcaagtggtggctggcaccaactaccgcttcaagtgcaagagcactgtgccgcttgccaaaccgatccatggcgaagccgtggtacagatcttcaaatcactggacggggatgcccatatcacctccattaccccaatctga

SEQ ID NO: 231 - DNA, 273 bp, Haemophilus piscium
atgtcagaacaagcagtgttgttgggtggatggaccgcataccacaagctgagcgcaaaagatcaggcggtatttgacctggcactgaaaggatttgtcggggtgcagtaccagccgtttgaagtctccacccaggtggtggctggcaccaactaccgtttcaaatgcaaaaccacggtgccgctgcccaacccgatccacggggaagccgtggtgcagatcttccagtctctggatggctctgctcatatcacctccatcaccccgatctga

SEQ ID NO: 232 - protein, 578 aa, Pseudomonas sp. VLB120
MSTSFTQFTSPAGQAPKDYNKLGLEDQLPQFETDWNNNLTGWTQSSIIGNPWSNLNDAPRSGYYNPLVEGFGDVTVPAITWAPFPNRLWTFFYNNGAAIVPQLGGNAMTLEQVMELADHGQITLNNTLYKLYDPDNQGTLLQLPAKRCPSIDWKGQYTAFSPSGPRGWLDEYCEWSIVRDTDGNMRKITFTCENPAYFLAMWRIDPNAVLGLYRDYIDPNVQLEDLYLRYAVDCPTGKAGDPVIDPTTGQPAYDTVNKWNAGTACVPGQYGGAMHLTSGPNTLSAEVYLAAAATLLRPVSSSQNAQSLICCAQYGQNYRNSDPHIGFMANTKAVNNRLSLTNPIGLYLQQPTDFSAWKGPQGQDVSQYWRITRGTAKSAANGSDQILQAVFEVPQSAGFSINDITINGQRVDYVWVIAQQLLVGLSVTAKPITVTPPSFPCVQARVEGLQPWPVQLLPVDLFYGQSPTDLPAWLAPGSSNSFVLVVQGADPSTTTQNARVQFSNPGITAQVTHYLPDASAIPGQTNSGGTQAYILTITVSPTAAPGLVMVRALNPGEDANVSAADHPWEAGLALVPGA

SEQ ID NO: 233 - protein, 534 aa, Pseudomonas sp. VLB120
MSRSRLSLISLLSGMLLYLSALPPAAAATMSDADSCVQQQLVFNPASGGFLPVNNFNATNQAFMNCFAWQLFIALNWPVNPGWPATASLAGEPDMNSTLAQFGVPSSPGQPMSVAPVWASYKDANDIFLPGAPTPTGWGVQTMVPSGCSTQGSLKALKVGARKFMNATSEGAINALHGFHLSTGTVASIPDPVMEASGGWLTDQSGNLVFFERKVGKAEFDYIVEKGLYDAANQLKVAQNLDGNTPEGLSLPLGEPMRSLPPTPVPQEQLGALELKAAWRVLTGKPELFGRYLTTVAWLKRPDTLECTQEVVGLVGLHIINKTQASPNFIWTTFEQVDNVPEPDQAPPQGTPPNGFSFNNPDCGSGPACEPNVARIQCKQYHPDKDCTDLFPRDQPVQTTREHPVPSDLQALNSAVQSNFAQQTHGQSVFQYYKLINVLWTLAPNPPSPEPGANAQVPLSYGPFISQGNVPVANTTMETYVQGDDCNKCHQYATIAGSPSLASDFSFLFNSASSAGHKSLIKRVKAFETLKDRP

SEQ ID NO: 234 - protein, 577 aa, Pseudomonas putida
MSTPFKQFTSPAGQAPKDYNKLGLEDQLQQFETDWNNDLTGWTESSIIGNPWSGQNDAPRSGYYNPLVEGFGEVTPPAITWAPFPNRLWTFFYNNGAAVVPQLGRAMTLNQVMELADRGQITLDNTLYTLYDPDKQGTLLQLPAKRCPSIDWNGRYTAFSPSGPRGWLDEYCEWSIVRDANGNMRKITFTCENPAYFLAMWRIDPQAVLGLYRDYIDPSVQLEDLYLRYTVDCPTGKAGDPVIDPTTGQPAYDTVNKWNAGTACVPGQYGGAMHLTSGPNTLSAEVYLAAAATILRPVSSSQNAQSLICCAQYGQNYRNSDPHIGFMANSTAVKNRLSLTNPIGLYLQQPTDFSGWKGPQGQDVSQYWRITRGTAKSAANGSDQILQAVFEVPESAGFSINDITINNQPVNYVWVIAQQLLVGLSVTVKPLATTPPSFPCVQDRQTGRQPWPVQLLPLDLFYGQSPTDLPAWLAPGSSNSFVLVVQGADANTTAQNARVQFSNPGVTAQVTQYLPDASAIPGQTNSGGTQAYMLTITVSPNAAPGLVTVRALNPGEDVNVSAADHPWESGLALVPGA

SEQ ID NO: 235 - protein, 528 aa, Pseudomonas putida
MSSLRLSLLSLLSGILLCLQTLQPAAAATLSDADACVQQQLVFNPASGGFLPVNNFNATSQAFMNCFGWQLFIALNWPVNPGWPATPSLAGEPDRQSTLAQFGVPTTAGEPMSVAPVWASYKDANDIFLPGAPAPTGWGVQTLVPSSCNSQGSLKALKVGARKFMNATSEGAINALHGFHLSTGTLASIPDPVMEASGGWLTDQSGNLVFFERKVGKAEFDYIVEHGLYDAANQLKLAQTEGLSLPIGEAMRELPPSPVPQEQLGAIELKAAWRVLTGKPELFGRYLTTVAWLKRPDTLACTQEVVGLVGLHIINKTQASPNFIWTTFEQVDNVPEPAQVPPQQTPPGGFAFNNPECGTGPECKPNVARIQCKQHHPDRDCSDLFPRDQPVQTTREYPVPSALQALNSAVQANFAQQSQGQSVFQYYKLINVLWTLAPNPPSPEPGANAQVPLSYGPFISEGPVPVANTTMETYVQGDDCNQCHQYATIAGSPSLASDFSFLFNTASSASQKSLIKRVKAFETLKDRP

SEQ ID NO: 236 - protein, 577 aa, Pseudomonas poae
MSTPFTQFTSPAEQAPKDYNKLGLEDQLPTFETDWNNNVTGWTQMSIIGNPWSNLNDAPRSGYYNPLESGYGTLTPKTITWQPFPNRLWTFFYNNGAAVVPQLGGKAMTLDQVMQLTDHGQITLNNTLYSLYPDPQATQLQIPSVLCKSINWNGPYADFSPSGPRGWLDEYCEWSITRDPDGNMRSIMFTSENPAYFLTMWNIDPGAVLGLYQAYVDPQVKLEDLYLRYTADGPTGKAGEPVLDPTTGQPAYDTVNKWNSGTVRIPGVSGGAMHLTSGPNTLSAEIYLAAAATILRPLSSSQNQQSLICCAQYGQNYRNSDPHIGFSANQAAVNNLISLTNPIGLYLQQPKSFSTWKGPQGEDVSSYWRVTRGTAGTGPNNSDQILQAVFEVPASAGFSINDITISGTPIDYVWVIANELNVALSVTPAPLTAQPKECACVAANTTDAQPWPVQLLPIDLFYGQSPSDLPASFAPGSSSQFVLVVQGADPNTTAADARVQFSNPGITAQVTQFLPDASAIPGQTDGGGTQGYIMTITVSSNAAPGLVSVRALNPNEAANPSATEHPWESGLALVPSA

SEQ ID NO: 237 - protein, 529 aa, Pseudomonas poae
MNGWLRPLRRARLRIVCTITCALLPWLAPAPASAASDAQSCVSQLVFDPTSGGFLPVNNFGTEQAFLNCFGWQLFIAMNWPVNPGWPANPSLAGEPDTQSSAAQFGVPPTPGQPMSNAPVWASYKDASEIFLPGAAKPSGWGVETLVPSNCTATGNLKAFATGARKFITATSESAINRKHRFHLSSGTQVTLPDSIMEASGGWLTDQSGNLVFFERKVGKAEFDYIVDNGLYDAANQLIVAQNSDNRHPAGLSLPAGKLVRELPAKALPQEELGALELKAAWRVLTNKPALYGRYLTTVAWLQRPDTLQCTQEVIGLVGLHIINKTQTQPNFIWTTFEQVDNVPDGGAAPPEGYSFNNPACTGDACTPNVPRVQCDATHTPPNCTPLDQPVQATRANATPQDMQALNTAVQQTFAQQTQGQSVFQYYKLVNVLWSKTPNAPNDPGPGPNVQVPLSYGPFVSDQSVVVANTTMETYVQTDNCNDCHQYAAIAGKSGLASDFSFLFSNADSAKNTRLIKRIESFKTLKDNP

SEQ ID NO: 238 - protein, 256 aa, Pseudomonas entomophila
MGSITDHDQLIAWVQSLDIPEPTKSIARSRNAVVRASSEEEGAAVVRGSVTSFVTGLKQQARDDVQNSTLLMQLAADKKYNPDTQREEWFKFYTDGLANLGWGRVSSIYQKYNPRNTNVTMDEVVLEVIAAVVGADSAVYKVTEKTFAALESNPKNQGALKLFDSTTTRDDIGTFQILPVMQDRDGNVVMVLTTVNASTTVQKGSFLFWSWSKTTAWMYRAAQQTVLNESVYSRVRESVIQKLGKNAEDFIDGLDI

SEQ ID NO: 239 - protein, 260 aa, Pseudomonas entomophila
MALSADEVYVVSGNLLSAMPKLVDPVMFEDFANSNLLCQLAADKNQGTRFVDPPAWLDFYRNALGKVFWRISNSGTVSFNIPPLVRSITIKEVLEKTFYKTLDHEVSLQLDSSIERLEEQPEESAAARLYRAKTQVTYKSAVSDLAVRPHPISTINLQISAVQSGGKISVCSVYFTTSADIESDVFNQKFLVSQLRGNVSVSTFDAKLLESSYAGIRQSVIEKLGPENIRENIIQVSAEVFSLAGPRHAGAKQFIQELEI

SEQ ID NO: 240 - protein, 89 aa, Pseudomonas chlororaphis
MSAQENFVGGWTPYHELTPKDREVFKEALAGFVGVNYTPEKVSTQVVNGTNYRYLSKATVPGSSDSWQAVVEIYAPIKGKPHITQIHRI

SEQ ID NO: 241 - protein, 89 aa, Pseudomonas rhodesiae
MSAQENLVGGWTPYHELTPKDQEVFDEALAGLVGVHYTAELVSTQVVNGTNYRYQTKATQPGSSNSWQAIVEIYAPINGKPHITQIIRI

SEQ ID NO: 242 - protein, 89 aa, Pseudomonas rhodesiae
MSAQENLVGGWTPYHVLTPKDQEVFDEALAGLVGVHYTAELVSTQVVNGTNYRYQAKATQPGSPNSWQAVVEIYAPINGKPYVTQIIRI

SEQ ID NO: 243 - protein, 90 aa, Aeromonas hydrophila
MSEQAVLLGGWTAYHKLSAKDQAVFNQALEGFVGVQYTPFEVSTQVVAGTNYRFKCKSTVPLPNPIHGEAVVQIFQSLDGSAHITSITPI

SEQ ID NO: 244 - protein, 90 aa, Aeromonas veronii
MSEQAVLVGGWTAYHKLTAEDQAVFNQAMKGFVGVQYVPFEVSTQVVAGTNYRFKCKSTVPLAKPIHGEAVVQIFKSLDGDAHITSITPI

SEQ ID NO: 245 - protein, 90 aa, Haemophilus piscium
MSEQAVLLGGWTAYHKLSAKDQAVFDLALKGFVGVQYQPFEVSTQVVAGTNYRFKCKTTVPLPNPIHGEAVVQIFQSLDGSAHITSITPI